European Patent Specification EP 3 849 304 B1, published January 10, 2024. Title: COMPLEMENT FACTOR H GENE KNOCKOUT RAT AS A MODEL OF C3 GLOMERULOPATHY. Applicant: Regeneron Pharmaceuticals, Inc. The sequence listing filed with the application follows.

SEQUENCE LISTING (26 sequences)

SEQ ID NO: 1 - DNA, 97474 bp, Rattus norvegicus
  misc_feature (1)..(189): Exon 1
  misc_feature (59)..(78): rGU1 Target Sequence
  misc_feature (97)..(242): Deleted Sequence in Clone AA8
  misc_feature (132)..(134): Start Codon
  misc_feature (218)..(237): rGU2 Target Sequence
  misc_feature (18159)..(18344): Exon 2
  misc_feature (18640)..(18745): Exon 3
  misc_feature (21167)..(21243): Exon 4
  misc_feature (23369)..(23560): Exon 5
  misc_feature (23995)..(27715): N = A, T, C, or G
  misc_feature (30320)..(30490): Exon 6
  misc_feature (34023)..(34196): Exon 7
  misc_feature (48039)..(48233): Exon 8
  misc_feature (48597)..(48773): Exon 9
  misc_feature (60274)..(60456): Exon 10
  misc_feature (61569)..(61745): Exon 11
  misc_feature (67016)..(67189): Exon 12
  misc_feature (67904)..(68086): Exon 13
  misc_feature (68172)..(68351): Exon 14
  misc_feature (70591)..(70767): Exon 15
  misc_feature (73304)..(73486): Exon 16
  misc_feature (73657)..(73863): Exon 17
  misc_feature (74428)..(74601): Exon 18
  misc_feature (83593)..(83769): Exon 19
  misc_feature (85396)..(85572): Exon 20
  misc_feature (88223)..(88224): N = A, T, C, or G
  misc_feature (94119)..(94138): rGD3 Target Sequence
  misc_feature (94145)..(94327): Exon 21
  misc_feature (96799)..(97474): Exon 22
  misc_feature (96864)..(96883): rGD2 Target Sequence
  misc_feature (96993)..(96995): Stop Codon
cctaaactaactttcaacttccctttggggcaagtctgtctctgctgtaaccacagttcatagcagagaggaactggatggtacagcacatacttctcttcgagtcaactgctcccagatagatccaagacatgagactgtcagcaagaattatttggcttatattatggactgtttgtgtagcagaaggtaagcttaaaaccaccacctttctcccttctgactgagccgcattataaaacatttgctgataatatttctcatagcaattattcaaattaagtctagaaaatgtgggtaattactagtctgtaactgaatggcttttggtggtaagtttaaaaaccgtgaacctttcacttgactattgtaattgatagttcagcttgatgtaaaactcaagacagtgctttaaacatgtttttgcaatccataattaggcatagacatttaacttgtagttatcaggaaatacaggctcctctttttctcatgagtgtccctgaagtactatatgtaaaactagttagaaatatataaatatccaaagtcaatgaaagcacttacttttttctttaaatgggtggatcgatttcaggcttatttctaaaccttcctaactacatcacttagctgatatttccatggttttaaaagtttcgtatgtaagaccttcaagtatgagataaaaagaaaataaaatttgacatgtaacctgcattggacggatctgatttgtttctggttttgttttctgtgaatacgtgtggggcatgtttgtttctgaagccattttgaagtaggtaatgtgactgtcggagttctttcatgacaataacagggtctgactttattattcacttaaattctcccaagactgcttagtttatccaatgaaagagctttgctttcccagtttaggaagggtacctagttgtgggataaacatttaatcaactcttctttgtgttttgattgtttaagatagggtgtcactacacccttgagctcactgtagtcctcttgtcagcagcttcctatgggctgaggttaccagtgagagtgactgccatgcctgacttagcactttttatataaagtgaatgacataactttaataacttccttaaatgtttctcttagccaatgcattgtaatttgaagctttgctgtaaccactactcagtaaagaatactaaaattatcctctgactggatgtttaccaacccacataagaagagtagatatggtttctcagttgtatcttttactaaaattctgaaaaaaaaatttaagggtattttatactttttgaaagagtaaacattttcaattatattttttaatgttattccttgaattttagcttaagagtcttgtattcagatgccttatagactaaggcagtcatttccttgtatatgaaaatataagtattgctgaaatgaaatgtgattatattggccaggaattctaaagcaatgttgatattaccaagcataactaaactttttattttgttaaaggcaatgttttcatcgcttattttagtgttctacttgaataataatgtttactaagaggtttttaaagatatataagattaaagaaagaactattttatgtttagctaacttttaagtcttaattgatataaatcgaattaaggtgtctacacaattacaaagcagaatttcaatattaaaaaggaagtgccgcgatgtttgcgtgatactttaacgctaatgatttaaaaatcctcatttatgccatggatgtcagctgatttttttgttattgctggatttgaattttcatcagtatgtattcaaatgtggtgccagttcttgctgatgaggtgggcagttacactgtgtccgatactgtttcacagggattttcctttcattcacagatgaaaagagagtttagtttctaaatcattatgtagggtaacctcatggtctccacaaaatgaatgtaaacagatgggagaagtttcatggattttcagtggacacagtactcccactttagtcttagcttggctggtgacccgtgtctatctcaaatgtaaacaatttaatcagtctatcaacttaagaggaatttcagcagaagagcttggatcaattaaaacaattatgtatatgctgcaatgtttgctcctgtttctattctattagatgctggctactaagctgatttaaaaaaaaaaagtttgtgaaatgctctcatattaggctttctgaaacagggaagaaaagatttcataagtattttctgccctgataaagatcaacattcatctaaaaccaatgttagctgggccagcaggaacggtaaacacaataatgatcttgcttggcaaagaacctggctacttgagttcaattcatgggccccacctggtgaaagggggaaaaaaagcctctacagactgtcctccagtttcctcatacaggcatggcaactgtatgttacacccactcaaattaaaagaaaataataaccataacaaaaaatttaaactccactattaataattaaagaataataaccaaaagaagaactatgaacccagcttgtttgcctccctccctccgtgcccctctctctctctctctctctctctctctctctctgccccgcggggccgcccccacagccccctatatccacacccccaagaggggaggggagaaggccgggcgccaccacccccgccccaccaaacaaccccccagaccggccctacccacgcgcggacaaccacaccacgccggcgaacacccaccccccacagccgaaccaagcaacacacaccacaacccgcgaaggggacccgtaaccggccctctctctctctctctctctctctgtcccccccctctccttttccccttttctacttgccaagggctttctcatatctttttagtgcagtgcttgactgtattcacacttctagctgccaagaacagtcaatggtgcttcctgcaaaaccacacgctgatcagaattgggtcagatttacaggacaacctgtaacataagagagttccttggttgagccgtataatttcagttctggggaatggattatacccaagctttccaagcattttactctcacaattgaatattgtatgaaattaggccgcagcccaggattgctgaaatgaaccaattaaacctgtgctgaaacaaaaccaaataaccactgcgtgctttctggggagataagtgttttctaatcctggaggtttaaaggacaaaaaggtcctttcaggcttagagactttaatcatagaatggagaattggtttaattctataatgttttaagtatatgattttttcaaacttagtttaacattgatgtggaaaaattgatgttatatacattaattatgagttaataatagttgctttgggggaaatttagagaaaagttaattattcttttatgtaaaatgatattatattatgtcaaaaagtcaagtgattcaatgtaagatatttatacttttccttaagaaaaagaattaatatggagtgtgtcttacttttcccttcactctgtgtccaaagttgaaagcagctgattctgcagcgttcaccacatcttaactataaaccatgtctacagcttttcctttggccttagccatattgaatatgaaggtttcacatgtcccaagtgactgaatgaagacggatgcagcaagttgcaatacagaagtgatatgtgcgtcactgtgtatgtattgtcacatacagtactgcatacacagagttctgtcagtagtatcactgctgtcctttgtcttcaattactttagttcttcgagatagagtccccctgtttggcccatgctggtccttaaactcctagtcttctggccttagcctccctagtactgaaattcaatatcaagaatatcttatgcagattttctgttgctttcattcaactaaattgacagcaatagctggaccttccttagaaaaatggaaaaatatttaaatatcaaaaccttctaaagaagcaacctatagttctctttttctagacagaaaataaaaaaaaatccaaaaagtaaaggtcaactttaaaacatacatataagtaatattatatatactgatcatgttatatttagaaatatatatgtatatgcatatatgcatataattatagttatgaaaataagtagtcatggggtgaaagaaagtaaaggagataggtgggcagtattggagagacaagaggaaaggggaaatgatgtaattagattataatctaaaaaatataaaagaaataagaataaaaaagaaatggaaattttggtggtaaactaaaaaataacgtgtggatttacaaagagaaaatacatgtctgcatgtcttcaatgctttcattgacacagaaaaccaatttcggtatcttgcttttatgctcctttatcacagcaaaaatttataaacatgtcacaggacaaaccgggacttttaaacctttcttgtatttcaaattataataaatatttggatttattgctgcagtctctactgtgagcataatgtttactttctttctttttttaaaatcataatgttttcaaagccagaagacatctgaaaactctgaagttgactatctttggtatttctttggctttcttgtttgggacaaaactgaaggaattcacaatgtcaaccaaaccacctattgccattaatagtacctacttgcaaagtcctaagtttccattaaccaaacagcacaaaccgaatccattgcagttgtttcgtttctcccattgaggaaaaaaaaacaacatcctcgtagcctcccttttctgaaccttgaaattggaacagtaatctttttcacacacaccatggaggcagtgcatagatagatccccacatttctttaaggaaagtggttggattgaataatcaggtgtgggacagagatgtcaacattgaaattcttccttgagtttgaattttgagaagagtctaaaagaggtcaggttgaaagaacttgcatcctgtttgataaggttcttcacacagtctagcatatttattaagcttctcggttgtactctcccaggccccagaggtcagaggtccatgtatgccaccttctatcacacttgcttaaatccaccctagtagatgcacatgagtattagagatcattatgtaaactagacactagggcactactagtttattacctaaattaggcattaatgtcagtggagcaagtaacctctatccctacaacacatgttttcaggatagaattatatttccctaaatcatgttacttggcattgtgccccaattgtcttcagtgtcttctttcatgcaactcttaaagtatttgacatgtttatcgtaccacaaactcaaccaacctgttatttatgtgtaagggaccacatagttaaatttagtgctattatgtgtaatttactgtgaaatttcactgatagaggatagaactggaaaatggtaagggacaaaatagaccaaagacattctgagacaggaagcttcctaggatgaaatgctgtaacaggtgacaaagggtggagaagttgctcgcaggcagggtgaaggtggtcagtgaaaacaagccttgcttatcatcagcacagtcatgttctaggaatgtgcatgccctttgccaggatgctatttaaaactaaaccatttaagtagtgcaaagcggaatttttctaaggtaggaactgccacagagtaaatagtctgcctctttgtccttagattgctcaattttgaactctctctccccttccaaattaatccatgtttatttcctgactctgattgttagtctttacttcctccttctctctctccttccctcactctctccctcagccctccctccttcctctctctctctctctctctctctctctctctctctccacacacacacacacacacacacacacacacacacacacacacacacacacacacacactacctctacctctcgacatttaggcagatgctgtccaccaaatcctcaaacgctcagttgactgatgttaactttagcttttctcagagcacaaaacatgaaaaacagataaagtaattgggaaaaaaaatgttactttttttttttggtttaaaattagaagaaaaaaaaagtctggttcagataaagtcaagcaactaaacagaaaaaaattccaaccgtgaaataataaaaagaacacacggatttgacagaacacttttgttttgacattttcacttagaaagtctagtttctcacagagtgttaactggaaatgggatagatagaggacgattatagaaacaccccttcaaaggttccgagggaacttttatacttcgagctaaattcaagtgactctagacttcaaaaaccgcaacatagacagatgtgcaaactctgtagagaactttcagtgcatgcaacaggcattcaactccaccagacagtggtgctcttgccactgcctcctcctccttttcctcctcttttttttccctcaagttgtctctttcttttcctttttccaagtcttgtcttttaagtttcccatttgccactctcagctgttggtggccctattgactatatgggtgtacactgtgggaaagttcctacagtcttttttgcgttcgctctctcctctattcacaatcccttttgaataacttttaagtactgcgcaatataatactttccaaaaggttgtcatttagtggagaggaaaagaatgaacagtgtattgaaatattcacatacagtagctcatcttataaactattatgactcagattttaaaaagttcctaaagcagaaaactgaagttgaaaagatgtgctgtatacacaaaatgaatttttgttcagctacaaaaaattatgaaatttataggaaaaattgatgaattcagactcacagggagacaaactctgcatgctctccttcacattttgattctagtttttaatacatatactttatatatactgcatatatctttgtttaatatgacgtgtgtgtgtgtgtgtgtgtgtgtgtgtgtgtgtgtgtgtgacttatggatagaagacatggaactagaagtggaaaaagaaccgtggaggaagggaaccatgaaaaacacaagtggattgaccaagacagaggagggagacagggtagaaaggtgaagagaagaaaataaaactgtttttacaagtcataaaaaaggctggatatggtggcacaccatagtccctgtatgagggaagaaaatacagggcagttctctaagttcaaggccagcttaatctacaaagtgaattcgaggacagtcaggcctacacgaaaaactatgtcttggaagaaaaaaatgcctcactataatataatataaaatataatataatacttcatatattaacttaaaaaataacatgaaataataattggaatgggaaaatgggtcaggaacaggagagggtgagggtgacggtaactggatacagatgttctgctgacttagttctatgttgtttctctgagaaaagtcagacaaagctctcaattcacaatcttctctctccagtatgctcaaaggacaggcatggagcctcaagtagataggctacggatgctgcataggagttagtcagaaagaccaaagaggatgttaacagaaaaacatcagatatacagaaagaactataggttctataaagctgtggggctcatctccacacctacaacttaacttggcttaagtttcacaaggattagtgggaggttaggaaagaaaaagttttcccttttatttatttttgttttgttttgtttttgatttttttaatttatatttcaaatattatcccctttcctggtttccctttcataaaccccctactttatcattttatccccctgccccttcttctatgagggtgttcagccacccaaccacacacaccttcccgcctcccctctctgacattcccctacactaggggggtccagccttggcaggacccaggggttctcctttcactggtggccaacaaggccatcttctgccacatatgcagctggagccataggtctgtctgtgcatactctttggatggtggtttagtccctgggagctctggttggttggtattgttgtttttatggggttacaaaccccttcagctccttgaatcctttctctaactcctccaatggggaccccattctcagttcaatggttggctgctagcatcctctgtatttgtcatgctctggcagagtctctcatgagacagctatattaggctcctgtcagcatgcacttcttgacctcagcaatattgtcgagtttggtgtctgtatgtatatgggctggatccccagttgggacaggttctgaatggccatttcttcagactttgctccaaattttgtctccctatctcctcctatgaatgtttttgttccccctttcaagaagaactgaagcatccgcattttggtcgtctttcttgagtttcatggtggtctatggattgtattttgggtaagctgggcttttgggttaatattcacttttcagtgagtgcataccaggtgtgtgtgtgtgtgtgtgtgtgtgtgtgtgtgtgtgtgtgtgtgtgtatgtgtgtgtgtggttgggttacctcactcaggatgatattttctagttccatccatttacctatgaatgtcatgaagtcattgttttcccttgttctaatccttatcctcggcatcccactgatacctctcatccactccagtactggagctgctaaaacattcagccttagttactccatcttgtggctaaactgctttgtgaggcagccgttcaagcctaatgaaaccgttcaatgtatgctaacagtttattttaaaaagacaatattgaacctggacccttcttggtgttaggagactcttgtgtaaatgctgcctttttcagaaattgacttcaagctgactcctcaggaggcaaaaattccaactactctggtcgatttcactcaggtttagccatatacctgcctattatgatctaggtgcttctcgagggtattagttttataaagaaaatttataattatttctgtatgttttagaaatagaaatttattttccaatgttcattaaatataaccaaaacttaaatttttgtagtttgttttttaaagtactttattgcaatttatatttactttgttcaaaaaaattcaacctaaatattcttgcactatttataaattaatctaaatatttttagtaaacaaaatactctttggatcatatacatgcataaacttaatactcatttatatcaataagaaagcagatgagaaatttaatgaaactaacattcttgctcttcccactttattcttttacttttttctgagtaatgtgtatactccaccatctgctaataaatatatttttaaaatgatgcctctcattctttttccaaaatccttgtagaagctataggaagagaaaaaaagatgacctctccatctttagtctttcaaaagtgtgggtacaactgatgttttacaaaatataaaaattcattaagacttacttcattgcagcaagaacatttcaaagaacaattctgagacatattggcattcggaaaaggaattgcacttggtttgtcagtcctaattctttaaaatctgtatatgaaaaactggtaatcatgattattaaaacagcaaatatttgctttaaagttccatcgattatagttatcttcctcaagtttaagtaaaactcttgttttcagattatcaaacctacacagtcattctgtttctggaaaacattcaagagtggcatttgcatctaagtaaataggaaattaacaaagaaaattcttaaaaagcaaaatcaactatttaattaggattggaccaggtttcatttgttggaatctgagtaaatatttaggtacaagaaaagtgagtttactcattcacctggacatagaagctgtcaacttccccgtgtcttaaaagtcttaagttgaatcacccgtctgaaaatgtgttcatcctttcgaaagcacttctctactccctatgtaagaaccacctgccctgctttcattaacaacttctcatttatttcaagcaaatgtgtttggtgtttggtgtacatttaggttgacagatggagaacatgaatgagcagaacttgttcctgtctagttagaacgcctggacggctactttcagtggaacgtgaaaaaatgtttgccaccctcaagacacacttaactgttattgtcgaaatacagtgaacgattactttaactatttaagccagaacacgagttatggatacacattatgttgagactctaaacaaagacaaacagcaactgaaaacagagggattgtttattttcccgagagcaacaatttttttttttttccgaagaccctggttttggcggtggcagtggtggggtattagcgccacctagtgtggagaagtttaactactgaaatgatgatcaaactaaagctcaaaaaactagcgaaagactcaaaggaaacccgacagcctaaacaattgctctattcttctataaaacatagcagtccttttatttcacatgctgtgtaccatcttgtagatggaagttccaggtgaaatatacgcagtagggtgatccattgctttttaaaagagtagaaaagattagtaaagtagagcgaattgtcataaaatcaagaagtaaaagacatgggcaatttgaacagtatttttagaaataaaatgaataatgagcctagaacctgccatctaagaagcaccatgctgggttttactaacaaccatttaaatatcagggtatttgttacaaagttaagcagcaggcaatattaaatgtgattctatgccttagcactaatgttccatggtcacaattccagcgcctgggagtttaaggcaggaggactatgagatggagaccaacctggtctacaaagattttgtctcaaaaacaataaataggcaaagggaaggatacacggaaggataggtgcacaactactgtagtaaaatgttgattgttggacctgcgtgttagcgtcattggttttttactgtaaaatcaaactttcaaatacattttgaattttctgtaaaaaaaaatgttaagcgaaattcttctctgataaaacttaagaacacagctcaggatctccaatttacttcctatgcccaaacttaagtactagttgaaaaacgcgagccccaaacttaagtccagttcaaaaacacgagccctgttgtctgcacacttatcttctgcttctgccactttcagaaatcttgaaaaagttagtagatatttgaatttccatgtctttacataacaaaaagaagacaatgaaaataaataaagaaatacaatcaagaaacacaaactccccacaaacattttctccctattcttttaattatttgggaatctcatatcatacatatctacaattgcactcatctcctcttctcacatttgcccccttacctgtgagctccctcacccacaaccccgagagagagagagagagagagagagagaggagggaagagcgaaggaagagaagagagagggaagggaagagagagggaagggaagagagagggaagggaaaagggaagtgaagggaaaagggaaaggactagccaaggcaagtattcactgaatcacggtcaaattcctagtggccaagagaggttttttttttttttcctctgcccgcatccttggttgccagaagccaggagctgaggcaagccatgtagtagctggagcagggtaaatctagcaatcccaagcacatgtccctgcctgtactgcagtgctgtgggccagtgaaggacagggccagttctctcagacccatggacatagatagcgtggcttcaggcaacagcagacatcaacgtggtccatggccatatcaggaccactgaccaactaatggccctcaggggatgaatgcatggaccacgagcctccacatggtcttacgccacatcagcatgccccccatctcccgaccccgaggcagcaaagccagacgacatcactaaggtatcacacagcaatatagatctcatacgtccacatggatctcaggtttcttttggggctggtgcaacagcatagaccacagacaccatgatggcccttcaaggaggttgattccagaaagtgaacctttccttgtcttgggcctccattgttgctcataacttggggcatcttgaaactgtgtggcatgttgagggacagggggtggggagtatgggctacatatgatccaagatgataagttatgccaactctactgggcaatgacagcatgttgagcttagccccatctcacacttgtctctagttctgcttctctctctaggcacacacctctccatgtgtgcctagttcacttatgtgttcataatagtagtgctgggtggctttaggtcgactcacagctaccatgtctcaaccggtacttgcttcccattatgtacataacatataaatatatattatatgcatatatgcatatattgtatactacttttaatatattgaaaagtaaaaggaatagaacaaatgctaattttattaactttatatatttaaaatatataacattgtgttctgggtgatgcttgcttcccgttttacatacatatatacacatatatatatatacatatatatgtatatattatatactatccttagtaaacatattgaaaagtaaagggaatagaatacattttgttaactttttgtatttaaaatatgtgacacataccattgaattaattatgaacatagtatattactaattattattcatccataccacaaaacatagaatttccagcacctcagaagatctctgttggtttcttgcatatggaatgaattattttcatagttataggtacatatttgctcttaattgtttcacctcctatatgtgcctatgtgatttgtacaacagcacctcagtgcatggccactgtcaccctacaccactttgtgctggtcaggaagcacagagacactgctctgagggtgagaaagcacagactgagatgtgggagagccagagctggtttgggggtccccaggcctgtggggcctgcaagaaggcagggccccaggttggggacagcatctagctcagggcttgaggagagggcagctctggaccagcagggattgtccttagcttggaagaggaaggcttcttagcagttgtggttgggagtgctgagaagcctgctacaggagacttagctgctgccctgtagagctagttacctggaaagaccaccttcatgacattccccatggtggtggtagatgacagagacagtctgtgtttacccatattgtttattggctgttcattatggaaaatggatgcatacccacttctcagggtctgacctaagattaaatacctttcaacgtctggaatgtctgggaaggaaagcttattggctaagccctccgggcctctaggtaccttattagcacggagaattctgttctgccttacatgacctgtcacatttccttatacggggagtgtggcacaaattccaggtacaaaatactcacattttcaatgatcattttattcacttcagctgattcattctttaaacttcccttatcttgaggatcagtttcctttaacctaaagaactttagtgtacatttataattgttaaagtttctacttcgtttgagaaagtgtcctattccaaagtaaacacagaaatctgaaggttctcatctaacatccacagtgaaagaaaatatgcaaactctccctttggagtctgggatagcttattccacatgatttgtttccaactccacctgcgaatttcctacttttccccactgtgtaaacagaccatatttttgttatccattcttcagctgatagacatcctggctgtttctacttcctggatattgttggtagagcaacaacgatcatgggtgaacagatatctctgtggtagggtatggagttctttgggagtatgtttagaagagtagtatagttatattctatggcagacctgttgctagcttttgggagaaactttactctgattttcataatggctgcagcagtttgcactcccatcagctatgaaaaagttccccctttcctcacattccacactgatatctcttgtcattaatttatttaatcttattcaggctgggagaagatgaaatcacagagtagttttaacttttattccccaaatggctaatgatattaaacatttttaaaagtttctcaattatttttatatcatttccttcattgaaaataaattttgataaaatataatatattttgtttatagtttccccttctccaactcctcccagatccctcttcccaacccacccaaatctataccatttctttctctcatttgtatacaagcaggcgtctaaagacaaataataataataaaacaaaattacataaagtaaaagtcaaacaaactttataagaactctcctgtttttaaaatggcttgttctcattcttgatgctaaggatggcttttagtagagcctgagaaagttgtttggctttttgttatcattgtttttataaatagatactaggaattttatgcaatcattctgattttgagttgataactttagtcatatttggaaaactttaaatgttcaggtgtcatttctgctagttctctcatctacctttgaaccttcagatagatgtagcctgcatcttttgctttctgcacaaaagttggcttctgcagatagttctctttccaccatatttgaacatttctatctcaattttcttcaagtggagtacatttctttctgatttcagatgactgcagatcaaacaatataacaatattatttgtgatattaattcataacattaagataacataatttagagccatttttattttgaacttttaaaattatttttgtctttttcttaaagttcattaaagatgattgacttagttatttaaaatatatttttgctaactaatatctagatcagtgttgattttactgcttatttactcttcatgtctattttcctttttgtattttattttttaattttgtattgttattttacttatttacatttcaaatgtcatcccttttcccagtttccctctacaaactcctatcccattccccttcctcctgcttctatgagggtgctctcccacccacaaacccactcctgcctcaccaccttagcattcccctacactggggtattgagtcttcacaggaccaggggtctcccctcccactaatgccaaataaggcccatcctctcctacatatgcagctggaaccgtgggtccctccatgtatactctttggttggtggtttatgccttgggagctctggggggtgtggttagttgatatggttgttttctatggggttgcatcatgctcagtctgatggttggctgcaagcattggcatctttactggacaggctctggcaaagcctctcgggagacagttatatcaggctcctttcagcatgaatttcttggcttcatcaatattgtctgggtttggtgtctgcatatggatggatccccagttggggcaatctctgaatggtctttcctttagtctctgtgccacgctttgtcttatgtcttggaatatcctctttgtattttaattttcataatagttactatattttatagaaaatatagtgactaaagtttacgttatgcactcatactaagaagaacatttatcccaagactgaacccccagagaactggatggttgggggtggaggggaggatagggaggggaacatccatagagaaggggaggaggaggggttagggggatgttggcccggaaactgggaaagggaataacaattgaaatgtaaataagaaatacccaagttaataaagatgaaaaaaaaatgcttggaaaccatggggggggggaataaacgtctattcttgaaccttaaaaaaatgaagaacatttatctttcttacttcaatcattaatttaattaaattgtatctgggctgcaattttagcttgcattagctcacttctggtctcaaatatttcaaagcaaagaccttcttatgtatgagcttttgcacatgtgtttaagcacaaatctctcctttctaatagactacaataaatctgtcttctttcctgctatcttgagacatgttttatattagacactaaaagactcaaatattctaatgtgttgatgaactcaccagttctgtattttaaggaggactattaatcttgctgtgacttctgtgagactataggaacatccaggcttcacttaggaatcaggtaattccaataagacaactagattcagattctgcatgattcagaatgtttcaggttagacacaccttcaatatacatgtcttatttctaacatcgctaccattcttgaattcacataacccgggaccatcaattcacatacagaactaacacatataagaaatactgtagacctcagatatgaatagtacaggcccattccacctagatttagttcatgaattttcattgctcttaaaatctgtgctaaggcactcttataaatacctccacaccaacttttctgcactccatatttatatagtaggaacataactctgttctatctttttatattatttgaatgttgaatgtctccatatagtttcatgttaacttatatagaccaattttaattcagcaatatggctgctttagcaagggatcacatacaaagactttatctatctagaatgccacacctttaatccctctgggtggaaatagagatatgcccttagtacacacctttaatcccaaaccatgaaagtaaagctagttgttaaaaaaaaaagcaaccatgtgtggatgtaatgtcaaattgaggggcaaagtgatgaatcagagaaagattagacagaatgagttagtaataggatatgcccaactctcacgagaacagacaggaaaaggggatgagatgacttaacagtgcagcagggatggagagagagagagagagagagagagagagagagagagagagagagagagagagagagagagagaagaggaggaggaggagaaggaggaggaggaggaggagaaggaggaggaggaggaggaggaggaggaggaggaggagaggagagacgagacgagacgaggagaggagaggagaggagaggagaggagaggagagaagagaagagaagagaagagaagagaagagaagagaagagaagagaagagaagagaagagaggagaggagaggagaggagaggacaagagaagagaagaggagaagtcctggagcagagacaggttgtaggttaaggcagaatgagccagagaatgagaaggagccaaaagattagaaaaaattgtcagagtttgtttgagatcaagcagaataattcagtgataactcaagagaagtttgaatcagttatgttggaaagaagtttggaccagaacggttgagttgagtcagccagccagagtttcaaaagaactggaaagggtgagcttattcaacagtaagcctgcaagagtacaattatatctggtgaatgagttattttataaccttacttgctttatttttataagtagaaattattctataattcatggcatgagtttagaaaatactgcttagatttgctactaggaaatattttgagaatagtttattttatccatagttttgtttgtttgatttttttgtttgttctttacaacttagaagattgcatagtaaattttcataaagtcgtgcacataaatagctggatggacctgtaattggtatgattcaaagaaaaacaacatgcatattgtttttgaataggtatttcaaatactggtatgtttttattacttgtagattgtaaaggtcctcctccaagagaaaattcagaaattctctcaggttcgtggtctgaacaactatattcagaaggcactcaggcaacctacaaatgccgccctggataccgaacacttggtactattgtaaaagtatgcaagaatggagaatgggtaccttctaacccatcaaggatatgtcggagtaagtacttcatgtttgtaaaacttaagaaaatttcagctttgtactaaatcctttacattgtagcaatataaattatattactactgtaactaaagtgtaatcattttaaaatgtacttgtcctaaaaaaaaaaaaactaaatatggaagcgtgaagttaccttcaattataaaacatgtttttatattttcagtttctcttctattcaatgatatccaaatgtgctttcctgacttctacaaaaggtgtatttcatggaccatacactaatattatcttctttttattttagaaaggccatgtgggcatcccggagacacaccctttgggtcctttaggctggcagttggatctgaatttgaatttggtgcaaaggttgtttatacatgtgatgaagggtatgttgttaatattaaaaggcttatccttgaaaccatgtaggaacgctacaaatttgtactttagcaagaataaattttctattaacatctaaaatgtaatacagaaataaaactacgtcatgaatgcttttaattggatatcatgtgatctccataacactggaaagtaagcaatttatggctgttctgacatagtgttgaaataagggtgtattaagttgctatacacttaatacacaaaaattaagcattcaactcacaagtccttagtacattccactattgtacaatatcgtatgagatgggatagtttttttttttttatattagggacaatgagaattgtgaaaacaactacattatatggtaaccctcttaaagagattttatagtattcaaagaaagcaaaacttttatgtgtgaaaaattctttctcttgaatgctatttttaaagttgtatgcaaattactcttattccataggtgcgaaaggctaatttttcagaatcattgacttccctctctgcacagccactggttcgtcattcactccacagttcttcatttcctatcatacaagaaagttagagttgtaacattattccaaataattataaagaaaagtaaacactttgaatggaatctttttagttgccttttatttcctaacttgagacagtgaactataacggtttattctattcaagttttagaattagctccaaaatatccctatgctcaaatgctcaatgtttgtaacatcttactccgatcccctctcttacagaagcagaaaagtgcttatgagcatcataggattagcaggagaaataaatatgacccacccttgcagcacttcaaaatgatcccagatgaccacaaatacccactagatgctcatttttttatttaacttctccttgtttcacaacgtgaaggagacttttcaaactacaattttcaaggtcactgctgaccttattatttaaagccaacaaagatttctttggcctggatttttcaggttgttccattcttcacctttgaattagctcatcctaggccgtagaaactctctcatttctagtcctataggaaacaccaaatacgactcagcagttgtgacttcagtaggcaagcagacagcacacacaaattggaagctacagactagtccttttggcaggtcaacaccagacccaaaccagcagctgtccaaagctgaaggaaccattgggcttaccaaccatcctgacgtaatactgtggaatctgcaaattgccagaggaacttcaggagaatttcttagagaagcttctcagtggcagcatagtgaagaatagtgagacagagtaaacaaaatcaatgctcagtactcgtctcccactatctgtgtgatcataattatactctgtcgtctagagtcctttcatgtgtgtgccccagcaaaacatcatttgacataacttactttccaaaccgactagaagtttccacttcacttatttacctctgattctggctctcttcaagtcactgttgccaccttgtatttatcaagtgtaaacactgatagaacccatctaggtcaatagctgtgtatattgattctgaatcaccaatatcaaatcaatcaaattactgacaattatcgcgtaaagtcctcataccacgtaggataaaaataggtaaaaagcagttcatattcattcaaatttctgttgatgaatgttctatctatcttgggataattgctttttttaaacccagaagtgaaaggtaaggataggagaggcttatttcaaccctattttttttactcatcctttttagtcctgtgcttttggctaaattttctctgctaaaaataaacaaatataaataaatataaatatagggttttatgtactttgtagtagaatgactccttaggaacaataatgttattgtccaaaaccatcgtgaatgattttgagatgacactgcaaactgattttcccccatatggacaaccattttttttctcctttcccctccctccatgaacagaaatccagtaaggttttgtgtagaattttatagattgtctgaaggaacttagtgtgatggatggatctctgcagtgaataaaaagtctttaccaggagcttcatttcttttctactggaaaagaaattattctgtctcctctacagcaagcatcaaggaaacacttaagtccaatatccaaaactaacatattctattgaagtattttatttccacaaagatttaatagagagatgaaaataataaaagaatgagaaatatttttcccttccaaatctcttactggaggatatccaagactgcacagagcttcaaactacacaaaaacacatgatgtctcaacacaaattattatgcttgcatttttaggtaccaactcttaggtgaaattgattaccgtgaatgtgatgcagatgggtggaccaatgatattccaatatgtgaaggtaaatgaaaaacagatttgtatgtatgcctaaagatctaaaatagataagatttcccaagctgtgtagaaaaatattcttaaagtatatacttaagtatttcatatatttatgtgtgtgtgtgtgtgtgtgtgtgtgtgtatatatatatataattttatataacttcaattctctttttacagtccagtcattatccccctcccagtctgccctcatcccagtcccccaccccatcttaaagaggatgtcctcatccccttcatccctgccccaccagaccttcctactccctggggcttcaagtctcttcaggattaggtgcttttttctcactgaggccagatcaggcagttctctgctacatatgtgttgggaatctcatattcgctggtgtatgctgcctggttggtggcttgtctgagagttctcgagagggtccagattagtctggtcttcctatgaggttgtcctcctcagcttctttcagtttttccctaattcaaccacctgcgtctgactctttcagctgttttttgggcctatcagagggcagccatgttaggctcctgttcttaagtacaccatagcattgataatagtgtcaggccttagagcctcccctcgagatggatcccaatttgggatgattactgagcctcctttccctccctcagtctcttctccatttttgtctctgtagttcttatttatatcttttagtttctagtataaaacataagtactttgttatagtactattttgtatttgtatcaatattctgagaacactaagtctagagaatggtgaatttctcaggactactgtagattccttgaggtcttaggcttgacacacattctcatcaatataacttaaaactatctaaaacataatagatataaatagagattgatatacttttatgatcaaagttctgaatattagaaataccaaagccattttttccattttacatttcaaacactaacaatacataagaccatcactagcctataaaaaaagaccagaatttgaggtatgtttgtgaagaatgacacccctaataacatctagctagttacaggtgtgtaggctatcacatccatacattcctggtagagaatgttattgaaatacctttcacaattatgatgctgtgaaggttttatccatagtcttaattttagaaaaaaaagggggggagggaagcaagaattacaaaagaactcttgcctttcaattcttgctcacatgctgcttataggtagagcaaacagcaagaatgagaaaatgcaggtcttgtttgtaagtttggcgatagcatgtaaataacaaaggtccatccaaatgctgtatcctacttccatgggaagcaataaattagagaaagaagtggagtggaaggagagagggatggagaatgagaaggcacagtaagttctcctaatgagacttttctagtaaggaaatgagaagatgttcccggaacgtctgcatcagaatttacatggtgcttgtttaaaattgatgtttgaggcccctgaatggcctgttgagaaagtatctttgagtgagaagagcagaaaacctcactagcatatccattacatccaaagtttccttcagaaaagcaacttcaaatttcttcatggcggagaaattctaaattaaaaaaaaagtttaaaatttttgagcaatgaggtgaaaaggaaggaaacattacaaaaagtttttttcccctatgagaagaaatatcttcaaaattcattgatttaaaccttattagaatgcaatatcacgttgctttgaagaataaataatacatttgtattagactattccaaaatctcatatgtgttcaccatttaggagacacttgctatcacgaagatgtaaactgtcactctaagtaatagttttcttttcccattcccatagaagctgataagcgaactacccgagctacttagatgttgtgcaaacagtgatgctgaatgtttctcaaacctttaagtcctttccggcaggttgagcaggctgcgtggtgttttcattcatatacgtgtgttttatgtggaagctggtaaggtctgttagtaaaagcgatgcctgtattttcagttgtgaagtgcttgccagtgacagaactggagaatggaagaattgtgagtggtgcagccgaaccagaccaggaatattattttggacaggtggtacgctttgaatgcaactccggcttcaagattgaaggacagaaagaaatgcactgctcagaaaatggcctctggagcaatgaaaagccacagtgtgtgggtaagatacacagatgtgtctgcttcacatattctagtgaaagtatacatttcttttttaaagtacatttttaattataatagaattgcacaactcggatgctaatgaagtatgactgtttccttgtaactgaagttctttgcatgaagccttctattttgctttcagaactatatatttcatgcccttgtgtagtctctttaattgaaatagccaaggtgtccatgcttactgtggcttaatgacttggacaagatgtaaacacaggtgttgcaattcagtctagcctcagcgtctctggtgagtgttgtaaaactaccttgcagagcatatttttttaataaggtttttggaagctaaaggcttggcatgtgtttacaatcacacattatgatgatattttgttttcaatttatagttaggatgtatattttttagaaatctatttgctgcaagnnnnnnnnnnnnnnnnnnnnnnnnnnnnnnnnnnnnnnnnnnnnnnnnnnnnnnnnnnnnnnnnnnnnnnnnnnnnnnnnnnnnnnnnnnnnnnnnnnnnnnnnnnnnnnnnnnnnnnnnnnnnnnnnnnnnnnnnnnnnnnnnnnnnnnnnnnnnnnnnnnnnnnnnnnnnnnnnnnnnnnnnnnnnnnnnnnnnnnnnnnnnnnnnnnnnnnnnnnnnnnnnnnnnnnnnnnnnnnnnnnnnnnnnnnnnnnnnnnnnnnnnnnnnnnnnnnnnnnnnnnnnnnnnnnnnnnnnnnnnnnnnnnnnnnnnnnnnnnnnnnnnnnnnnnnnnnnnnnnnnnnnnnnnnnnnnnnnnnnnnnnnnnnnnnnnnnnnnnnnnnnnnnnnnnnnnnnnnnnnnnnnnnnnnnnnnnnnnnnnnnnnnnnnnnnnnnnnnnnnnnnnnnnnnnnnnnnnnnnnnnnnnnnnnnnnnnnnnnnnnnnnnnnnnnnnnnnnnnnnnnnnnnnnnnnnnnnnnnnnnnnnnnnnnnnnnnnnnnnnnnnnnnnnnnnnnnnnnnnnnnnnnnnnnnnnnnnnnnnnnnnnnnnnnnnnnnnnnnnnnnnnnnnnnnnnnnnnnnnnnnnnnnnnnnnnnnnnnnnnnnnnnnnnnnnnnnnnnnnnnnnnnnnnnnnnnnnnnnnnnnnnnnnnnnnnnnnnnnnnnnnnnnnnnnnnnnnnnnnnnnnnnnnnnnnnnnnnnnnnnnnnnnnnnnnnnnnnnnnnnnnnnnnnnnnnnnnnnnnnnnnnnnnnnnnnnnnnnnnnnnnnnnnnnnnnnnnnnnnnnnnnnnnnnnnnnnnnnnnnnnnnnnnnnnnnnnnnnnnnnnnnnnnnnnnnnnnnnnnnnnnnnnnnnnnnnnnnnnnnnnnnnnnnnnnnnnnnnnnnnnnnnnnnnnnnnnnnnnnnnnnnnnnnnnnnnnnnnnnnnnnnnnnnnnnnnnnnnnnnnnnnnnnnnnnnnnnnnnnnnnnnnnnnnnnnnnnnnnnnnnnnnnnnnnnnnnnnnnnnnnnnnnnnnnnnnnnnnnnnnnnnnnnnnnnnnnnnnnnnnnnnnnnnnnnnnnnnnnnnnnnnnnnnnnnnnnnnnnnnnnnnnnnnnnnnnnnnnnnnnnnnnnnnnnnnnnnnnnnnnnnnnnnnnnnnnnnnnnnnnnnnnnnnnnnnnnnnnnnnnnnnnnnnnnnnnnnnnnnnnnnnnnnnnnnnnnnnnnnnnnnnnnnnnnnnnnnnnnnnnnnnnnnnnnnnnnnnnnnnnnnnnnnnnnnnnnnnnnnnnnnnnnnnnnnnnnnnnnnnnnnnnnnnnnnnnnnnnnnnnnnnnnnnnnnnnnnnnnnnnnnnnnnnnnnnnnnnnnnnnnnnnnnnnnnnnnnnnnnnnnnnnnnnnnnnnnnnnnnnnnnnnnnnnnnnnnnnnnnnnnnnnnnnnnnnnnnnnnnnnnnnnnnnnnnnnnnnnnnnnnnnnnnnnnnnnnnnnnnnnnnnnnnnnnnnnnnnnnnnnnnnnnnnnnnnnnnnnnnnnnnnnnnnnnnnnnnnnnnnnnnnnnnnnnnnnnnnnnnnnnnnnnnnnnnnnnnnnnnnnnnnnnnnnnnnnnnnnnnnnnnnnnnnnnnnnnnnnnnnnnnnnnnnnnnnnnnnnnnnnnnnnnnnnnnnnnnnnnnnnnnnnnnnnnnnnnnnnnnnnnnnnnnnnnnnnnnnnnnnnnnnnnnnnnnnnnnnnnnnnnnnnnnnnnnnnnnnnnnnnnnnnnnnnnnnnnnnnnnnnnnnnnnnnnnnnnnnnnnnnnnnnnnnnnnnnnnnnnnnnnnnnnnnnnnnnnnnnnnnnnnnnnnnnnnnnnnnnnnnnnnnnnnnnnnnnnnnnnnnnnnnnnnnnnnnnnnnnnnnnnnnnnnnnnnnnnnnnnnnnnnnnnnnnnnnnnnnnnnnnnnnnnnnnnnnnnnnnnnnnnnnnnnnnnnnnnnnnnnnnnnnnnnnnnnnnnnnnnnnnnnnnnnnnnnnnnnnnnnnnnnnnnnnnnnnnnnnnnnnnnnnnnnnnnnnnnnnnnnnnnnnnnnnnnnnnnnnnnnnnnnnnnnnnnnnnnnnnnnnnnnnnnnnnnnnnnnnnnnnnnnnnnnnnnnnnnnnnnnnnnnnnnnnnnnnnnnnnnnnnnnnnnnnnnnnnnnnnnnnnnnnnnnnnnnnnnnnnnnnnnnnnnnnnnnnnnnnnnnnnnnnnnnnnnnnnnnnnnnnnnnnnnnnnnnnnnnnnnnnnnnnnnnnnnnnnnnnnnnnnnnnnnnnnnnnnnnnnnnnnnnnnnnnnnnnnnnnnnnnnnnnnnnnnnnnnnnnnnnnnnnnnnnnnnnnnnnnnnnnnnnnnnnnnnnnnnnnnnnnnnnnnnnnnnnnnnnnnnnnnnnnnnnnnnnnnnnnnnnnnnnnnnnnnnnnnnnnnnnnnnnnnnnnnnnnnnnnnnnnnnnnnnnnnnnnnnnnnnnnnnnnnnnnnnnnnnnnnnnnnnnnnnnnnnnnnnnnnnnnnnnnnnnnnnnnnnnnnnnnnnnnnnnnnnnnnnnnnnnnnnnnnnnnnnnnnnnnnnnnnnnnnnnnnnnnnnnnnnnnnnnnnnnnnnnnnnnnnnnnnnnnnnnnnnnnnnnnnnnnnnnnnnnnnnnnnnnnnnnnnnnnnnnnnnnnnnnnnnnnnnnnnnnnnnnnnnnnnnnnnnnnnnnnnnnnnnnnnnnnnnnnnnnnnnnnnnnnnnnnnnnnnnnnnnnnnnnnnnnnnnnnnnnnnnnnnnnnnnnnnnnnnnnnnnnnnnnnnnnnnnnnnnnnnnnnnnnnnnnnnnnnnnnnnnnnnnnnnnnnnnnnnnnnnnnnnnnnnnnnnnnnnnnnnnnnnnnnnnnnnnnnnnnnnnnnnnnnnnnnnnnnnnnnnnnnnnnnnnnnnnnnnnnnnnnnnnnnnnnnnnnnnnnnnnnnnnnnnnnnnnnnnnnnnnnnnnnnnnnnnnnnnnnnnnnnnnnnnnnnnnnnnnnnnnnnnnnnnnnnnnnnnnnnnnnnnnnnnnnnnnnnnnnnnnnnnnnnnnnnnnnnnnnnnnnnnnnnnnnnnnnnnnnnnnnnnnnnnnnnnnnnnnnnnnnnnnnnnnnnnnnnnnnnnnnnnnnnnnnnnnnnnnnnnnnnnnnnnnnnnnnnnnnnnnnnnnnnnnnnnnnnnnnnnnnnnnnnnnnnnnnnnnnnnnnnnnnnnnnnnnnnnnnnnnnnnnnnnnnnnnnnnnnnnnnnnnnnnnnnnnnnnnnnnnnnnnnnnnnnnnnnnnnnnnnnnnnnnnnnnnnnnnnnnnnnnnnnnnnnnnnnnnnnnnnnnnnnnnnnnnnnnnnnnnnnnnnnnnnnnnnnnnnnnnnnnnnnnnnnnnnnnnnnnnnnnnnnnnnnnnnnnnnnnnnnnnnnnnnnnnnnnnnnnnnnnnnnnnnnnnnnnnnnnnnnnnnnnnnnnnnnnnnnnnnnnnnnnnnnnnnnnnnnnnnnnnnnnnnnnnnnnnnnnnnnnnnnnnnnnnnnnnnnnnnnnnnnnnnnnnnnnnnnnnnnnnnnnnnnnnnnnnnnnnnnnnnnnnnnnnnnnnnnnnnnnnnnnnnnnnnnnnnnnnnnnnnnnnnnnnnnnnnnnnnnnnnnnnnnnnnnnnnnnnnnnnnnnnnnnnnnnnnnnnnnnnnnnnnnnnnnnnnnnnnnnnnnnnnnnnnnnnnnnnnnnnnnnnnnngtggcaggggtcctgccgctcctgggccctcccccacgggagcccagaggccttatacagtttcctcttgggccagggatgtgggcaggggtgagcagtgttggtggtctcttccgctctgcagcctcaggagtgcccacctgaccaggcggttgggtctctttctcaccgggtctgggagcagagagctgctgcgggccgggatctgctgcaagttttaattttttttttttttgattcttttttttcggagctggggaccgaacccagggccttgcgcttcctaggtaagcgctctaccactgagctaaatccccagccccgcaagttttaatttttaagacattctaatttttattaatattgttaggataaaatatatacatatacatatatcatacaacacacacagacatacacacatatgtattgcatgtttacaatcagttttaggtatcttaattgaatccactaagcctttgaattttgacaaactgatataatatattgttacttaatatttcttttctttcctcctcctcctcctcctcttcctcttcttcatcttcttcatcttcttcttcttccccttcttcttcttcttcttcttcttcttcttcttcttcttcttcttcttcttcttcttcttcttcttcttcttcttcttcttctagacagcctttcataatgtaatcatggccggcctgaacctgatatgtagtccatatagcttctaccttgcagcaggctccttagagttccgacaagagttttgaaattgcctgcatgtggcactggtcttatactatatttatttttcaatattatctaacacctccattattttcaccattccttagtattgtccaccttagactaaagaagacagtgttttcttcttttcaaatttagtttgcttttgagattataactacatcatttctttcctcaaggattgactagttgctgctaacaactctaacagcactgattcatcatgagaataatgatataccaatatgtatagtcaatgtggcatatatttgacatattgaagtttaatggctgatatcttttggactttaactaattgtctattgctaatgaaacctaggaaattctgatccttgagattatttttaaagtgcacataaggtatattcaggtgaaaataaagaagacaagcatagcagcccccagaaggccatgtggagaaagataaaaaaaaaaaaaaaccagcaaagtatctacagcaagatgtgggcctgagggtcttctgtgcagctcagttcaaccaaaagtatatcacagcagttactactgtttatgtatgcattcggaagacgggagggacctagtcaatatggtcaatttcaaggacttcctgaagcttttgaattgtttacttcctgagcttccttagaggatgggattttttagttccctttagagcaatggttctcaacctgtgaccccctctgaagtcaaacaaacctttcacatgggttgcctaaaaccattgtaaaacacagatattattattaataatagttgcaaaattacagttatgaaatagcaacaaaaataattttatggttatgggatcgccacacaagaggaatggtattaaaggaccaaagcattagggaggttgaaaaccattgctttatctcatcctatttttatgggtgcttctctctgagacggagtcttttatcttaaagaaaattgctattcaacaattgaagagaggtattaggtcagtaagagtatggtatggtcataggccagcacaattcctgcatatgcttgtcataaataactcacctcttcttcagattgactgggaaaagacaaaacatttcaaagtgatcttttaaaagtttccttcgttataaagaaggaaaaatggattaaaaggatggaagaaaatgctttgaaagaccagttactactgccatagtcttagagtagtgtatttgagagaactgtgttaaatgtggttgctaggacttttgaaggtttttttctcccgtttttgtttttgccttttgtttttatggtttgcttgttttgttatttgtgtgtgtgtgtgtgtgtgtgtgtgtgtgtgtgtgtgtgtgtgtgtgttgtgtgtttgtgtgtatggagaaggcaccatgacttttcaaagataaaatgaaaagtgaatctaatggatttccttgaaaagctgtcttgaaaattactgtcagtaatccaaagttgtattattttgaagattattcaatgaaaatattaatctacaaccacgtgtctatttttattttcacaagagtctgagattgttactggctgtcgtttatttcaatttgtcatcatgttcaatataattaatcatatacttttaatttcttccaaaaatgaaaatttgaaatgacagatatatgatcaagagggcagtcaggccaaaacaatgtttgtttggtcactgattttgactgattgacctaatgggaacaaaacactgtcattataaaagtatgttactcagcagatttcctcttatagtaaacactatacaattactcttttgcatttagaaatttcttgcctgccaccacgagttgaaaatggagatggtatatatctgaaaccagtttacaaggagaatgaaagattccaatataaatgtaagcaaggttttgtgtacaaagaaagaggggatgctgtctgcacgggttctggatggaatcctcagccttcctgtgaaggtgacattattcttattttctacgtcttttattatataagaagtagaacagtgaatggaaaagaaagatggtgtcacaaatccatgtttagctgattgcattgagtctaaccatctgttttcatggtgtttatgtatcctagtcagagaagtatctcagtagtcctttggcattaaacctctgcacaagattaactccaggtgtcctcctaaatagaccatttatccactaaaggatcaaactataacccatgatgtagctattttgtattgtcttgtgcttaagaggaacttttcaaacaatcattccagtttcaggtgaatccagttttccatggaagcattaggattcaatagaatagtcatgccacaccaaataacagagcagagcagaatgcctgttctgtactgaattcacctaaagctgaaatgatttttacctagttaaaatctcttccttaacctagatttgttttcaaactgagaaatatatttggttccctaaatgtgcttctacagatgctacatagccttgcttcttttgaaccctaggaaagaggagaggagtgtgagtagagggagagaatagaggaagggaagaaaggaagcagggaatgaaaaagactctccattaaagttcattttgaccatttctcaaacacaaagtcaagtatgaaaagtatagttctgtgttcttgggggtctttttcttcagggaaataggtgacagagggtactctcatctgatagtaaataagcatttgatgatatgaataaagagacctgcatcttaactcatataggcatgcaaatctctaacaatggacttcattttactgaagaaaactttatactcctatatgaaaagtagtttcttattaatgaaaatagtgcatcactctgtacctcagctgatatgtttggccaatgcattgtctttgttttcctggagcagaaaaatagcttacttgtgttgatgtacaattatctggaaattatcagaacactttaatctctctgacaccatatagtggaatacattatttgctgcagctgactttacaagaatcttagactctataagacaccaaaattaaaataagataatataaaaataaataaactttgttccacctgatcataatgtgaacagggggtttaaaacaacttcccagagcatttggatctctagtatatagtagacagtctctaatgacaagcaggaatgatgaaaaataccacaatcttctgaacaatttattttgatgcatctgtttcctgtacagagtagattttgtaaaattgactttccaatgtaagagaactaaacttgaaatatcccattccaaatgtctctactaaataatttgaaataagaaaactgtacatttgggaaaatgtacaagggaaaaaagacactatgcatttgaaaaattaactacatatagtcaatcagacattatcaggggtttatgttggcagcttagggtaatctccaaaagtctttttgttaataagttttacaaagttcttcccatactgtttgcttgtcctcttaaattcttggacatattgttgttgtttgatatcttatagctgtaccttaaaaagatactgagtaaagctgcaatattaagaaaacctaagtagaaaagcataaactacaatggtcctatgaaaacatgacaagcagagtgctgtgaagagaaaaacgatcaaaggaacacaatgttgattcaaaaattgttgttaagtggcataaaagttaggagacatacttgatttgagtagttatcttagggtgaagagacaccatgaccaaaggaatatttaattagggctggcttacaagttcagaggttcagtatactatcgtcaagggggaaagcttggcagcatccaagcaagcatggctttgaagaaggtactgagagttctacatcttgatccaaaggcagtcaggagaagactggcaaagcccaccctaacagttatacatttccttcaacaaggccacacctattccatcaaggacacacttcctaatagtgtcactccctggtccaagtatattcaaaccatgacagtagtcagatattactttagctaagtttttactactatatatgtatattacctgtcttcatgagggaccccagcaactgaagcaaggactgtcgctgactttgttgcctgtctgtggatcctatcccccttgactgggctgccttgtctggcctcagtgagagaggatgtgcctagttttacagtgacttgatataccagaatgggctggtaaccagggggccctccccttttcagaggagaaggggtagaagggatggggcaaggggctatatgtggagagactgaaaggaaagtagagggcttcaatagggataaaatttataaaaaaaagaaatacatatatactgtggcacaaatttaataccagtagaaaggttactgccatactttcaagggctaagtgtacacattagcattatatatggaaaggcaaaaattcaaataacacttaaaaccaaagaattatgtgccagattgagtataagaatgatgaataaatctccagactcttatcataatatttttgttttataagttaaaatattagatttagatggaaaagtatgaatggaggaaagttaatgatagagattgccattttaaaaactggattgccttcaaattctgtatatgagcatgattcatttacctatatggattttgattaaaactacagaattattagcataagagccagactttaattatggaggttatcttgagtgccataaaggacagaagaaaaaagaacactagtgaagaatacatgctcataaaaaccaactataaggcaaaaaagttatttgtgcagaaactgtagctacttaaaaataattttttaaatgtagcaatggtatcaattagaagatctgggttaagatgatttaaggcacataagacataaaatgtacatttgagaaatggcttggtgtttgtgaaggttagattcatgattttgaaagtcaaaaattacactatgtttcttccttgttcagtagattttcccaaataagtcagaggacatgttcaattcaaagagaaagaggtgtaaaatcttcatgaatatttagaattaaggacctgtgaatattaataaataggctcaaatgagaatcaaggccagcaatttcaatgaaagaaatagaaactggatggaaacatgtttcttgcactgaaggtctgtatgatgaagttattatcatctttagaagcataaggtactatatgggacagcatcaagagagaattagtaccagagaggcacacatacaccaggaggagagagaagaagtctgactgatatgcctagcctatgaagatgcattcttttcaatgtctattatatagttatcagtacaaataactggtgtctgccatttagttttaatattcttaacctaaatgagattaaatatttctcattacttatatctgattcttttcagaaatgacatgtttgactccatatattccaaatggtatctacacacctcacaggattaaacacagaattgatgatgaaatcagatatgaatgtaaaaatggcttctatcctgcaacccgatcacctgtttcaaagtgtacaattactggctggatccctgctccaagatgtagctgtaagcttcacttatatctttaatctccatgatcctgaaattagactaataagcatgcatagaagaaaatatagtaatagcaaatatttaattttttatctatgtacaacacttaaaaatattctacttttaaaagtcaagaaaaattaacataatattatattttaatattaaaatttaaaattgcaagtaatatttaaaatacattatagaaaactaaaatttttaatttacttctacttaaatatataggcatctgtacattttttttcttttttttcatttattttttttttattaacttgagtatttcttatttacatttcgagtgctattccctttcccggtttccgggccaacatcaccctaacccctggttgcttggcattgttgttcataagaggtctcgagccccttcaagcttgccagttctttctctgattccttcaacgggggtcccgttctcagttcagtggtttgctgcaggcatttgcctctgtatttgctgtattctggctgtgtctctcaggagagatctatatccggctcttgtctgcctgcacttctttgcttcttgtctaattggatggttgtatatgtatgggccacatgtggggcaggctctgaatgggtgttccttctgtgtctgttttaatctttgcctctctattccctgccaagggtattcttgttccccttttaaagaaggagtgaagcattcacattttgatcatccgtcttgagtttcatttgttctaggcatctagggtaattcaagcatttgggctaatagccacttatcaatgagtgcataccatgtgtgttttctgtgattgggttacctcactcaggatgatattttccagttccctccatttgtctatgaatttcataaagtcattgtttttgatagctgagtaatattccattgtgtagatgtaccacattttctgtatccattcctctgttgaagggcatctgggttctttccagcttctggctattataaataaggctgctatgaacatagtggagcacgtgtcttttttatatgttggggcatcttttgggtatatgcccaagagaggtatagctggatcctcaggcagttcaatgtccaattttctgaggaacctccagattgatttccagaatggttgtaccagtctgcaatcccaccatcaatgcaggagtattcctctttctccacatccttgccatcatttgctgtcacctgagtttttgatcttagccattctcactggagtgaggtgaaatctcagggttgttttgatttgcatttcccttatgactaaagatgttgaacatttctttaggtgtttctcagccattcggcattcctcagctgtgaattctttgtttagctctgaaccccattttttaatagggttatttgtctccctgcggtctaacttcttgagttctttgtatattttggatataagccctctatctgttgtaggattggtaaagatcttttcccaatctgttggttgtcgttttgtcctaaccacagtgtcctttgccttacagaagctttgcagttttatgtgatcccattggttgattcttgatcttagagcataagccattggtgttttgttcaggaaattttttccagtgcgcatgtgttcgagattcttcccaactttttcttctattaggtttgagtgtatctggtttgatgtggaggtccttgatccacttggacttaagcttgtacagagtgataagcatggatcgatctgcattcttctacatgttgacctccagttgaaccagcaccgtttgctgaaaaggctatcttttttccattggatggttttggctcctatgtcaaaaattaagtgcccataggtgtgtgggttcatttctgggtcttcaattctattccattggtctatctgtctgtctctgtaccaataccatgctgtttttatcactattgctctgtaatactgcttgagttcagggatagtgattccccctgaagtccttttattgttgaggatagctttagctatcctgggttttttgttattccagatgaatttgcaaattgttctgtctaactctttgaagaattggattggtattttgatggggattgcattgaatctatagattgcttttggtaaaatggccgtttttactatattaatcctgccaacccatgagcatgggagatctttccatcttctgaggtcttcttcaatttctttcttcagagtcttgaagttcttattgcacagatcttttacttgtttggttaaagtcacactgaggtactttatattatttgggtctattatgaagggtgtcatttccctagtttctttctcggcttgtttctcttttgtgtagaggaaggctactgatttatatgagttaattttatacccagccactttgctgaagttgtttatcagctttagtagttctctggtggaacttttgggatcacttaaatatatatcatatcatctgcacatagtgatattttgacttcttcttttccaatctgtgtccctttgacctccttttgttgtctgattgctctggctagaacttcaagaactatattgaataagtagtgagagagtgggcagctttgtctagtccctgattttagtgggattgcttcacgtttctctccatttagtttaatgttagcaactggtttgctgtatatggcttttactgtatttaggtatgggccttgaattcctattctttccaggacttttatcatgaaggggtgttgaattttgtcaaatgctttctcagcatctaatgaaatgatcatgtggttttgttctttcactttgtttatatattggattacgttgataattttccgtatattaaaccatccctgcatgcctgggatgaagcctacttgatcatggtggatgattgttttgatgtgcttttggattcggtttgccagaattttttgagtatttttgcattgatatttataagggaaattggtctgaagttctctttctttgttgggtctttgggtggtttaggtataagaataattgtggcttcatagaacgaattcagtagcactccatttgtttcaattttgtggaacaatttggatagcatatgaggtcttctatgaaggtctgatagaattctgcactaaacccgtctggacctgtgctctttttggttgggagacctttaatgactgcttctatttccttaggagttatggggttgtttaactggtttatctgttcctgatttaacttcggtacctggtatctgtctaggaaattgtccatttcctgcagattttcaagttttgttgaatatatgcttttatagtaagatctgatgattttttgtatttcctctgaatctgtagttaagtctcctttttcatttctgattttgttaatttggacacactctctgtgtcctctcattagtctggctaatggtttatctatcttgttgattttctcaaaaaaccaacttttggttctgttgattctttctatggtcctttttgtttctactttgttgatttcagctctgagtttgattatttcctgccttctactcctcctgggtgtatttgcttctttttgttctagagcttttaggtgtgctgtcaagctgcttacatatgctctttcctgtttctttctgcaggcactcagagctatgagttttcctcttagctcagctttcattgtgtcccataaggttgggtatgttgtaccttcattttcattaaattctaaaaagtctttaatttctttctttatttcttccttgaccaggttatcgttgagtagagcaatgtgcaacttccacatatatgtgggcgtttttcccttattgttattgaagacagctttaggccgttgcggtctgatagcacgcatgggattatttctatctttctgtacctgttgaggcccgttttttgacccgtttttaaatggtcaattttggagaaagtaccatgaggagctgagaagaatgtatatccttttgctttaggatagaatgttctataaatatctgttaagtccatttggctcatgacttttcatagtctgtctacgtctctgtttaatttctgtttccatgatctgtccattgatgagagtggggtgttgaaatctcctactattattgtgtgaggtgcaatgtgtgttttgagctttactaaggtttcttttacgttttaggtgcccttgtatttggggcatatatgtaggattgagagttcatcttagtggatttttcctttgttgaatatgaagtgtccttccttatcttttttgatgacttttagttggaaattgattttatttgatattagaatggctactccagcttgcttcttccgaccatttgcttgcaaagtttttttccagcctttcactctgaggtaatgtctgtctttgtctctgaggtgtgtttcccgtaggcagcagaatgcagggtcctcgttgcgtatccagtttgttaatctatgtctttttattggggagttgaggccattgatgttgagagatattaagcaatagtgattattgcttcctgttatattcatattttgatatgaggttatgtttgtgtgcttttcttctctttgttttgttgccaagacaattagtttcttgcttcttctagtgtagagtttgcctccttatgttgggctttaccatttattattctttgtagtgctggatatgtagaaagatattgtgtaaatttggttttgtcgtggaatatcttggtttctccatctatgttaattgagtgttttgcaggatacagtaacctgggctggcatttgtgttctcttagggtctgtatgacatctgtccaggatcttctgactttcatagtctctggcgaaaagtctggtgtgattctgataggtctccttttatatgttacttgacctttttcccttactgcttttaatattctttctttattttgtgcgtttggtgttttgactattatgtgacggggggtgtttcttttctggtccaatctatttggagttctgtaggcttcttgtatgcctatgggtatctctttctttaggttagggaagttttcttctatgattttgttgaagatatttactggtcctttgagctgggagtcttcactctcttctatacctattatccttaggtttgatcttctcattgagtcctggatttcctgtatgttttggaccagtaactttttctgctttacattatctttgacagttgagtcgatgatttctatggaatcttctgctcctgagattctctcttctatctcttgtattctgttggtgaagctcgtatctacggctccttgtctcttcttttgtttttctatatccagggttgtttccatgtgttctttcttgattgcttctatttccatttttaattccttcaactgtttgactgcgttttcctggaattctttcagggatttttgtgattcctctctgtatgcttctacttggttatttatgttttcctccatttctctaaaggagttcttcacgtctttcttgaagtcctccagcatcatgatcaaataagattttgaaactagatcttccttttctggtgtgtttggatattccatgtttgctttggtgggagaattgggctctgatgatgccatgtggtcttggtttctgttgcttggattcctgcgtttgcctctcgccatccgattatctctagtgttactttgttctgctatttctgacagtggctagactgtcctataagcctgtgtgtcaggggtgctgtagacctgttttcctgttttctttcagccagttatgggaacagagtgttctgctttcgggcgtgtagtttttcctctctacaggtcttcagctgttcctgtgggcctgtgtcttgagttcaccaggcagctttcttgcagcagaaaatttggtcttacctgtggtcccgaggctcaggtttgctcgtggggtgctgtccaggggctctctgcagcggcagcaaccaggaagatctgcgccgccctttacaggagtttccgtgcaccagggttccagatggcgtttggtgttttcctctggaatcagtaatgtgggcagagtgcagtctcttctggtttcccaggcatgtctgcctctctgaaggtttagctctccctcccatgggatttgggtgcagagaactgtttatctggtcggttccttcaggttctggtggtgtcttagacgcaggggacctgctgctgctgtgcccttatccaagggaacgcagaggccgtatacagtttcctcttgggccagggatgtgggttaagggtgggcagcgttggtggtctcttctgctctgcagtctcaggagtgcccacctgtccaggtggtgaggtctctctcccatggggtttgggagcagcgagctgctgcgggcagggatccgcgggttttcatctgtacactttttaactaaacattttctaagaattgtatgaaattaataggtaagagacgcaggggacctgctgctgctgtgcccttatccaagggaacgcagaggccgtatacagtttcctcttgggccagggatgtgggttaagggtgggcagcgttggtggtctcttctgctctgcagtctcaggagtgcccacctgtccaggtggtgaggtctctctcccatggggtttgggagcagcgagctgctgcgggcagggatccgcgggttttcatctgtacactttttaactaaacattttctaagaattgtatgaaattaataggtaagaatattgtcaggtaagaactgattttacttatttatttacatcatagtaaatatccttcaatagtatttgcctcatagcaaacctttgtcatccctccatttttgttagccacatttgaagataacttggctgctggctgcatgagtgtggtgctgtcagacattgtcttggctcttagtcatcaggagactttgctgggctgtaggccatatgttcaacataccacattcactaggatttggcaagagggttcaattccttatcagataagcctgtggatagattgattcacaaaattgattcttgccttagagttactgatcaaagagacattggggggcctagaatccatccataacctacctataccatacaatgtttttgctatggctgtttcttgtatactgggttcaatatgcatatgaagaaggaaattatgtttatctgtagagagttgctttgaatgatgtcggtggcttctcaacacatgcataccacagtgttatttgagtcaagaatatttaattcctggaatattccattcttttcagatttttgtctatctacatccatatatttttcttttatctaacagtctatgttaaatgtttatcatacgtaaccctgatatcccctaaggaataaagtgtatgacagataagcagccaaggatctcttcctactcatctttctgttgtgatgttaatattactgaattaactacttagaagaagaatttattttgttttgctgacttgaattcatggtcaagttgttctgtcattttcatcctgttactaggaggttatttatgttagggaatgagtggtaagtctaagctgcttggcttatgaccaccagcaagtagagatataagagaatgaccaagatctcaatatccccttcaaaggcatagtcccaatgacctaatttatttcactgtgtccagaaattctgaaatttataaccttcctaatagcaccagcaatgacaaaccaagcttttaactaaggtgaaattctaggaaatctataatatccaactcaaaagaatgaaagaagctatttacactaagaaatagtattgataaatatagtaattgtataaaaattgaatttttaaaaatattaaaatttagatttcttacaaattatttttcttacttttattggtcctatttatttatttattatttgtttttgtcattaggttgttttttataaaatttattctctcatatattacatcctgattgcagtttcttttcccttaatgtcccaactcctccatcccctcaacctcattcctccccatccactcctcctttatttcccttcagaaaatagggggaccctcagggaaatcaactgattattccatatcagatttcaatgtgtcagtacaaggcaccccagtatgaggacaagggtccccaaaataggcaaaagaatcaggaacaactgcaactctctctgttaggaattccacaaaacaccaggcttcacaactataacaaatatacagagggtcaaggttagatccaggctctctgattgtcagttgaatctcagtaaaaccctgagtccaggtgagttgactctgtgagttttcttgtggtgtccttggctgctctgctcctataatctttcttctctaacttcaacaggattccccaaactctaaactaaaggtcagtggaaaagtaccttttcttctcctgagtaattgcttcaaagcctctgctaacctaggcctagttctttaatctttctctagcctctgtataatcttatctaggtcaagaatgtttacagtttttgaaacttacttgtgaataagatcacatcgtcctatttctttctgaactctggctggcttgttcagctcaactgttctggcttaaactcctctgcaaactgtttcaaactgacttctttttcagcctttgacttggtgctatgcttggcctcagattaaccctggcaatctgttttaatcctccgactccttcttattctctggcttctcttacctttacttgtgactagcttgttctctctctgcagcttgtactggtaaaactgcccctccctcacctctttctctgtgctgccctctcgtaaagaggtagcctctttctctctgttctcatgagagttgggcatatcttattctgttaaatctttctctgatttaacatctctttcaaacaagggtgattccttctacaaaataactttaccttcattgttttggattaaagccctttgtagtgttactaaggacttgtctgtattccagccagaaggattaaaggtatatgctgaggctgcgccacaccacagctaaaaacaggtttttcttgtaaacaacacaatcttggatttcacagtgttaccaaaagtcctaaaacagtttgaatctctgcatctgtttctattagttgtggagtagagcctctcctatgatgactgggctaggcaccaatctataagtacagcagagtatcattaggcatcattgaattgacttttttttctttgccagtcatggttggttctattctaggtctctgggccgtacagcctctggtttctggtcctcaagtcagtgtcaggcatgggtttcaagctgtacctgtcattagttagtcactttcacaatttctgtgccaccttcaccccagcacatcatacaggtgagacaaattgtaggttgaaggttttatgtctggtttggtgtcccaaaacctttgtagggttatgtccctgttttcattactgactttgttagtttttatatttaatctgtctttcagttagtttggctaagggtttgtctatcctgtagattttctcaaaagaccaactcttcttttcatagattctttgtattgttctctttgtttctattttattgatcttagccttataatgtttcttagccccaagttggtttatttcctgctctctactcctcttccagagctttcaggtgtgctgttaagtcacgagtataagatctctctaatttctttatgaaggcacttagtgctatgtagtttcttcttaacaccacttttattgtgtcccatacgtttggtatgttgtgccttcattttcattgaatactagaagccttaaattctttatttcttccttgacccagtggtcgttcagtaaagaactgttcagtttccatgagtttatggagtttatgttattgttcaagctcagctttaatccatgtattctgaaaaaatacagggggttatttcatttttcttgtatctgttgagactcgctttgtgacggagtatatggtcagttttagataaagtactgtgagatgttgagacaaaggtgtattcttttgtctttgggtgaaatgttttatagatttctgttaagtccatttgattcataatgtcttccagttccatttttctgttccttttttgtttggatgacatgtccattggtaagagtggggtatggaagtcttccactattaatgtatggtgttcaagatatgttatgaaatatttttgttagttagtttgttttatgatttttatgattgcggtttcccttgcatttggggcagatgttcagaactgagaggttatactcatgaaatattctttttgattagtatgacgtttcctttgtaccactaatgattaattggtttgaataatattttgttaaatattggaatggctacatgatcttgattctttggtccatttgctagggaaatcttttctagccttttattattaagtaatatccacttctgatgttgaggtatatttcctgtatgcagaagaagggtggatactgttctcacatccattttgtgaaacctgtgccatttttattggagaattgaatccattgatactgagagctatcaatgactaatgattgttcattcctattattttgatggtggtggtggcagtgtttgtgtttgagtgtgtgtgtgtgtgtgtgtgtgtgtgtgtgtgtatgtctttttttgctcatatgagattgtttattgcctgtggtgtagatgatctttttgtgttagggtacaagttatttatttcttgggtgtagttgatctccttgggttggaattttctttctagtaattttttttgtagggcttggctgtggatagatattgtttaaacttggctttctcatggtatatcgtgttttctcctactcttattgagtattttgctgactacttcagtcaggatgcaactgtgattgttcagaatgcccaggcccttcttgctttcagagttttcactaagaagtcaactatattctgatagctttgcctttgtatttcacttgcttttttcctttcacatctttcactaatcattatttgttttgaatatttagtattttgattactgttttgacaggacttcattttctttttccatctagttggtgttctataagcttcttgtgcttttatacgcatctccttctttaggacctttttcttttattattttgttgaaaatattttctgggccttctaaaatttattccttgtaagtttcacaagcacctgatcccattcttctttccattcttccatatctactcttttcccttgtaaatgttcccccaaaacaaaacaaataaaaacaaaccaacaaacaaatagacatcttgtcaaggtagctataggcattgcagtgtgtcacacagggacaaaaatctcttttgtccaaacagctttacttgcagatattcatcgcatttagtcatttctttggttcaagatctctggcttctagtacaccacaatacattctgaatattttatctttcacattgctccaactcgataaacaacacatcatccatatctgtcctttccccagaatcataattttgagtgtttttgtatgatgcatttggcttaactcaggaaatatgtggaccacttgaattggagctgtattttcgaacctgatttactcacgagtgggtatatacctgaaagcactgactccctatgtttctgaatctattagcgtaaaatagttccaaggtgagggccaaggttccctatgatcttactacagtcatgcctggatatgagggcccattcttaagaggtgtctgtaattgttgagagtttgtgattttaatgataatgtttttgttcagaagatatcatagtcttaatcactctagctcttagaacctatgtgctccttcattcacaggttgcttgtaggggatagtgctcctgttttgtttaacacttcacaatacactcactatttctagtaccttgtgtattactacatctatagttttattataatttaccagaaaaaagagtcttctctgatgttgacagtgttattagctatgaatataaacatagttacttataaggttgctcagtgttaagtcaatgtattttaatagcagaattaatatgtgtgtctgcactcagatcttatgacatccttgccatgggcttttaagtaggtttacaaatacaagcctgggatctgtgtagcgcaatgagtcacaaacccaactatgtttgagtttccccaatgtagatttacccaaatatatctgggctgcttgtaacttaaatatatatgaatttcgtttattctacactgaactttctgatacttcctggataagataaaaatgattaatctctctgtaatgtcattaaataactttttctacttaaaatctttagtactcactcctaagggatgtttaattactcaccactttcatcaaatcttttactatttgggagaaaatgcattgtaaaatgataactggcacaattcagaagatggtgattgtgaatctgtgttagaagtgattctagaaattaatcttttgtgtcatgttgaagatgtagtaggatgagatttatcaataaaaattagaagatcttgggattgaagatcagtaaaaactggaatatcttgcgctgtgttcataatatttagaacagttgtaaaactggtcaatatattgatcagcagtctgagtagagtgcatcaacactgtgatgtatggtccaggaatcactgctgatgcagccacgacctgcatctggaaagtgtaagatgttaaacaaagctcacttaggtactgaccacctcaggtgtctgttactttaaggagtattatgtttgcttcaagaaccatgtataacggagtaaacctgtgcccactggagaatgaagaataggtaaaagtctgaggtctgtggtaataatgatactcctactctgaaccatgctttctttcattacttttcaaaacaaaatctcagtgagctaatttgacttattgatgtcctatgagaagtgtgattcttaaaattgttaaagaagaacaatttttaaaccatgtaaaaatgtgtaaaaaaactcttgaaatatttaataaaacaaaaactaaaatgaatgaggaagcttgaggaaatttgtttgattttttatgtatttgttgaaataacttttaatgtattgcatgaggttccttgaagcagaatcatacttaatataaaagggatattattctcatactaaagtacaaatgataaatagtaatcacaaataattacatgtaataaagtaatcatatattacatataaacttaatataatgaacaatatggcatttcaatacaaaggtacaaaaatagctccatatcgttccatgttcatactatattttagtttcagtgaaaattataaataagaaattatattgaatattaacaagtatctccaatccaattatctggtggagtatcagctacaacttgacttcatgttgaaagacatcctcacaaaccactgttgtcttttgttttattttcttatcccacacattcactgttctgtcattctgttattttgattagtttaaagtaatttactgatcaagagttttttttcctctgatatgagtgttttatggttgttttattttattatttttttctttcaagtgaaaccttgtgattttccacaattcaaacatggacgtctgtattatgaagaaagccggagaccctacttcccagtacctataggaaaggagtacagctattactgtgacaacgggtttacaacgccttcacagtcatactgggactaccttcgttgcacagtaaatgggtgggagcctgaagttccatgcctcagtaagccaatgcctttatagttaactatgttgattcttttaaagagagagcacatacataattaagttattcataacaaaaataagaccaacaaaagaatttgtgagcaaaatggctagtttctgttatgaaatgtttcttcatgaaacatgcaatagggactatggaaatatctttatcacttgcatattttatttttacaaacgaaagataaatgctattctcttaaatgtttgttattaattttatttttgaatgatgtgcatactcattaaacagttttaaagataacatttatcttagtttatttttaaacaaattaaagattttatttttttaatttttaattattatgtttcttagggcaatgtattttccattatgtggaatatggagaatctttatactggcaaagaagatatatagagggtcagtctgcaaaagtccagtgtcacagtggctatagtcttccaaatggtcaagatacaatattatgtacagaaaatggctggtcccctcctcccaaatgcgtccgtatcagtaagtaactaatacttagatcgcaagaagatcgtgactctctgtcccatctgtatttgtttttattggctaatttttatgtacatttcaaatgttattctttttcctggtttcccatacataagccccctatccaatccccctcacacttctttgagggtgttccccttccccaagaacccatcctttcccacttccctaccctgacattcccctactaatacttagatcgcaagaagatcgtgactctctgtcccatctgtatttgtttttattggctaatttttatgtacatttcaaatgttattctttttcctggtttcccatacataagccccctatccaatccccctcacacttctttgagggtgttccccttccccaagaacccatcctttcccacttccctaccctgacattcccctacactggagggcccagccttagcaaaaccaaggacttctcccctcattggtgcccaacaaagccatccttgttatatacagctacatatgcatctggagccatgagtctgtccaaatgtcctctttgggcagttgtttagaccttgggaactctggttggttggtagtgttgttcttatggggttttaagacccttcagctccttcaatccttcctctaattcctccagtgaggaccccattctcagttcaatggttggctgctagcattctcctctgtatttgtcacactctggttgagcctctcaggagacaactatatcatgttcctgtcagcatgcacttcttggctccatcaatattgtctaggtttagtatgcatgtgtgtttatatatatatatatgtatatatacaggtgtagtatgcataagtatatatgtatatgtctatgtttatttgttggatccccaggtggatcaggctctgaatgtccattccttcagtgtctgctccaaacttggtctcaatatctcttcctacaaattttcttctattagttcgagagtatctagcttcatgtggaggttcttgactaactttgacttaaggatttttgcagggtgatgaaaatgggtcgatttgcgttcttctacatgctgacctccaggataaccagcaccatctggtgattccactgaatgattttagttcctttgtcaaatattaagtgaccacaggtgtgtgagttcatttttgggtcttcaattctactccaatgatctacttgcttgtctctgtatcattattgctctgtaaaacagcttgaggtcatggatgagattaccaaagaaccttttttattattgaggatagttttcactatcttggatttttttgttagtccaaatgaatttgcaaattgctctttctatgtctatgaagaatttagttgggattttgatagggattgcattgaatttgtagattgcttttggcaaaatggccatttttactgtattaatccccccaaaccacaagcatgggaaggttctccatcttctgagatctttgatttctttcttcagagacttgaagtaattgtaagatctttcacttgtttgagtagagtcacaacaaggtattgtacgtaacttgtgaccattgtgaagggtgtcatttccctaatttctttttcagcctggttatcctttgagtagaggaagggtactaatttatttgagttaaatttatacccagccaatttgctgaagttatcatgcttagtagtttgctgatggaacttttggggtcacttaaggatagtattatatcatctgcaaatagtgatattttgactcttcctttccaatttgtatcccattgaccttttgttgtttgattgctctgaccaaaactttgagtactatattgaataagtagggagagagtgggcagccttgtctagtccctgattttagtgggattgcttcaagtttctctccatatagtttgatgttggctactggtttgctgtatattgcttttaatatgtttgggtatcggccttgaattcctgatctttctacggcttctatcatgaaggggtgttgaattttgtcaaatgctttctcagcatctaatgaaatgatcacatggtttttttctttgagtttgttaatatagaggattacgttgatgaatttctgtattttgaaccatccctgcatccctgagatgatgcctacttgatcatgagggacgattattttgatgtgttcttggattctattgacaagaattttattgagtatttttgcatcaatattcataagggaaattggtctgaagttgtctttctttgttgggtctttctgtggtttaggtattagtgtaattgtgacttcatagaaggaattcggtagtgccctgtttctcttttgtggaatagcttggaaagtgtgaatatgaggtcttctatgaaggtctgatagaattctgcacctaactcatctggtcctgggccctttttttcttaggagacctttaataactgcttctatttctttaggagttatggggttgtttagatggtttatctgttcctgatttaacattatacatggtatttgtctagaaaattgtccatttcctcgatattgaatataggcttttgtagtaggatctgatgatttttttaatttcctcagattctttcgttatgtctccattttcatcttgaattttgttaattggaaatactctctgtgacctctggtttatctggctaagggtttatctatctggttgattttctcaaagaactatctcctggttttgttgattcttttttttttcttccttttattgaatatatttttttcagagggaaaatgtttattagtttcatagttttatacctttcagcttattttaacttggtctctggagcatttggaagactagctgcttacatcagagcagtgctgaaatagagacaactataaatccagagacaaacatagccttcaaagttatttagccctacttctaaacagatagtctataatatttattctcaataactgtaaagaaacttatattctccccctcccacaaaacatcactgaaagacgaaagaattggttccatgtatgaccttcttgtttgaccagtggcttcattagggtcatttacaggagcatgccaagaagttacttaaaagaatagtaatgattcaactgaagtttcattaaagatatgtctcatcacagaatgcttttcaattcataaatcacctctagaatgctatccacaccatcgagaatcctgtgatctcctctcaatctataataacatattggcttggggagggtttatgaaagaatagtggggtgtgtgtgtgtgtgagtgtgtgtgtgtgtgtgtgtgtgagacaaaaaaattgatttaaagttaacttctaagtcccagctaacaaccaatgttctgatcagagagctttcagaatagactctattttctctatattctgctccaaacaactttcctgatggctgtctttctataagtagtttgctttgcatgacacagctttctcttactattcctttttttttttaacttaagtatttcttatttacaattcgagtgttattccttttcccggtttctgggccgacatcccctaacccctccccctccccttctttatgagtgttcccctccccatcctccccccattgctgccctccccccaacaatcacgtttgctgggggttcagtcttagcagtccccttccacaggtgatcttactaggatattcattgctacctatgaggtcagagtccagggtcagtccatgtagagtctttaggtagtggcttagtccctggaagctctggttgcttggcattgttgtacatatggggtctcgagccccttcaaggtcttccacttctttctctgattgcttcaacgggggtcctattctccattcagtggtttgctgctggcattcacctctgttttagctgtattctggctgtgtgtctctcaggagagatctacatccggctcctgtctgcctacacttctttgcttcatccatcttgtctaattgggtggctgtatatgtataggccacatgtggggcaggctctgaatgggtattccttctgtcactgttttaatctttgcctccctattcgctgccaagggtattcttgttccccttttaaagaaggagtgaagcattcacattttgatcatccatcttgagtttcttgtgttctatgcatctagggtaattcaagcatttgagctaatagccacttatcaatgagtgcataccatgtgtgtttttctgtgaatgggttacgtcattcacgatgatattttcctgatccatccatttgcctatgaatttcataaatgcattgtttttgatagctgagtaatattccattgtgtagatgtaccacattttttctgtatccattcctctgttgaagggcatctgggttctttccagcttctggctaatataaataaggctgctatgaacatagtagagcacaagtctttttatatatccgggcatcttttcggtatatgcccaagagaggtataactggatcctcaggtagttcaatgtccaatattgtgaggaacctccagactgatttccagaatggttttaccagtctgcaatcccaccaacaatggaggagtgttcctctttctccacatgctcaccagcatttgttgtcacctgagattttgatcttagccattctcactggtgtgaggtgaaatctcagggttgttttgatttgcatttcccttatgactaaagatgttgaacatttctttaggtgtttctcagccattcggcattcctcagctgtgaattctttgtttagttctgaaccccattttttaataagattatttgtctccctgcggtctaatttcttgagttctttgtatattttggatataaggcctctatctgttgtatgattggtaaagatcttttcccaatctgttggttgccgttttgtcctaaccacagtgtcctttgccttacagaagctttgcagttttatgagatcccatttgtcgattcttgatcttagagtataagccattggtgttttgttcaggaaatgttttccagtgcccatgtgttccagatgcttccctagtttttcttctattagttagagtgtatctggtttgatgtggaggtccttgatccacttggacttaaggtttgtacagggtgataagcatggattgatctgcattcttctacatgttgacctccagttgaaccagcaccatttgctgaaaatgctatcttttttccattggatggttttggctcctttgtcaaaaatcaagtgcccataggtgtttgggttcatttctgggtcttcaattctgttccattggtctatctgtctgtctctgtaccaataccatgcagtttttatcactattgctctgtaatactgcttgagttcagggaaagtgattccccctgaagtcctattattgttgaggttagttttagctatcctgggttttttgttattccagatgaacttgcaaattgttctgtctaactctttgaagaaatggattggtattttgatggggattgcattgaatctgtagatcgcttttggtaaaatggccattttgctatataaatcctaccaatccatgagcctgggagatctttccatcttctgaggtcttcttcaatttctttcttcagagtcttgaagttcttattgtacagatcttttacttgcttggttaaagtcacactgaggtattttatattatttgggtctattatgaagggtgtcatttccctaatttctttctcagcttgtttctcttttatgtagaggaaggctactgatttatttgagttaattttatacccagccactttgctgaagttgtttatcagctttagtagatctctggtggaactcttgggatcacttaaatatattatcatatcatctgcaaatagtgatattttgacttcttcttatccaatcggtatccccttgatctccttttgttgtctgattgctctggctagaacttcaagaactatattgaataagtagggagagagtgggcagccttgtttagtccctgatttcagtgtgattgcttcaagtttctctccatttagtttaatgttagcaactggtttgccgtatatagcttttactatgtttaggtatgggccttgaattcctattctttccaggacttttatcatgaaggggtgttgaattttgtcaaatgctttcccaggatctaatgagatgatcatgttgttttgttctttcagtttgtttatataatggatcacgttgatggttttccgtatattaaaccatccctgcatgcctgggatgaagcctacttgatcatggtggatgattgttttgatgtgctcttgaattcggtttgccagaattttttgagtatttttgcgttgatatttataagggaaattggtctgaagttctctttctttcttgggtctttgtgcggtttaggtataaaagtaattgtggcttcatagaaggaattcggtagtgctccatctgtttcaattttgtggaatagtttggatagtattagtttgaggtcttctatgagggtctgatagaattctgcactaaacccggctggacctgggctctttttcgttgggatacctttattgactgcttctatttccttaggagttatggggttgtttaactggtttatatgttcctgatttaacttcagtacctggtatttgtctaggaaattgtccaagtgtttcttttctggtccaatctatttggagttctgtaggcttcttgtatgcttatgggtatctctttctttaggttagggaagttttcttctatgattttgttgaagatatttactggtcctttgagttgggagtcttcactctcttctattcctattatccttaggtttgatcttctcattgagtcctggatttcctgtatgttttggaccagtagctttttctgctttacattatctttcacagttgagtcgatagttttctatagaatcttctgctcctgagatcctctcttctatctcttgtattctgttggtgaagctcgtatctacggctccttgtctcttcttttggttttctatatccattgttgtttccatgtgttctttcttgattgcttctatttccatttttaattccttcaactgtttgattgtgttttcctggaattctttcagggatttttgtgattcctctctgtaggcttctacttctttatgttttcctgcatttctctaagggagctcttcatgtctttcttgaagtcctccagcatcgtgatcaaatatgattttgaaactagatcttgcttttctggtgtgcttggatattctgtgtttgctttgttgggagaattgggctctgatgatgccatgtactcttggtttctgttgcttgggttcctgcgcttacctatcgccatcagattatctctagtgttactttgttcttctatttctgacagtggctagactgtccttataagcctgtgtgtcaggaatgctgtagacctgttttcctcttttctttcagcaagttatgggaacagagtcttctgctttcggccgtgtagtctttcctgtctactggtcttcagctgttcctgtgggcgtgtgtcctgagtccattaggcaggtcacttggagccgaaaagttggtcttgcctctggtcttgggccaaaatttgctttccgtgagggctgcaatcaaagggcttgctcagccttctctcaggcctagatggcactagaacttttcctctagagtcagaaatatgggcagagagtagtctcctctggtttcccaggtttgtctgcccctctgaaggtctagctctcccttccatgggatttgaatacagggagctgtttgaccgggtcccttcagaactgggcgcagtctggaacctagcgctcctgcagcttgagtgaccatatcttcctgttcccagaggccctgtacagtttcttcttgggtcagggatgtgggcaagggtgggcagtactggaagtctctcctgccttgcagtctcaggagtgcccacctgtttggttgatgagctctctctcccacggggtttgggaacagggagctgtgggccaggatcagcgaggtttgggccccagctagaaaccagaagtgtctggtcccagaagaattttgcctttgtgtatcctgaatccagcaggcaggtcacttggagcagaaaagttggtcttacctcttgtctcgggcctgaagtcgctcctcggagctggttttcagctctccatcagggcagcaaccaaaagggcctgccccgccttctctcaggaccctgtgcacagggggcccagatggtgctagacctttttctctagattcagaaatgtgggcagagagtagtttcctctgccttcccaggcatgtctgttcctctgaaggtctagctttccctcccatgggatttgggtgcagggagctgtttgaccaagcgctcctgcagcttgagtgcccctatcttccttttcacagaggccctatacagtttcatcttgggccagggatgtgggcgagggtgggtagtactggaggtctctcctgccctgcagtctcaggagtgcccacctgtctgggtgatgagctgtctctcccctggggtttgggaggagggaactgtgggccaggatctcttcacctattcttaacattaataattcaacacacacacacacacacacacacacacacacacacagcccctagtgagtcactatactgctggtagcctgaatgtatgttttatgcttgatcacttgggattagataacttatcagagagaggcttattcttagagtagattgaattttcagcaagtattaattacctgttgttcttcattgagagggttagtgattatgaaaatttctccatatgcattgaaatgtcaactggtattgtagtaaactcacatagacaatcatagttttgaaatttcatgggctctgcctgcctgtcatatatagaaagcttttctcatagtaggcatcctagtttttgcccttaaattctttctgctccttctcaaatgatgattccccaagccttaggtttgtttagtgactactacttacataagacttaatatcttataatattagacattaaatttatttgttcctaaacagctacatttaaaatatttaaacgaaagtgcaagttgtagaaatttattgttaagaaatatactatttctattaataaatatagtatgtaatatttacattaggtttaaaatatctagatgtttgagcactttgaagaaatgtcttgctatggtctcttgccatgtgacttttagagtaagcttgctcatgcatgaaaaattcatttctggattcaattttgagaaaattgatacagcaccattaattttttctattaataactacgatatgtctatgatttagttagacccttagtctcttgtggcactgttctgttttatgcagcaacttcagtagatggatagctaatagacgttttcaaattgtagtaattgtattcatgttatctatttttcttgggtatagtttatggttttcattaattctattcattttatcttgccaaattaattgacgtgaatgttcataatattctccaattatttttgaaatttatgtaaaagcacataatgatacaattcccatcattgctgataatgttaatttgatctttctctaccttttccctacctttctctgctatgtctgcttaaaagatgattaatttaggtgtctttcataggatcgagatgtaaagttaattctgctttgtgttattttaaatgacatgactcccactcccaattctactccccctttctttaaattttctgctttttcctaatgtcttaatgagatctcaggcaactgatgtgagcccgtgttccttgtccatttgaatgttgagtgcagccagatttttgttatcatcccacatagttgtgtgtgttaatttatctattggtacttggatacaatgggtgaacattatcagtttattgttggggaaataattcagtgccacaaatgtatatgttttcattcacctctgccacaatcccttgaataataaagcagcactccatgaaaactttttgctagtgcttgggcttggaaaattgcagaataaaaatactgagtttgattttcctttgaaattattttagattggtttgccacacattttttgtacaacttgagtgttcagaatatcaataaaactctccagggggatgtctttctaaaggattatggtgattacacgaatctttactgtctacacctttgaatatcttgaattgttggtgttctgggtaccttttcctgtaatttttggggtagttattcttctcatgttcttcatcagagaatcttgtaatgtgctagactgtgctgatagaggatggcaattgagaaatgcagagttccgctccatattttctttgttcttgcttttctatgccacacgttcagtgactccagtctttttgagcaaagtaatttttgttgcttaaattcaataaaatacccatttttcttctttagttcacaatttgcaattttctggaaaactctcctttacataaagccacctcaataatgaacatcattaatctgttgcctctggtactggtaattttcaactaaatatgttcttatcatttgagtctgctacactattttatttttgtttctttataattttattatatccttttacagcaacaaaatctcattactttttctaatctttattaacctttgaacaaccattctattttaggcatgcagctgaaattattggcactggagtctgtagtaactttggatatattttttaagatcatcattcgactccagaatccctagtgggatgaaatgagatctaggttcctaagagatccaattattcttaagcagaaagaaaaaaaatgaaagaatgaatgaataaaaaaagagagaaagaaaggaagagagaaagaaagaaagaaaaaagaaagagaaaaagaaagaaagagagaaagaaaatattgtccagagttctgatggtctataagatatatattcatttggacaaaaatgttaaacatatttaagaacatattataaatcctttcaattttactttgttagaaaaaaactttctcagaggactatgatgatgtatgtttaaaacgaaaggtttgttgttttttcttttctttttcttttcgtttcttttttttgtttttttttgtttttttttctttttttggcctagtgatgggaaagactttgattatttcatgtacaaatgactaatgactacttctgcacctttaatattgtagatccctaggctgccatgcctatactcacctcttttcttactttttacccttttagagacttgttcagtatcagatatagaaattgaaaatgggtttttttctgaatctgattatacatatgctctaaatagaaaaacacggtatagatgtaaacagggatatgtaacaaataccggagaaatatcaggaataattacttgtcttcaagatggatggtcacctcgaccctcatgcattagtgagtattttattatattgttgcaattatactaatgatgcataggagtttagtgttattctttttgtatatgattgatattctttcatttgtaaacagctttcaaacttcaagaaaaaatacacagcattttttttatttagacattcctgcattgtaaaatatcagttcatttgcctttttctaggctctaaaatagcctagttttaaatctagtgaagaagtctttgaccagatgcaaattcctgaatatatgataaccttataatatgtacgtgacactatgagttacgatctatttcagaacatctcccttttagaagatctttttaaatattttgatattggaaagaaagaaatgcttccaggcaccaggaaattttggtatttggaaacattcttttgttttaggacatacagttaatgaggattttctaggattaacaattagctcatctagtcttatttataagaaaaatacccagtgctatttttcaagatgtattcaatttataccttattgtttaaggtatgatttaaagtattcactaagttcataatttttcgtctactgtgattttacaggatttaattaaagaaaaggaaattaaaattattcccatataacattcatttatattaaattataattggtaaggatttattgaatttttttactgtgaaagggaaaacccttgatataatatctgcttaaattcaattcatctactttcctatattttatgagtcatttgatgtactaattataggaccttaattcgcaaaatgctatcatactttcctaaaattatgtatttgcacttgtctattttttggagtatgtgataagtataagaaaaattgagctgagaaatgatttctaaaataaaattttataaaagcttaagaaaggagatgaatgttacatagagtatatctcaattttaataactttcaagaaaataaattattactggtctccttagtttccttcaatacagtatttaatttgctatcatatattaatttataaagacttttttctcatgagaattatttctacttgctattgacacattagaaatgacattgtctctcttattttgcattagagtcttgtgatatgcctgtatttgagaatgctatgactaagaataataacacatggtttaaactcaatgacaaattagactatgaatgtcacattggatatgaaaatgaatataaacataccaaaggctctataacatgtacttatgatggatggtctagtacaccctcctgttatggtaagtactattttctctggaatatttttagataaaaataaatgtttgtgttattaataactgaatgttctagaatcttccttatgagttaatgtagcctaagaaaaaggactgttatgaaagctatcgataataatatttacatttattatatcattacattcatttatttatcctgtgtgtatacatgcacacatatgtgtgtttctggaagtgtgtatactgcattatacaggtaggtgtcagagaacttgtgagagtcagttccctctttcatcatatggatctgagggattgaagaggactccaggcctaaaggcaagcactcttactgactgagccatctttctggcctgataatctgtttttaaaaaattctatattcatcagttgtatatggcactggattatgattctagcaattaggaccctgaatcaagagatttttaagtttgaaggtatattggactacatactaagttctgtttctaaaaccaaacaaaccaaaaatttcattaaattaatgattcctttgtgtggcctgtgtgtatcatgtatctctgatttgaggacaattcttttgttattcaagctcttatgtagactaggtctccattatcaaatttatgatctgaagcatgaaactaggtaatgaaaacttgaggcctggagagatggctcagcaggtaagagcatgggctgctcttccagagatcctgagttcaattcccagcaaccacatcatggctcacaatgaaggaggtagaagtatggcattcttgaaatctaggccagtctgggctatgtaggaattgtaagtggtaagtgcaggaattgtaggaatacagctctgaagggaaaagcttccccaatggagatgctgcagctctgagtgtctcagtgcaagtatgacagctctgaagggaaaggtatcctggcagtagggagctaaggaaaaccacaaacttacactgcacaaaacaaacctggcacaagaactttattgggaaaaacataagaaagctgtttctgctccagattaaagcagcaaagaacaagctcagtgattggtgagattttgagtttatcttgggcttccaccccatccctaccctccagaaaggaacttggccattagcacctcaaggggctagactgccattatagtagtctggaggtggggcttggtcacttgcgtgacttcaagggacttaccttaagatggtggctgcctctgtttgaccaacatacaacaggaaactgagcaggagacagataaatataagttgtttttttttccgggggtctgggggtagggtgggttttggaggataaacatttccaaggtggggaatggtgagattttcaagatcaagactggtgggtattcacactcagggcttggtagggtttcctatttagggattggtaggtttgggtaggttttaagccatgaaatgggctcagaacttttaccctaaatgaagacatctcacaaacagacaaacagcaacaaatgatgtacatagtaagaaaaaaatcaaactaaacaaacggtgatcactagtttctctctgattataagcagttcaacattatgaaatcaggactttctataatacaatactaaagtagaatggaaggggagggatattagtttcacaatacaatactttgcctaaggatcagtactaacactacaagtataaaataaaatataatataaaattatttatatactattctgatgtgtgagaattttttttctgtgaagtcaatatacaaacatctactcaccccaagaaagagcccatgacagaccaatgtacagataccactaatttccaacttcatgaaccttgagtcattgtgtccagttgcaaaatccccaaagagactacccggaactgcaacttccacacacgcacaggagagtctttattcaagctcgagcttgggctacgtaccttcctgatggaataggaaggagagagatacttgagtctaggggcttagggcttatatagggaaaaatctcaagctggagtcttcaagccttggcattacatgtttgggtaaaggggtaaaggaatgttaaccttcagactgatatcatcagggggagaccacacatttaaaagaggcatcttgtccttggaatgatttatgtttttttaacttattattgtgaccagttttcctgttgttgcaagctggccactgctgttatatctattttcaactgctgggaagggttggttgtctcttttccagagcccaagatgggggccatatcacttcaaggacagcagttttctccaaggacagcagcttttcccaaggacagcaattttctccaaggacaagatcttaaaattgaatttaaaggaaaagatggaatccctcctgctgccttttgccttttcagagttttattaaggttgctttcagaaatatgaatgagggtgttctcataggagaagaaatggctcaaagacagctacatcaccaaagcctacccagtatggctgacaattcacaaaacacaatggatcatataacataatgtgtaggcagcacatagattgaggagtgtcttttcaagtgagtcagctgatgaagcacctaccactgggtaggatccttcttctaggaagttaattatctcattctttgctccatctagggagctctgagctccttccttgcagttttgcttgtctgagtgattctcaccaattcagctagcttgtttactctggaagtaaggggcctgctaaatctgcttagtttcagggactccctgaagctattttgagttgtttacttccctccttaaggagcttccctgcagtatggagtatttcagtctcaaggaaactgttgcccaacaaattcccatggtctttcaatgtctccaggtctgacaggtgattgtaaagcagaggagaattgcacaaattattttttcactttaagacagagtattatggtatgtttgctaaacaatttgtataaaataagcaaagagaatacacaaataggtgcaaaacaaaaaatagttatagatgattatattgtgccattcaaatccacttggaaagagcacacacgtagattcaattcaagtttaggttaaatgaatttcttcttatttctatcaacacagaagggggaggaagggagggtttataaagttggattcctaaagttgcatattacaattagccatgaaatctgcagctggaccaaaaagtgtttttgcatccctcagttgttctttacctttgtatgccaataaaaagatcacttcatccctgtcccacaaaagcaaaaaacaaactgtcaaacatcttacaacaggaactctagtaacctatctaaacttttctgttttctttacttttctttttacttattcttctctcttacaataaatatatcctgattgtagcctcccttcccccaactcctccctgttcccactttcccttctctaccagacctactgctcctccctttcccttcagaaaagagcaggcgattcatgaatattaatcaaatatgacataacaagatataataagcctaggcataagcccttatttcaaggctggatgaaacaaccaagtaggataatggtctcaagagcaggcaaaagaattagagacacccatgactcccattgttaggagtcccacaaaattcccaagctaaagaacactatgcaaaggacctagcacagacccatacaggctctttgatttcagctcctgtctctgtagcctctatgagtcctacttagttgattctgtggcccacgtttttctgctgttaccattccacacacaaaattcattctattgccccttcccagggtgatttccttcttacttctctccacttcttacttagcctccctttgtctgtgtgctgtcacatgattagcctttacttagctctaataactacttatgaatacataattatttttgtctttccaggtctggttgcctcactcaggatatgtttttctagttccatcatttgcctgaaaatttcatgatggcatttctctaacatctttcataatataccattatataaatataccacatttttatgcactcttcagttgaggggacatctaggtttctaagctatccagtctctgtttgctggccctcaggttagtgcctggcatggctctttctcactgcattgggatgaagctgtaccaatcattgattggccactcctgcaagttctgcagccgtatcttgcaggagaaatagtcggctgaagattttgtggcagggttggtgccccaattcctcaactggaaatcttggttagaaaagttggctggttcaggctccttaaaccccagtactaggagtctttactaggctcacactcaaagattccttggaatttcccttgcactaaggtttggtcttgtccctgaaataccccaaattctaatcatctctttcaatactttctcactccaccacacctgatttctcctcttaccatcccttcagttttgaacatagcagttgtcttttatgaatgactctaattaaaaattatgacttttaatatatacattggaaagaaaggagatttttaaggcagaaatgtgttatttatttatttacatatttttggtaacactcaacaatgacaaaaattgaagaaaaaatttttcatacaggagaatgtgtcatacattcttaatttgagtcagaataattcacaattaattaattaaaaccagaattataaaactggtttaatgtaaaggttttgcacaacttttttatagtctacttaatcataaaatatactatattttcctaacttcagataaattagaaattattttatatattttagtttctcattatattaaactgaaatgatttcaatatatgatgtagatatagtatgacactaatttcaaatctgaaggaaagaattttgtgttgtagaataggaaagttattactttaacattaatatttatctgcagcagctcagatccactggaagacagttggttttattaaatcagttttgtgattaatacattatgctttgttatgtttctcagagacgtccacattgacttagaggctatattaaagctaggacacaatgtttttcctaaggaagagggtttctgaagcttccctgtgaatgtacatgagaaagataaaaatacttatcaatgattaatggtatattctaattatcttttcaagaaagagaatgcagcattcccctgttacaccaagacttagttgtttttcccagagaagtaaaatacaaagttggagattcgttgagtttctcttgccgttcaggacacagagttggagcagatttagtgcaatgctaccactttggatggtcccctaatttcccaacgtgtgaaggtcagtatctgttttatatttgatgaactaagatcagaagtttattttttttcctcttttagtattccccagttatcaagtatgtctataatataaaaatcttcagagaaatgaacattcattcagatacacagccacatgtttatgaggttaatttgaagctaacttgcttctttaaatgtgttatccatgtgtttacacatgcagacatgatggctgagactgatgggatttctttcattttgcctatattaccattagtgctggtgtttttataccataggccttcccgcatattgtatagagtacgtccaaacctgtaaaagcaggttgtaattaattcaaaaccaggttcaatatctatttaaaatagatacgaggtacaatgctgattttttttacaatgtggtaaatgtatgataaaatagtaccagtcaatgtgaaaatcattataatcaacacaacaattactgagtgattgcatgtatcttcaggctgtcaggtttatcaaaaattcttccacctccaatatatttgcaatgctattgcaacagttgtattaaagttgtgaaatgtaaatttagtgtaaatactatttagaaaagtgtaaaagaaagttatatagtgtatacatttaaattttctccatttactaaaattttagactgtaagatggacattttcttttatatttatacagtatttctgtaacaggccaagtaaaatcatgtgaccaacctcttgaaatcccgaatggggaaataaagggaacaaaaaaagttgaatacagccatggtgacgtggtggaatatgattgcaaacctagatttctactgaagggacccaataaaatccagtgtgttgacgggaagtggacaaccttgccgatatgcgttggtaattaaaataattaacacttaaaaattgttttgcatctcatgtgacgttttaattataagtaacttaagtgaaatacctacagagtatgagagaacatgtggagaccttcctgcacttgagcatggctctgtccagttatctgtccctccctaccaccacggagattcagtggagttcacttgtgcagaaaccttcacaatgattgggcatgcagtagttttctgcattagtggaaggtggaccgagcttcctcaatgtgttggtaagtatgtgtgcataaaatggatacttcataaagtttaatatttatattgcagaaatatttgctactgtgtacttctgaagtaagtagtcattttggaaatatctagtcttaaataatatgaatccaaactttcattgtttatattttgatggatgtctacaggtgaacagaaattcttaacatacaatatataaaagtttgttcattaccacaagataaatctagttgttaattataaattgtcatgtgactgacatgtgaatattaacacccaagtaggtttgactatggtacaaaaaagatcattgtttttattgtatgagactctcctctcaggacttggaaaggtaagaattaaagtctgctaatcacccatttcctactctcattatagacttaccctgaagcatgtctgtaatgtttgtgtttattctacagactgcattctaaagtcaatgtgccaaagttgggactctccaccctgccatcagctgtagaactcagggattagatgggaaacataatcccatatatgactccacttcacactgattccccatgttcctttgctgattcagtcttaatgagttactggaagaatcttggtgtctacattttcttttctctgaaatggaagtttttcattgattgaccttggtcatccaggcttcactatttgttggagttttggatattctttaatgccagggaaacatggagctcctttggaacgggcacctattcttgtgctgcttaatgatatgctctctctgcccagacacccaaacttcataacagtttgccatgtaaatgaatacctttactacatatcaatcataacaatttttgctcagcaagcagattttgccaaacccatcttcatcattgctttaaaactgtttaacactttcataagaagaaagatcagatataatatcatatataaaaactgaatccttcattttatattagtttatgcttatttttatgtactctattgtactctagtatttgttcatatatcagaggtttagtttggtttatctgcctgcagccaccttaatatgactccagttatgtcttcctggattgcaaagttaatgttatgatacaaatatttttaccttgacactctaccttacttttctccaaacccttggctttcacctgatgaataagagattcagaagcaaatcaaccacacagtcaccatgcccctttgactttcttctttttcctttacagaaattggctttgtgtgtgtgtgtgtgtgtgtgtgtgtgtgtgtgtgtgtgtgtgtaccaatctttagtaagggacgaattctcaggagtctttagtgtttgcatcactctatcaacattttaaatattatacaactttgtctaattatttacttttatttgtactgtgtttattttattttagatttcaaattattgataaaaattatccatgacctatacagaaatgtcaaattcaaaaggactctcattttcaccaaataattaaaatgtatagtacactaaaatgcttccatatatatatacatatatccttatttaacttataaaacaaccatacaatcagaacaatttattattataacttaatattgctgtattatagaataacgtcatatgaaaatatatcttatagactcatatgtagggtgtataaaggagatagatgttgactacaagcccctaatatcctataccaattctctctcataaaatagtttgaaatatttgtattctatacaatataaattaaatgttattttcttgtatcacatctattaaaaaagatgtcccgatatcttatcaacacattttttattttaaaatttttaacattttaacattatgaaaaaatctgagagtaatgaatttgcatatttttataggttttaagtctatgaccaaagctggtcatatcataatcatttcttatgtagagcatctgagaaagtgtttttttaatgcttttgtaattgtctagtacccaagttccttcatgacacaaaatgtctctgagacataaatgagtgggcatgatatctagttcttatactataggccactttcgcatggtgagtctcaacattttagttggcagaatttatagtactaagttgtgtttcattgtacatttactgcatgcacattttaatgtagtagctcactcacttcttataagtgtttttatttttcatgaaaatattttcatacagcaacagatcaactggagaagtgtaaagccccgaagtcaactggcatagatgcaattcatccaaataagaatgaatttaatcataactttagtgtgagttacagatgtagacaaaagcaggagtatgaacattcaatctgcatcaatggaagatgggatcctgaaccaaactgtacaagtaagttcttcttggcattgtgttctcatgagtgttctagccttttctcaactagagcagttgtgtctttatttacttaaaaaatttttcctcaaattttatgggtaaaacctgtatttatattatttttacctctccctcttcccactccaactcaactccttttgtgtccctccaattttatatccaatttatgtcctcttcttgaagtatatgtgtaagcatacataatatatgcataatatatacaaatgaaacttgtatatataaattcaacctgattagtccattcagtgtttctcctatgtgtatgtgctaagactaagtgcatgggtttcaataacctatttgtttgctccagagagaaggctgattattccactctagacagccattaatcacctgtaggggaagggtcatgtagcattttccctatccatactaatttgtcagttggtaatgtcatcatggatatcttgttgggtgaccacacttttgagatttcatgagttcatctactctgccatatatgaagatattatcttctaacacattttctggaaaaaatattttttaatctagaggttgatttagaaattacaatatcatgcttgttagtgacctatagtgtaaaacacagaaacaaacttgctcaacatggcttttcctatgtgtcataatggattcttaccattccactacatgtgattaatttatcacaacaaatgtgttatgcctctcctatgcttcatcatcatgtctttcggtatgattgtgtgttctgtcagaccaaccatttatttaactctcctaacaatcagcttacctggaaaacctcgatttatttgacaccttctattctatgttactgggcaacagggccattctactactatttctgcttccctatttgtctttatcaccgttgttgtggaggccctgtctcatttgatattttaaatatttcttaaagacgaaagttcacagaaagtatttccatgccattctaaaattaaacctactacaggcatgttaatgcagtgcatgtgttgttttgaaattgtctatgttaggatatcatttctggtgtcattttgattatagtattaagatagtaattgcttttctcttatgtatggctagctagttgttcaaagaatgtatttactacgtagtgctgatttctatttattccactctacttaagcaaaaatataaaaagaatgaaattattagtaaccactaagaaagtaccctttcatattatgaatctgagaggagagtctgagtgatgaatgtgaggtgtcttgattttgtagctacgtagtgaaaaacttgtcagaagcactacattatcctggctgcgaaccatccgttttcacatgtgtaactagttcaggttaaatggaatgtccagcataattgaaattttgtacaacatagtataaaccactttgggtcacactccatattcttgttgaccaagaaccaaggttaagttaactatcaattgtgataactaattcttatttgctatctgacagagtccacaatttcctaagaaaaacgtatctgagcatgtttgtaggggcgtttctagtttaggttaactgaggaggaacaatacactgtatgtgtagatggcaccattttatgggcagggttcctagcataaataaaaagagaaaggtgactgtgaatcctgagtatagatacagtatgagcaacagcctcacatgtctactgccattgctttcctgcgcgatgagctaacttaaactattccttcttcttttctaccctccttcctatcttccttcctaccttccttcctttcttagcttcttttgtcaagtgcttcatcacagaaatgagaaaagtcactagtatatcaagtaaatgaaagtaccacttttcctaatcaactttcatttataaaatagtccctgaggatttttaatgtaagtcaacatattagattataaatagtcatagacagctctagaaaaatattcatgtaagcttaatcttaacataatatattttttatgactcacttaaaatattttaaaatctagaaatgattgaagtatgttttataaaaatatataaaactgcattaaaatgaatgagaaaaaatttggagtacaagaattgctatattaaattgctatacaattgaaatatgcaaaatatagacaatttttttgcaactcaacaatcagatttatatgctaaattctcaatccacaatagattcacacagtaaacttacaagcaatcgataaggatataaactgccaacctagatgagataaatttgcctacagaaatccatgccaacaaccttggcaatactatatatatatatatgtatacatatatatgtatatatgtgtgtatatatatgtatatatgcatatatagagagagacagttattaaatttcattactaacttactttttaatgaaaattatcacttcaataatttaagatattctctttagtaaagaactctgattatttttttctaggaaatgagaaaagattctgccctcctcccccacagattccaaatgcccaagtgattgaaaccacagtgaaatacttggatggagagaaagtatctgttctttgccaagatggttacctaactcagggcccagaagaaatggtgtgtaaacatggaaggtggcagtcgttaccacgctgcacgggtcagtagataggatttactttgcaccattagaacgtaggtgaggggtgggtattgaaaaaaaaagggcatactataaatgttctggacacattattcaaattgtgtatatttatttctaatgtaagtttttatttcggcttgactatttcatttctgttctctatgtagaaaaaattccatgttcccagccccctaaaattgaacatggatctattaagtcgcccaggtcctcagaagagagagatttaattgagtccagcagttatgaacacggaactacattcagctatgtctgtgatgatggattcaggatatctgaagaaaatagggtaacctgcaacatgggaaaatggagctctctgcctcgttgtgttggtgagactgacatgaaaattcaattttcattttcaatatgtcattaccaatattctactcttatccaagccagagagaaagaataatttaggatagcacatatatacatttatatattttactatacatttatacttgcacactataatctatgctgttttagttcattgtgccatttctgtagacatatactttcactcttgcattaccgtttttaaatatgatgtattacagactccatgtgctcatgtgaattctactgtttgatttgccaccaagtattaaagtccaaagtatcttttgcctaaaatgtcctccccactcccatcccacaatacatggtattttctgatatttgtaatactttcaagttgtttaacagatgcaagacaacagaatgtgctattaggaagcactgcccaccttccttatgatgatgcatctttcatattaacacttccttcttgtacccctacacacagaactgatacatacaagcaaatttctgtattagtgcaatgtggaattgtttaactatgtaactctcatttgtgtctttttcaggaataccttgtggacccccaccttcaattcctcttggtattgtttctcatgaactagaaagttaccaatatggagaggaggttacatacaattgttctgaaggctttggaattgatggaccagcatttattaaatgtgtaggaggacagtggtctgaaccacccaaatgcataagtacattttaattttcattcttttgtctagtatataatacaattcaatctatatgtggtacaattaagaagctaagtcatactttgattccatatctcctcctatgaatatgtttgtttcccctctaagaaaaactgaagcatcctcactttggttatccttcttgagcttcatgtggtctgttgattgtatctttgggtaaactaaggttttggactaatacccacttatcagtgaatacatagtatgtgtgtttttttgtgattgggttgcctcactaaggatgatacttcctttttttatttttattatttttatctttgttaacttgagtatttcttatttacatttctattgttattccccttctcggtttccgggccaacatccccctaactcctccccttcccctttcatataggcttcccctccccatcctccctctattaccaccctccccccccaaaatcacattcactaggtgttcagtcttggcaggacccagggcttccccttccactggtgctcttactaggatattcattgctacctatgaggtcagagtccagggtcagtccatgtacagtctttgggtagtggcttagtccctagaagctctggttgcttggcattgttgttcatatggggtcgcgagccccttcaagttcttccagtcctttctctgattccttcaaaagaggtcccgttcttagttcagtggtttgctgctggcatttgtctctgtatttgttgtattctaggtatgtctctcaggagagatatatatcaggttcctgttggactgcaccttttgcttcatccgtcatatctagtttgatggctgtatatgtatgggccacatgtagggcaggctctgaatgggtgttccttctgcctctgttctaaactttgcctccctattccctgccaagggtattcttgttcccgtttaaagaaggagtgaagcattcacattttggtcatccttcttgagtttcatgtgttctgtgaatctagagcaattcaggcatttgggataatagccacttatcaatgagtgcataccatgtgtgtttttctgtgattgggttagctcactcaggatgatattttccagttccatccatttgcctatgaatttcataaagtcattgtttttgatagctgagtaatattccaatgtgtagatgtaccacattttctgtatccattcctctgttgaagggcatctgggttctttccagcttctggctattataaataaggctgctgtgaacataggggaacacgtgtcttttttatatgttggggcatcttttggatatatgcccaagagacgtatagctgggtcctcaggtagttcaatgtccaattttctgaggaaaccccagactgatttccagaatggttttaccagtttgtaatcccaacaacaagggaggggtgttcctccttctccacatcctggccagcatttgctgacacctcagtttttgatcttagccattctcactggtgtgaggtgaaatctcagggttgttttgatttgcatttcccttatgactaaagatgttgaacatttctttaggtgtttctcagccattcggcattcctcagcagtgaataatttgtttagctctgaaccccattttttagtagggttatttgtctccctgtggtctaacttcttgaattctttgaatattttggatataagccctctatctgttgtaggattggtaaagatcttttcccaatctgttggttgtcgttttgtcctaacaacaatgtcctttgccttacagaagctttgcagctttaagagatcccatttgtcgattcttgatcttagagcataagccattggtgttttgttcaggaaatttttcccagtgcccatgtgttcgagatgcttccctaatttttcatctattagtttgagtgtatctggtttgatgtggaggtccttgatccacttaaacttaagccctgtacagggtgataagcatgcatcgatatgcattcttctacatactgacctccagttgaaccagcaccatttgctgaaaatgctatcttttttccattggatggttttagctcctttgtcaaaaatcaagtgcccatatgtgtgtgggctcatctcagggtcttcaattccatttcattggtctatctttctgtctctgtaccaataccatgcagtttttatcactattgctctgtaatactgcttgagttcagggatagtgattcccccagaagtcctttcattgttgaggatagttctagctatcctgggttttttgttattccagatgaaattgcaaattgttctgtctaactctctgaagaattggattggtagtttgatggggattgcattgaatctgtagatttcttttggcaaaatggccatttttactattttaatcctgtcagtccatgagcatgggattctttccgtcttctgaggtcttcttcaatttctttcttcagaggcttgaagttctcatcatacagatcatttatttgcttgattaaagtgacaccgagggattttatattatttgggactattatgaagggtgacgtttccttaatttccttctcagcttctttctctttcatgtaggggaaagctactgatttatttgaattaattttaacccagccacattgctgaaagtgtttaacaggtttagtagttcccttgggatcacttaaatatactatcatatcatcagcatatagtgttattttgaattcttcttttccaatctgtatcctcttgatctccttttgttgtctgattgctctggctagaacttcaagaacaatattgaataagtaaggagagagtgggcaaccttgtctagtccctgattttagtgggattgcttcacgtttctctccatttagtttaatgttagctactggtttgctgtatatggcttttactatgtttaggtatggaccttgaattcctattcttttccaggacttttatcatgaaggggtgttgaattttgtgaaatgctttctcagcatctaatgaaatgatcatgtggttttgttctttcactttgtttatataatggattacgttgataattttctgtataataaaccatccctacatgcctgcgatgaagcctacttgatcatggtggatgaatgttttgatgtgctcttggattcggtttgccagaattttttgagtatttttgcgttgatatttataagggaaattggtctgaagttctctttctttgttgggtctttgtgtggtttatccatcttgacctgggctctttttggttgggagacctttaatgactgcttctatttagttcagagttatggggttgtttaaatggtttatctgttcctgatttaactttggtacctggtatctgtctaggaaattgtccatttcctgcagattttcaagttttgttgaatataggcttctgtagtaggatcttatgattttttgaatttcttctgattctgtagttatgtctcccttttcatttctgattttgttaatttggacacactctctgtggtctctcattagtctgactaagggttaatctatcttgttgattttctcaaagaaccagcttttggttctgttgattctttgtatagtcctttttgtttctacttggttgatttcagctctgagtttgattattttctgccttctacgcctcctgggtgtatttgcttctttttgttctagagcttttaggtgtgctgtcaagctactgatatatgttctctcctgtttctttctgtaggcacttagagctataagttttcctcttagcaccgcttccattgtgtcccataattttgggtatgctatactttcattttcattaaattctaagaagtctttaatttctttatttcttccttgaccatgttatcattgagtacagcattgttcaacttccatgtatatgtggacgttcttcccctattgttattgaagaccagctttagcctgtgatggtctgataggacaaatgggattatttctatctttctgtatcttttgaggcctgttttatgacttactacatggtcaattttggagaaagtaccatgaggtggtgagaagaagttatatccttttgttttaggatagaatgttctataaatatctgttaagtccatttggttcatgacttctcttagtctgtctatgtctctgtttaatttgtttccatgacctgtccattgatgagagtgtgtgtgtgtgtgtgtgtgtgtgtgtgtgtgtgtgtgtgtgtgtgtgtgtgtaatctactatcattgtgtgaggtgcaatgtgtgttttgagctttagtaaggtttcttttatgtatgtagatgccttgtatttagagcatagatacttaggattgagagttcatcttggtggatttttcctttgatgaatagaaagtgtccttccttaccttttttgatgacttttagttgaaaatcaattttatttgatattagaatggctactccagcttccttcttcagaccccttgcctggaaagttgtttttcagcctttcacactgaggtagtttctttctttgtctctgaggtatgtttcctgtagacagcagaatgccaggtcctcattgcatatcaggttcattaatctatgtctttttattggggcattgagacgtttgatattgagagatattaaggaatactgattattgcttcctgttatattcatatttggatgtgaggttatgtttgtgtgcttttcttctctttgttttgttgccaagacgattagtttcttgctttttctagggtgtagcttgcctccttttgttgggctttaccatttatcctttggagtgctgagtttgtagaaagatattgtgtaaatttggttttgtcatggaatatcttggtttctccatcaatgttaattgagaattttgcaggatacagtaacctgggctggcacttgtgttctcttagggtctgtatgacatctgtccgggatcttctggctttcatagtgtctggtgagaagtctggtgtgattttgataagtctgcctttatatgttacttgacatttttccttactgcttttaatattctttctttattttgtgcatttggtattttgactgttatgtgatggcaggagtttcttttctgatccaatatatttggagttctgtaggattcttgcttgtttatgggcatctctttctttaggttagggaagttttcttctatgattttgttgaagatatttactggtcctttgagctgggaagtcttcactcttttctatacctatttatcttctcattgagtcctggatttcctgtatgttttggaccagtagctttttccattttacactatctttacccttgtgtcaatgatttctatggaatcttctgctcctgagattctttcttctgtctcttgtattctgttggtgatgcttgtatctatggctccttgtctcttcctttggttttctatatccagggttgtttccatttcagctttctttattgcttctatttccctttttaattccttcacctctttgattttgttttcctggaattctttctgggatttttgtgattcctctctatagggttctacttgtttatttatgttttactgcatttctttaagggagttcttcatgtctttcttgaagtcctccagcatcattatcaaatgtgattttaaatctagatcttgcttttctggtgtgtttggatattcagtgtttgctttggtgggagaattgggctctgatgataccgtatagtcttggtttctgttgcctgggttcctgcgcttgcctcttgccatctagttgtctctggttttatcttctgctatttctaacagtggctagaccttcctatagggctatgtgtcaggagtgctgtagacctgtttcccttttttcgttcagctagttgtgggaacagagtgttctttagggtgtgtagtctttcctgcctagtggtcttcgctgttcctgtgggactgtcctgagtccaccaggcaggtcacttggatcagaaaagttggtcttacctgtggtcctgtgtctcaagttgctcgtggggggctgcttttgagctctctgtgagggtggcaaccaggagggtctgtgcagccttttccatgagcccccgagtactggggtcccagacggcattaggtgttttcctctggagtctgaaatgtgggcagagtgtagtctcttctggcctcccaggcgtgtctgcccctctgaaagtttagctctctctcccatgggatttggctgcagagagctgttgattggtcccttcaggtcaggtgggtatctggatcccaggggacctgctgctccagtgcccctgtcttccatttcccagagactgtatacagtttcctcttgggccagggatgtgggcaggggtgggcagtattggtggtctcttctgctctgcagtctcaggagtgcccacctgtccagatggtgagctctccctcccacaggatttgggtgcagagagctgttgatccggtcctttcaggtccaggcgatgtctggagcacaggggacctgcagctccagtgcccctatcttccagttcccagaggccgtatacagtttcctcttgggccgcggatgtgggccggggtgggcagtattggtggtctctccctctctgcattctcaggagtgcccacctgtctgggcggcgagctctctctcccaggggtttgggagcagtgaagtgtggccgggatcagcgagattcgggctccagctaaaaaccagaagtgtcctgttccagaggaattttgcctcagtgtgtcctgagtccaccaggcaggtcgcttggagcataaaagttggtcttacctgtggtcttgaagctcaagttgcttgtgagggggctgcttttgagctctctgtgagggcggcaaccaggagggcctgcaccgccttttcctggagcccctgtgcaccgggatcccagatggcattaggtgttttcctctggagtcagaaatgtgggcagagtgtagtctctttttgcttcccaggagtgtctgcccctctgaaggtttagctctccctcccatgggatttgggtgcagagaactgttgagcagtcccttcaggtccgggcagcatctggaacgagggggacctgctgctccagtgcccctgtcttccagttccaggaggccctatacagtttcctcttgggccacggatgtgggcaggggtgggcagtgttggtagtctctcccactctgcagtctcaggagtgcccacctgtctgggtggtgagctctctgtcccacagggtttgggagttgggagctgtgggccgggatcagtgaggttaggaggatgatactttctagttccatccatttgcctatgaatgtcatgaatcattgtttttagttgctgagtaatactccattgtgtagatgtaccacattttctttatttattccactgttgaggaacatctgggttctttccagcttctggttattataaataaggttgctatgaatataggagaatatgtgtcctggttatatgttggaacatcttttgggtatatgcccaagagaggtatagctgggtactcaggtaggtcaatgtccaattttctgaggaacctccagactgatttccagaatggttgtaacagcttgcaatcccaacaacaatggaagagtgctcctctttctccacatccttgccagcatctgttgtcacctgagttttttatcttaagaatgtccattcagatactgccccacctggggatccagccaatatatatacagccaccaaacccagtcactatatgccaagagctgcatgctgacaggaacctggtatggaagtctcctgagaggctctgccaaagcataacaaatacagagatggactgagaactgggtgcatattggaggagttagagaaaggattgaaggagctgaaggtgtttgcaaccccctaagaacaacgatacccaccaaccagagctttcaggaactaaatcactgtccaaagagtacacatggacagacccatggctccagttgcatatgtagcagaggatggccttgttggccaccaatgggaggagaaacccttggtcctgtcaaggctcatcctccaaccctttcctatctgacattcccacccccccccccagtttaggcgactgtaagataggaaagggttggaggatgggcaggggaacaccctcatagaagaaagtggagagggaatgggacagggggtttgtgggcaggaaactggaaagtgggatggcatttgaaatgtaaaaataaaaatatccaataaaaaaactaatgaaggagaatcgggtatagttaaaaaaaaaaagaaacgaagccataattctagcatataaaaagtttttgctgcataatttgaatgctggaagacaaatacgatatgagtcaaaacaaaatttttcctttccagcccacctaagttgtttttgttccatgtagtctgagatatctgaattatcagaattctcagaatccaggaacacacaggctcctctaaacagtctcatcactacaatgacagttttagagcaatgccactacaattacatatgctctaaatttttcaaataattatgagtaagttacattttataaagtcaaacataaatactctaattttggaaagtacaagaaaaattgaatgcaaaatttaaaatttcaaaaattataaccatcaggattctgtgtctatcttatttattttcataaatatagaagaacgtcagtgtaactaagtaaaaaatggaaaacctactgtatgtattgttttctatgaagttaactattgtttcatatatcgtatgttctacaacttcctgaaaacaaacacccacatactcttttatttttttaagaaactgattgtgacaacttgcccacatttgaaattgccaaaccgacagaaaagaaaaaaaaatcatacaggtcaggagaacaagtgacattcagatgtccacctccgtatcgaatggatggctctgacattgtcacatgtgttaatacgaagtggattggacagccggtatgcaaaggtatttgaatgggtttttaacatgcatttattctagtgtcaaagaatgacataactgaaaatggtgcagagattacttttaaagtaagatcaagtttgtttgtatcaaataataaaagcattgaattaaaaaaactgatggctaagctgatagcatgatggtgttcagagtttgatttcatggtcagcatcatcagtatcattagaatacaaacattttgaaaatgtaaattaacagctaggagtacatgctagatatcctaaataggacgacatctaaagatgagaccttcaatctccttttagggatctgtgtatgactaagtttggaatgtgctgtaggctgtcaatatttgttaatatgttgttaaataattagccttcaattgaaatcttgcttatatctcattttatcaaattcattggaatattaggatattttatttgattatcactttcttatgactatattattcttaaaacaatgttctttttcctctaacattgcaaatagatttttttctcacataatacatatcctgattgttttctcttccctccactcatttcagctccttcctaccccttttttcatctaatttttcccctttctgtatttcaggagaaaggaaagtcttctaaggagtaatactaataaaacaaaaatgaaacaaatacagtaggaggtaacaaacaaataattttagggaaaacagcataagaaaatagataagaaacaaaatagacaaaatgtcccactttatacacctaggaatcccttaagaatactcacctgaaaaccataatatatattgaacagcatgcaaagtaccttcctgtaccaaagatgcttcccttaggggtgaaggctctatgtaggcatcagtgacactttgctatgatcagtgagttgcatatttgttgtttttcacagtgtagacttgccttcaggttgtgtggtataatctgtagtcttctcaacagcctgcctgtgttattcggaagtttccatgtgacccctctggtacacatttaattagatgtaaccttatcacagtactagaagcttcattagtgacatgatatgtccctcggggctctgtctccttacacttttggtgattgcacttatatttcctttatatatgtatgtattttagaaagcttatattgaattaggttttgataatatccctcaaatgacacttaacttttgctgttcctctctgtattctgatttttgtctacccttcttgacatccataactatctactctatttctccatcctaaggagacagtactttgcccccaattccttaggcctacacctaaattctgttgttctgtggattgtaaagtgactttcattggctttcagctaatatctacatatcagcaaatatatacatgtgtgtctttctgggtctgagttcttcactcaggatgaatttttgtctattacccatcatttacctgtgacattcatgatttcatttttgcatgtaaataaatgtagcaaattttctttatccattcagcaagtcagaaatatatttggaatcttatgcattaattggacactcaagatgagcaaataggtactaatactttattttactctttagataattcctgtgtgaatccaccacatgtgccaaatgctactatactaacaaggcacaagactaaatatccatctggtgacaaagtacgttatgactgtaataaaccttttgaattatttggggaagtggaagtgatgtgccaaaacgggatttggacagaaccaccgaaatgcaaaggtagggcatcatttcccctaatgtttatttgacaatgcaatttagttattgtacattagtgaaaggaaactgaagcaatttttaaactttttttaacttttacaattattttatttatttacatcccaaatgatgtcctctccctgtccccactccaagaactctttcccccatacccctctacttcacctctgagatggtgcttacccatccctcttgcctggggcatcaattttttaaaggattaggtgcatcctatcccttcgaggccagaaaagggagtcctctgctatatgtctgccaggagcttgtaattagcctctgtatgctctttggttttgtggcatagtctgcgagctgcaagtggtgagtggtccatgttagttgacactgttggtcttcctatggggttcccattcccctcaacttctttaatacagcccctgacacttccataggtcaactgctggtagagtttattagaggaaagccatgctaggctcctgtctgcaagcacaacatagcatcagtaatagcatcagtgcttggtgaccctccccacctccatgagacagaactcacattgggccagcaactagtcaataattccttcagtctctgctccttttttgtctctgcatttctttcagagaggaacaatttggagtcaaaattttgaagttggtttggttgtcacacccctcctctgggtgtcctattgaactattggacttcaggttcctcttcccaccattgagtattttgcttaaggtcacccacattaaaacctgggagtctctccaccctgggtttctaggattttaagcagtttctgttgattccctgtctctggaaaatttatgtttccacttatttttctggtctgctgggcttctcttccgttttgccccatatctgaccctgccccaccccatgcccccgttatcccttcccctcccttctcccacctaggtaaccccctccctctacctcccatgattattttgcctcatattctaaggtaaatttgaagcatcccacatttgggctttccttcttgtttaacttcttaagctatatgggggaaccccatgggaattctggactttttaactaataccccttaccaatgagtccataccatgaatgtcctttgagtcttggtttctcagtcaaaataatttttcttttctttttatattttgtttactcttttttacactccaaattttattcccctctttgtccaccctccgactgttccacatcacatatgtcctcccttcccctgcccctgccttccatctaggaggatgtcccctacaccccaccccacccccagatctctaaactccctggagcctccagtctcttgaaggttaggtgcatcttctttgattgaacacagacctggaagtctagtgctgtatatttgttgagggtctcatatcagctggtgtatgctaccaggttggtggtacagtgtctgagagatctcaggggtccaggttagttgagacagctggtcttcctatgggaccaccctaatcatcatcttctttcaagcatttccctaattcaaccacatggatcagcatcttctgtccactggttgagtctaatatctgcatctgaattttccagcttcttgttgggtctttcgggtggcagtcatgagaggtccctttttgtgagtgctccatatccttagaattactgtcagaccttatagcctccccttgagctgggtcccaatttgggcctatcaacagatttcctttccctcaggctcttctccatttttgtccctgtagttcttacagataggaacatttctgagttacagtttttttgactgtgggatagcaaccccatccctccactttatcctttctcttcctactggaggtagactctacaagttccctctccccactgtagggcatttcctctaaggtcctgccttttgggacctgagagtctctcatggccaaggtgtctggtaatttatatagggttccctccatcttctacctccagaggttgcttatttccatttttttctgctaacccaaaggacttcagtcctgttttccctgcctccaatatgtgatcatgtcatccttttcactcgctcatccaagtacctctctctcctgactgccccatgattgcatggggtgttcaaatctcctattattattgtgtgaggtgttatgtgtgcttcaagcttcagtaagtttttttttaataactgtatgttgccttgcatttggagaatagatattcaggattaagagttcatcttggtagatttttttcctttgatgaatatgaagtgtctgttcttatcctttttgataacttttggtagaaagttggttttatttgctattagaatgtctactccaacttgtttcttggaaccaaatgcttggaaaattgtttttcagccttttattctgcggtagtatctatctacagtcactagagtgtgtttcctttaggcagcaaaatgctgggtcctctttctctatccagtctgttattggggaattgggtccattggtgttaagagatattaaggaatagtgattgttgttgtgtagctctcttcttttggtttcgttgtaaggagattactttcttgctttttctagggtgtagtttttnntgtggaaatatattgtataaatttggtttggtcatggaatatcttttttctccacctgtgttaatcaaaagttttgctggatatagtagcatggactggcatttgtattctcttagggtttgtatgaaatctgcccagtatcttctggctttcatattctctggtgagaagtctggtgtaactgttttaggtctgtctttatatgttacttgacctttttcacttactgcttttaatattctttcttcgttttgtgcatttggtgttttgtctattacgtgacaggaatttcttttctgttcaaatctatatggaattctgtaggcttcttgtatgtttatgggaatttctttctttaggttagggaagttttcttctataattttgttgaagatattactggccctttatgttgggagtctttggtctcttctatgcctattatccttaggttgatcttctcattgcttcctgaagtttctagaggttttgggttaggagctttttgcattttacattatctttgacatttgtgtcgatgttttctatggtatcttctgcccctgagattctctcttctatctcctgaatctctgttggtgatgcttgcatctatgactcctgatctctttcctaggctttctgtctccctttgtgatttccttattgtttctatttcaatttttaaatcctgaatagttttgctcaattccttcacctgttcggttgtgtttttctgtaactctttaaggaatttttgggtttcctctttaagggcttctgcttgtttacctgcattgtcctgtatttctttatgggagttatttatgcccttcttaaagttctctatcatcaccatgagatgtaattttaaatccaaatcttgcttttccagtgtgtttggacatccagtattttctttggtgggagaacttggctctgatgataccaagtagtctttgtttctgttgctttggttcctgtgcatgcttcttcccatcagtttgtctctgctgttagcttgtcttgctctctctgacagtggtttgaccctcctgtaagctatgtgtcagcattcctgcagacctgtttcctttcagtcagatctgggaagagagagctgttcctggttgtgtgtcctgaagcctccaagagggttgcatggagcagaagagttggttttacctctgttctctggtgtgtcagggctccaggctattggctttcagctctgggctcaggcagaaaccggattgattctgcccctgactattcctaggttcttgtattcagagggctctagacagatttctcttgggacaggaatgtgagcagaagtgggggtcttccctgatctctcaggattgtctgcacttctgagggtccagctgtctccctcacaggatttgggtacagagaactgcaggacctgttcaggaccttgtgcaggcagaaactggtagtggactgtccaagaagacttctgtctttgtgtgtcctgaggccaccaggtgtccacttggagcagaagagttggtcttacctctgctctctggtgtgtcatcactcctgatgactggctttcagttttgggtgcaggcagaaacaggaagagacctgcccctgactgctctaatttcttgtgcccagagagcagaggaggcactagacaggttcctgttgggccaagaatgtgagcagaagtcggggtctcccctgagctctcaggattatctgcacttctgagggtccagctgtctccccgataggatttgggtacagagaactgcaggaccagttcaggtccttgtgcaggcagaaactggaagtgtactgtcccagactgctcctgcctttgtgtgtcctgaggccaccaggcagatttcttggagcagaagagttggccctccctctgctcttagatgtgcaggcgctcctggaaaccgactttcagctctggatacaggcaaaaaccataagtttcctccgctgaatgctcccaggttactgtgcttagaggtcacagagggcactaggaaggttcctgttgggccaggaatgtgagcagaggtgggggtctctcctgagctctcgggattgtctgcacttctgagagtccaattctctctcccacgatatttgggtacagaaatgtgggaccaggtcagccctgggtgcaggtgcctatttctattattcttagatttgatattttcattgtacctggatttcctggatgcttcatgttgcaagatttttatgtcttgacttttctttgacagtgtgtcaatatcttctaaaatatcttctacatctgaaaattctatataatatctcttatattctgttgttgatgctttcatccataattcctgacctcttttctaggttttccaattcaagcactgcctctctttgtgttttctttatagtttctacttccacttttagctcttggaccacattcttcaattgcttcacctgatttctttctttcttttcccccctgtatttctttaaggaatttatttgtttcccctttaaaggcttctacccgtttacctatgttttcctgtttgtctttccatgacttacttctatcctctttaaaggatgctattatcttcatggatagtatattaggtcagcttcctgtttttcaagtttgttgttgcacacaaggcttgctgaagtgagagaattggtttctgatgacgccaaagtatattgacttctgtttcttatggtcttgggcttgcctctagcaaactggtcatctctggtgttagctgttctgggtgtctctgtcttcatcctacttcctatgtccctgggttgctagagttctctgggtaggcttgtgtttctggctgtagctgaccactggtgaagacttcagaatgtgaggtcttaataggggcatgtacactagtgacctgctgccctggctacagagacaatctgctgatctgttgccctgtgtgcagcagatctctttggaggccttcagactgtggggtctgttgctcagtgtgtagcagaattcgcggaggacttcacactggtcagttatcctgcatgtaccagaactcgtgagaggccttcagactgtagtatctttagaggagcagacaagctgatgatctgccattgcagaaggtgcaggatggaaagcattcttgtttgggagggtcccttacttattgccctgtgtgctgcagaactcctgagaggccatcaggctgtgataccttcagaagagcagccaagctggtaggggtcttatttctctttttatttcttgttttggaggagtggttctcaagaatttaacagtggcatgcatttttattacttttgaacacatagtctgagtatgctatctctaatagtttcctaaccatctgttactcaagtcaaccaggctgatattttatataagtagaaactgaacttatcttcaaaatccaattacattttccattttttgtgttttccttaaaaattccttcggagttttctcttacatatattaaatgccacccttttttatttttatttttttcagagtccatgatttatttgtttactctccttcctgggattgccctttcaataaatcccctttctttgcttttcattgttattcatcaattttttcttcttattattttatttacttacattccaaacattggcccccttcccagtaccatatcctcaagttattcattgtccccctttcctttgcttctgagagtgtgctccctgacacacccacctacctacacctcacccctaccagcatcccttctcccctcttttcagatttctacaggatttggctgttcctctcctactgaggtcagataaggcagccctctgccacatatgtaccaggagctatggatcagtccatgaatactcttttgttggtggcttagactctgggatctctgaggtgttctggttatttgatactgttgttctttctgtgataccacaatccccttcagcaccatcaatcctttgcttaactcatccatagacatcccagacctcattcactgttggctgtaaatatttccatctgtttcagtcagctgctaaatagagcctctcatgggacagccatgctgggcttctctctgcaagtacaacatggtgtcaaagtttggtgcctatacatgggatgcatctcaagttgagagggtcactggatgggctttccttcaggctctccacaatttttctccctgtgtttcctttagacaggaacaattcttggtcgaacatttataaggtgactgggtgaccccattcctcaactgggtgccatgtctacctactgttggtctctttaggttccaactcctcacttttggacattctgattaagcttatccccattggatcctaagagccccctctcatatctttgatgtctgagtctttctagggattctccagttcccccaaccattcactggtgcatatttctgttcattcttctggccctctagaattctgtcctgtgtccccccatattttatccagaccttcctcttctccctcctcatcccctctgccattcatgtccctccctccctctgcctcctatgattatttttaacactcttcttatatgcaagttttcacttgaaacacaaatctaattttatgaaaacaaagatcacctactatatagccctaatcttacagttaaatttgtcctactcttaatttttatttttcacttatataatgaattctggtagttattctttagggaggactctctgatggagataaatcccctttatctcttttatctgataatgtctcatcaatgtctttattcaaaaggcaaacaacacaggatatagaacttaaggcttacactcattttcttttccttactatggtctgcatggtgagaggataggagtcactttctttgggatctgggtccagtgtggttgatgatgacttcctactgatttttgtccaagatgttttctttaagcagtttcagtagagagatctccaggagtttcatgggacttgtcctatttgactttactcagttcttgaatatgtacagtcatctattatggagaattgttttcattttccttcatagtaaaacattaattttgcttgaatattgaatattttgtttttacctaaaaatatttgaatttttttcagtttcatgatgttcctcttgaggtcatactgaacataatcagtacttttgatttcatatttttcctgtgtcctcacaagaacaatcagtagtctaaaagaaaaacatataacacaacagtgtgacattagatgagtttggaatttctttgctagaattttcaatgtctcatctcttcatataatgtttactaaaaattctatgtccaagcttttcagatatacctagttaaagtatatcatagatgtctatgcttattttaaccatatcagaaacccagaaaacctcattagccttctgttacattataggctttcaagtcttgttttaaatgtacttatacaaaatgataaagagtgggaatatatacagtcatatactattgagtttcttcaaaaaaaaatgcctatctacattggccatagcacctaatccttctcaggttcagaagctgttaagagatttactactacttgaagttttcaggcagacatgtttgctgtagttaagaaatgtttcaggtgagaaaaaaagaagaacttgtaactctcagtttatatgattaatctttcttcaaataatcatttatacagccagaaatcactaaagacttaatacttaatgtttttggttctgcttgagcctgtagttttacttgatattcaaacattcaaatgttgtctccttagattcaacagggaaatgtgggcctcctccacctattgacaatggagacatcacctccttgtcattaccagtatatgcaccattatcatcagttgaatatcaatgccagaactattatctacttaagggaaataagatagtaacatgtagaaatggaaagtggtctcagccaccaacctgcttacgtaagtaccttattcacatagattataagaaattctgttttatattgtgggtatttttctgtttataatataacattcacaaaataaaagtactgttttgtttgtgtttcagtatcaaacatcagcatgtgataaaacaagattattagattctttttataaaaaatacctgttaaataaaattgtatatattattcttaataattgtttttttctaatatgtattaacatctacaaaactgggtgccagcataacattatataactgttgtctcagtcagtgttctattgttttaaagaggaactatgaccatggcaactcttttaaaagaaaccatttgttgggggttgcttacaattttggaaatttattctactctcaacatgtttgggagcatggtggcacagaggtaaacatgatggtgaagaagtagctaagtattccatatctggctctgcagggagcagaaagtgataggcatacttctaacaagtctatgcaaactcccacaaggccgtagccataatacttcacaagtaccaccattctccaatgaaaaatctgtatgtgtatctatggaggtcattccttttcaaataagcacatctgtatacatcttgcagttattaaatccatacaacatctcctttccttagataaggcaactgacatctattaatcactgttatgcattctaaagtaattctctctgtgagaaagagcacaaagtagttgtctttctgtgttggttatatttgacttaatgtccttcaatgcccttttctaagtaaaataataaaatatatctttaatgacttaatattttacatttaaatataccatgatgtcattataaattcaccaattagtattagttcagctttcttcaccttaccaacttccatgtagcagtttagaataaacatatagatccaggttgagtactttgattttatttcctttgcgtacattccagaagaaacaataggaacaatacataaatatctatttttaaatttgtaagaaatctcaatttttatccatagtaacttcacaaaatcatattcctgtcaatggtttgtgaagtgttcaccacacactaatgagcagttgtaatttttagggctccttcctctggtgctactttaactgagttaaaagatatcttactatggcttttcaatggaatgacagcaatgatatttatgtgtttttcttagaagtatctattcatttatccagatttgatcagcttatttttcctttaaaatgtgctttaccacagactaatatagttcagcgaaaggttatcagcagactggaatatttttcaattatttaagtataatttatgacagatatagtgcaaagccttttcacaatcaatttactaaaaaaggtgttctaacttctaacagaccagcaaggcccaaagcaatgaaatcaaattatataaaaacaaaacaaaagcaaataaatatatttatgcactttgtacgaaatggaggtcacatctttatgctttcttgacccaggacacccccctaaaagatatgtaaatacctaaaaataaagaatagacaaccatatacttcaattaaacttgctgccaatttcttaggtgtattgactatgctctgtgatatgcaccagtaccacaatgggatcaaatccacaggtcaaagtttgctttttgccttgtgatttggagtcccagccaaacacacagtgtcaaaaccatgaaatgtttccctgttgtgcttcctgatactttcagtggtttgttcttatatcaatgtctttgaccaaatttcagttgaatttgcccataatgacaaacagatataaaatttcaatcatcgccatatggatatcaattatcattttatcatttattaaatatgatatcagttcattaacataagttttgggaaagtttattaagatcagtaacctgtagatgcatagatcaattttcaaatcacttttctcattcattggagtcttccgagtgttctggttactgtggggttcctggtgtatattgaaataaagtattatggtatctcctgatttttcctttctgttctagttacagttgtctattcattctattgtagttccatacaagttttagatttttatccctattagtatgaaaaatgttattgatatttcagtgtcagctcacagagtctgctattagccataggatatgtggacatgtctatacctatattaattcttacaacccattaatatacaagctttctctatttctgtcttttcagattattttaccagttaactaatatttttgattgaagttttcacttctgtttataaattcatagctgaattaattttgaagatactgaaaatgacattgcatttatagttaattctcagaaaaatggaatttttctatagaaagggggtgatttctgtaggtttatatattaattgttgaactttggtaatttatctttcagatgcatgtgtgataccagaagatattatggaaaaacataatatagttctcagatggagggaaaatgcaaagatttattcccaatcaggggagaatattgaattcatgtgtaaacctggatatagaaaattcagaggatcacctccgtttcgtacaaagtgcattgagggtcacatcaattatcccacttgtgtataaaatcgctatacaattattagtaaaccttatggatgaacctttgtttagaaatgcacatgtatattactaatacagtttgaatttacatttgaaatattgtttagctcatttcttctaataagtatataaactttttttatatggtggttaatcagtaactttacagactgttgccacaaagcaagaacattgcattcaaaactcctaatccaaaatatgatatgtccaaggacaaactatgtctaagcaagaaaataaatgttagttcttcaatgtctgtttttattcaggacttttcagattttcttggataccttttgttgttaggttctgattcacagtgagtggaagacacactgactctgacttcaaattagtattacttgccaatacataacaaccaaactatcataatatcacaaatgtatacagctaattactgtgtcctacctttgtatcaataaagaaatctaagaaag

SEQ ID NO: 2 - DNA, 4236 bp, Rattus norvegicus
acagcacatacttctcttcgagtcaactgctcccagatagatccaagacatgagactgtcagcaagaattatttggcttatattatggactgtttgtgtagcagaagattgtaaaggtcctcctccaagagaaaattcagaaattctctcaggttcgtggtctgaacaactatattcagaaggcactcaggcaacctacaaatgccgccctggataccgaacacttggtactattgtaaaagtatgcaagaatggagaatgggtaccttctaacccatcaaggatatgtcggaaaaggccatgtgggcatcccggagacacaccctttgggtcctttaggctggcagttggatctgaatttgaatttggtgcaaaggttgtttatacatgtgatgaagggtaccaactcttaggtgaaattgattaccgtgaatgtgatgcagatgggtggaccaatgatattccaatatgtgaagttgtgaagtgcttgccagtgacagaactggagaatggaagaattgtgagtggtgcagccgaaccagaccaggaatattattttggacaggtggtacgctttgaatgcaactccggcttcaagattgaaggacagaaagaaatgcactgctcagaaaatggcctctggagcaatgaaaagccacagtgtgtggaaatttcttgcctgccaccacgagttgaaaatggagatggtatatatctgaaaccagtttacaaggagaatgaaagattccaatataaatgtaagcaaggttttgtgtacaaagaaagaggggatgctgtctgcacgggttctggatggaatcctcagccttcctgtgaagaaatgacatgtttgactccatatattccaaatggtatctacacacctcacaggattaaacacagaattgatgatgaaatcagatatgaatgtaaaaatggcttctatcctgcaacccgatcacctgtttcaaagtgtacaattactggctggatccctgctccaagatgtagcttgaaaccttgtgattttccacaattcaaacatggacgtctgtattatgaagaaagccggagaccctacttcccagtacctataggaaaggagtacagctattactgtgacaacgggtttacaacgccttcacagtcatactgggactaccttcgttgcacagtaaatgggtgggagcctgaagttccatgcctcaggcaatgtattttccattatgtggaatatggagaatctttatactggcaaagaagatatatagagggtcagtctgcaaaagtccagtgtcacagtggctatagtcttccaaatggtcaagatacaatattatgtacagaaaatggctggtcccctcctcccaaatgcgtccgtatcaagacttgttcagtatcagatatagaaattgaaaatgggtttttttctgaatctgattatacatatgctctaaatagaaaaacacggtatagatgtaaacagggatatgtaacaaataccggagaaatatcaggaataattacttgtcttcaagatggatggtcacctcgaccctcatgcattaagtcttgtgatatgcctgtatttgagaatgctatgactaagaataataacacatggtttaaactcaatgacaaattagactatgaatgtcacattggatatgaaaatgaatataaacataccaaaggctctataacatgtacttatgatggatggtctagtacaccctcctgttatgaaagagaatgcagcattcccctgttacaccaagacttagttgtttttcccagagaagtaaaatacaaagttggagattcgttgagtttctcttgccgttcaggacacagagttggagcagatttagtgcaatgctaccactttggatggtcccctaatttcccaacgtgtgaaggccaagtaaaatcatgtgaccaacctcttgaaatcccgaatggggaaataaagggaacaaaaaaagttgaatacagccatggtgacgtggtggaatatgattgcaaacctagatttctactgaagggacccaataaaatccagtgtgttgacgggaagtggacaaccttgccgatatgcgttgagtatgagagaacatgtggagaccttcctgcacttgagcatggctctgtccagttatctgtccctccctaccaccacggagattcagtggagttcacttgtgcagaaaccttcacaatgattgggcatgcagtagttttctgcattagtggaaggtggaccgagcttcctcaatgtgttgcaacagatcaactggagaagtgtaaagccccgaagtcaactggcatagatgcaattcatccaaataagaatgaatttaatcataactttagtgtgagttacagatgtagacaaaagcaggagtatgaacattcaatctgcatcaatggaagatgggatcctgaaccaaactgtacaagaaatgagaaaagattctgccctcctcccccacagattccaaatgcccaagtgattgaaaccacagtgaaatacttggatggagagaaagtatctgttctttgccaagatggttacctaactcagggcccagaagaaatggtgtgtaaacatggaaggtggcagtcgttaccacgctgcacggaaaaaattccatgttcccagccccctaaaattgaacatggatctattaagtcgcccaggtcctcagaagagagagatttaattgagtccagcagttatgaacacggaactacattcagctatgtctgtgatgatggattcaggatatctgaagaaaatagggtaacctgcaacatgggaaaatggagctctctgcctcgttgtgttggaataccttgtggacccccaccttcaattcctcttggtattgtttctcatgaactagaaagttaccaatatggagaggaggttacatacaattgttctgaaggctttggaattgatggaccagcatttattaaatgtgtaggaggacagtggtctgaaccacccaaatgcataaaaactgattgtgacaacttgcccacatttgaaattgccaaaccgacagaaaagaaaaaaaaatcatacaggtcaggagaacaagtgacattcagatgtccacctccgtatcgaatggatggctctgacattgtcacatgtgttaatacgaagtggattggacagccggtatgcaaagataattcctgtgtgaatccaccacatgtgccaaatgctactatactaacaaggcacaagactaaatatccatctggtgacaaagtacgttatgactgtaataaaccttttgaattatttggggaagtggaagtgatgtgccaaaacgggatttggacagaaccaccgaaatgcaaagattcaacagggaaatgtgggcctcctccacctattgacaatggagacatcacctccttgtcattaccagtatatgcaccattatcatcagttgaatatcaatgccagaactattatctacttaagggaaataagatagtaacatgtagaaatggaaagtggtctcagccaccaacctgcttacatgcatgtgtgataccagaagatattatggaaaaacataatatagttctcagatggagggaaaatgcaaagatttattcccaatcaggggagaatattgaattcatgtgtaaacctggatatagaaaattcagaggatcacctccgtttcgtacaaagtgcattgagggtcacatcaattatcccacttgtgtataaaatcgctatacaattattagtaaaccttatggatgaacctttgtttagaaatgcacatgtatattactaatacagtttgaatttacatttgaaatattgtttagctcatttcttctaataagtatataaactttttttatatggtggttaatcagtaactttacagactgttgccacaaagcaagaacattgcattcaaaactcctaatccaaaatatgatatgtccaaggacaaactatgtctaagcaagaaaataaatgttagttcttcaatgtctgtttttattcaggacttttcagattttcttggataccttttgttgttaggttctgattcacagtgagtggaagacacactgactctgacttcaaattagtattacttgccaatacataacaaccaaactatcataatatcacaaatgtatacagctaattactgtgtcctacctttgtatcaataaagaaatctaagaaag

SEQ ID NO: 3 - protein, 1235 aa, Rattus norvegicus
MRLSARIIWLILWTVCVAEDCKGPPPRENSEILSGSWSEQLYSEGTQATYKCRPGYRTLGTIVKVCKNGEWVPSNPSRICRKRPCGHPGDTPFGSFRLAVGSEFEFGAKVVYTCDEGYQLLGEIDYRECDADGWTNDIPICEVVKCLPVTELENGRIVSGAAEPDQEYYFGQVVRFECNSGFKIEGQKEMHCSENGLWSNEKPQCVEISCLPPRVENGDGIYLKPVYKENERFQYKCKQGFVYKERGDAVCTGSGWNPQPSCEEMTCLTPYIPNGIYTPHRIKHRIDDEIRYECKNGFYPATRSPVSKCTITGWIPAPRCSLKPCDFPQFKHGRLYYEESRRPYFPVPIGKEYSYYCDNGFTTPSQSYWDYLRCTVNGWEPEVPCLRQCIFHYVEYGESLYWQRRYIEGQSAKVQCHSGYSLPNGQDTILCTENGWSPPPKCVRIKTCSVSDIEIENGFFSESDYTYALNRKTRYRCKQGYVTNTGEISGIITCLQDGWSPRPSCIKSCDMPVFENAMTKNNNTWFKLNDKLDYECHIGYENEYKHTKGSITCTYDGWSSTPSCYERECSIPLLHQDLVVFPREVKYKVGDSLSFSCRSGHRVGADLVQCYHFGWSPNFPTCEGQVKSCDQPLEIPNGEIKGTKKVEYSHGDVVEYDCKPRFLLKGPNKIQCVDGKWTTLPICVEYERTCGDLPALEHGSVQLSVPPYHHGDSVEFTCAETFTMIGHAVVFCISGRWTELPQCVATDQLEKCKAPKSTGIDAIHPNKNEFNHNFSVSYRCRQKQEYEHSICINGRWDPEPNCTRNEKRFCPPPPQIPNAQVIETTVKYLDGEKVSVLCQDGYLTQGPEEMVCKHGRWQSLPRCTEKIPCSQPPKIEHGSIKSPRSSEERDLIESSSYEHGTTFSYVCDDGFRISEENRVTCNMGKWSSLPRCVGIPCGPPPSIPLGIVSHELESYQYGEEVTYNCSEGFGIDGPAFIKCVGGQWSEPPKCIKTDCDNLPTFEIAKPTEKKKKSYRSGEQVTFRCPPPYRMDGSDIVTCVNTKWIGQPVCKDNSCVNPPHVPNATILTRHKTKYPSGDKVRYDCNKPFELFGEVEVMCQNGIWTEPPKCKDSTGKCGPPPPIDNGDITSLSLPVYAPLSSVEYQCQNYYLLKGNKIVTCRNGKWSQPPTCLHACVIPEDIMEKHNIVLRWRENAKIYSQSGENIEFMCKPGYRKFRGSPPFRTKCIEGHINYPTCV

SEQ ID NO: 4 - DNA, 97328 bp, Artificial Sequence
  Synthetic
  misc_feature (1)..(96): Exon 1
  misc_feature (18013)..(18198): Exon 2
  misc_feature (18494)..(18599): Exon 3
  misc_feature (21021)..(21097): Exon 4
  misc_feature (23223)..(23414): Exon 5
  misc_feature (23849)..(27569): N = A, T, C, or G
  misc_feature (30174)..(30344): Exon 6
  misc_feature (33877)..(34050): Exon 7
  misc_feature (47893)..(48087): Exon 8
  misc_feature (48451)..(48627): Exon 9
  misc_feature (60128)..(60310): Exon 10
  misc_feature (61423)..(61599): Exon 11
  misc_feature (66870)..(67043): Exon 12
  misc_feature (67758)..(67940): Exon 13
  misc_feature (68026)..(68205): Exon 14
  misc_feature (70445)..(70621): Exon 15
  misc_feature (73158)..(73340): Exon 16
  misc_feature (73511)..(73717): Exon 17
  misc_feature (74282)..(74455): Exon 18
  misc_feature (83447)..(83623): Exon 19
  misc_feature (85250)..(85426): Exon 20
  misc_feature (88077)..(88078): N = A, T, C, or G
  misc_feature (93999)..(94181): Exon 21
  misc_feature (96653)..(97328): Exon 22
  misc_feature (96847)..(96849): Stop Codon
cctaaactaactttcaacttccctttggggcaagtctgtctctgctgtaaccacagttcatagcagagaggaactggatggtacagcacatacttcatttgctgataatatttctcatagcaattattcaaattaagtctagaaaatgtgggtaattactagtctgtaactgaatggcttttggtggtaagtttaaaaaccgtgaacctttcacttgactattgtaattgatagttcagcttgatgtaaaactcaagacagtgctttaaacatgtttttgcaatccataattaggcatagacatttaacttgtagttatcaggaaatacaggctcctctttttctcatgagtgtccctgaagtactatatgtaaaactagttagaaatatataaatatccaaagtcaatgaaagcacttacttttttctttaaatgggtggatcgatttcaggcttatttctaaaccttcctaactacatcacttagctgatatttccatggttttaaaagtttcgtatgtaagaccttcaagtatgagataaaaagaaaataaaatttgacatgtaacctgcattggacggatctgatttgtttctggttttgttttctgtgaatacgtgtggggcatgtttgtttctgaagccattttgaagtaggtaatgtgactgtcggagttctttcatgacaataacagggtctgactttattattcacttaaattctcccaagactgcttagtttatccaatgaaagagctttgctttcccagtttaggaagggtacctagttgtgggataaacatttaatcaactcttctttgtgttttgattgtttaagatagggtgtcactacacccttgagctcactgtagtcctcttgtcagcagcttcctatgggctgaggttaccagtgagagtgactgccatgcctgacttagcactttttatataaagtgaatgacataactttaataacttccttaaatgtttctcttagccaatgcattgtaatttgaagctttgctgtaaccactactcagtaaagaatactaaaattatcctctgactggatgtttaccaacccacataagaagagtagatatggtttctcagttgtatcttttactaaaattctgaaaaaaaaatttaagggtattttatactttttgaaagagtaaacattttcaattatattttttaatgttattccttgaattttagcttaagagtcttgtattcagatgccttatagactaaggcagtcatttccttgtatatgaaaatataagtattgctgaaatgaaatgtgattatattggccaggaattctaaagcaatgttgatattaccaagcataactaaactttttattttgttaaaggcaatgttttcatcgcttattttagtgttctacttgaataataatgtttactaagaggtttttaaagatatataagattaaagaaagaactattttatgtttagctaacttttaagtcttaattgatataaatcgaattaaggtgtctacacaattacaaagcagaatttcaatattaaaaaggaagtgccgcgatgtttgcgtgatactttaacgctaatgatttaaaaatcctcatttatgccatggatgtcagctgatttttttgttattgctggatttgaattttcatcagtatgtattcaaatgtggtgccagttcttgctgatgaggtgggcagttacactgtgtccgatactgtttcacagggattttcctttcattcacagatgaaaagagagtttagtttctaaatcattatgtagggtaacctcatggtctccacaaaatgaatgtaaacagatgggagaagtttcatggattttcagtggacacagtactcccactttagtcttagcttggctggtgacccgtgtctatctcaaatgtaaacaatttaatcagtctatcaacttaagaggaatttcagcagaagagcttggatcaattaaaacaattatgtatatgctgcaatgtttgctcctgtttctattctattagatgctggctactaagctgatttaaaaaaaaaaagtttgtgaaatgctctcatattaggctttctgaaacagggaagaaaagatttcataagtattttctgccctgataaagatcaacattcatctaaaaccaatgttagctgggccagcaggaacggtaaacacaataatgatcttgcttggcaaagaacctggctacttgagttcaattcatgggccccacctggtgaaagggggaaaaaaagcctctacagactgtcctccagtttcctcatacaggcatggcaactgtatgttacacccactcaaattaaaagaaaataataaccataacaaaaaatttaaactccactattaataattaaagaataataaccaaaagaagaactatgaacccagcttgtttgcctccctccctccgtgcccctctctctctctctctctctctctctctctctctgccccgcggggccgcccccacagccccctatatccacacccccaagaggggaggggagaaggccgggcgccaccacccccgccccaccaaacaaccccccagaccggccctacccacgcgcggacaaccacaccacgccggcgaacacccaccccccacagccgaaccaagcaacacacaccacaacccgcgaaggggacccgtaaccggccctctctctctctctctctctctctgtcccccccctctccttttccccttttctacttgccaagggctttctcatatctttttagtgcagtgcttgactgtattcacacttctagctgccaagaacagtcaatggtgcttcctgcaaaaccacacgctgatcagaattgggtcagatttacaggacaacctgtaacataagagagttccttggttgagccgtataatttcagttctggggaatggattatacccaagctttccaagcattttactctcacaattgaatattgtatgaaattaggccgcagcccaggattgctgaaatgaaccaattaaacctgtgctgaaacaaaaccaaataaccactgcgtgctttctggggagataagtgttttctaatcctggaggtttaaaggacaaaaaggtcctttcaggcttagagactttaatcatagaatggagaattggtttaattctataatgttttaagtatatgattttttcaaacttagtttaacattgatgtggaaaaattgatgttatatacattaattatgagttaataatagttgctttgggggaaatttagagaaaagttaattattcttttatgtaaaatgatattatattatgtcaaaaagtcaagtgattcaatgtaagatatttatacttttccttaagaaaaagaattaatatggagtgtgtcttacttttcccttcactctgtgtccaaagttgaaagcagctgattctgcagcgttcaccacatcttaactataaaccatgtctacagcttttcctttggccttagccatattgaatatgaaggtttcacatgtcccaagtgactgaatgaagacggatgcagcaagttgcaatacagaagtgatatgtgcgtcactgtgtatgtattgtcacatacagtactgcatacacagagttctgtcagtagtatcactgctgtcctttgtcttcaattactttagttcttcgagatagagtccccctgtttggcccatgctggtccttaaactcctagtcttctggccttagcctccctagtactgaaattcaatatcaagaatatcttatgcagattttctgttgctttcattcaactaaattgacagcaatagctggaccttccttagaaaaatggaaaaatatttaaatatcaaaaccttctaaagaagcaacctatagttctctttttctagacagaaaataaaaaaaaatccaaaaagtaaaggtcaactttaaaacatacatataagtaatattatatatactgatcatgttatatttagaaatatatatgtatatgcatatatgcatataattatagttatgaaaataagtagtcatggggtgaaagaaagtaaaggagataggtgggcagtattggagagacaagaggaaaggggaaatgatgtaattagattataatctaaaaaatataaaagaaataagaataaaaaagaaatggaaattttggtggtaaactaaaaaataacgtgtggatttacaaagagaaaatacatgtctgcatgtcttcaatgctttcattgacacagaaaaccaatttcggtatcttgcttttatgctcctttatcacagcaaaaatttataaacatgtcacaggacaaaccgggacttttaaacctttcttgtatttcaaattataataaatatttggatttattgctgcagtctctactgtgagcataatgtttactttctttctttttttaaaatcataatgttttcaaagccagaagacatctgaaaactctgaagttgactatctttggtatttctttggctttcttgtttgggacaaaactgaaggaattcacaatgtcaaccaaaccacctattgccattaatagtacctacttgcaaagtcctaagtttccattaaccaaacagcacaaaccgaatccattgcagttgtttcgtttctcccattgaggaaaaaaaaacaacatcctcgtagcctcccttttctgaaccttgaaattggaacagtaatctttttcacacacaccatggaggcagtgcatagatagatccccacatttctttaaggaaagtggttggattgaataatcaggtgtgggacagagatgtcaacattgaaattcttccttgagtttgaattttgagaagagtctaaaagaggtcaggttgaaagaacttgcatcctgtttgataaggttcttcacacagtctagcatatttattaagcttctcggttgtactctcccaggccccagaggtcagaggtccatgtatgccaccttctatcacacttgcttaaatccaccctagtagatgcacatgagtattagagatcattatgtaaactagacactagggcactactagtttattacctaaattaggcattaatgtcagtggagcaagtaacctctatccctacaacacatgttttcaggatagaattatatttccctaaatcatgttacttggcattgtgccccaattgtcttcagtgtcttctttcatgcaactcttaaagtatttgacatgtttatcgtaccacaaactcaaccaacctgttatttatgtgtaagggaccacatagttaaatttagtgctattatgtgtaatttactgtgaaatttcactgatagaggatagaactggaaaatggtaagggacaaaatagaccaaagacattctgagacaggaagcttcctaggatgaaatgctgtaacaggtgacaaagggtggagaagttgctcgcaggcagggtgaaggtggtcagtgaaaacaagccttgcttatcatcagcacagtcatgttctaggaatgtgcatgccctttgccaggatgctatttaaaactaaaccatttaagtagtgcaaagcggaatttttctaaggtaggaactgccacagagtaaatagtctgcctctttgtccttagattgctcaattttgaactctctctccccttccaaattaatccatgtttatttcctgactctgattgttagtctttacttcctccttctctctctccttccctcactctctccctcagccctccctccttcctctctctctctctctctctctctctctctctctctccacacacacacacacacacacacacacacacacacacacacacacacacacacacacactacctctacctctcgacatttaggcagatgctgtccaccaaatcctcaaacgctcagttgactgatgttaactttagcttttctcagagcacaaaacatgaaaaacagataaagtaattgggaaaaaaaatgttactttttttttttggtttaaaattagaagaaaaaaaaagtctggttcagataaagtcaagcaactaaacagaaaaaaattccaaccgtgaaataataaaaagaacacacggatttgacagaacacttttgttttgacattttcacttagaaagtctagtttctcacagagtgttaactggaaatgggatagatagaggacgattatagaaacaccccttcaaaggttccgagggaacttttatacttcgagctaaattcaagtgactctagacttcaaaaaccgcaacatagacagatgtgcaaactctgtagagaactttcagtgcatgcaacaggcattcaactccaccagacagtggtgctcttgccactgcctcctcctccttttcctcctcttttttttccctcaagttgtctctttcttttcctttttccaagtcttgtcttttaagtttcccatttgccactctcagctgttggtggccctattgactatatgggtgtacactgtgggaaagttcctacagtcttttttgcgttcgctctctcctctattcacaatcccttttgaataacttttaagtactgcgcaatataatactttccaaaaggttgtcatttagtggagaggaaaagaatgaacagtgtattgaaatattcacatacagtagctcatcttataaactattatgactcagattttaaaaagttcctaaagcagaaaactgaagttgaaaagatgtgctgtatacacaaaatgaatttttgttcagctacaaaaaattatgaaatttataggaaaaattgatgaattcagactcacagggagacaaactctgcatgctctccttcacattttgattctagtttttaatacatatactttatatatactgcatatatctttgtttaatatgacgtgtgtgtgtgtgtgtgtgtgtgtgtgtgtgtgtgtgtgtgacttatggatagaagacatggaactagaagtggaaaaagaaccgtggaggaagggaaccatgaaaaacacaagtggattgaccaagacagaggagggagacagggtagaaaggtgaagagaagaaaataaaactgtttttacaagtcataaaaaaggctggatatggtggcacaccatagtccctgtatgagggaagaaaatacagggcagttctctaagttcaaggccagcttaatctacaaagtgaattcgaggacagtcaggcctacacgaaaaactatgtcttggaagaaaaaaatgcctcactataatataatataaaatataatataatacttcatatattaacttaaaaaataacatgaaataataattggaatgggaaaatgggtcaggaacaggagagggtgagggtgacggtaactggatacagatgttctgctgacttagttctatgttgtttctctgagaaaagtcagacaaagctctcaattcacaatcttctctctccagtatgctcaaaggacaggcatggagcctcaagtagataggctacggatgctgcataggagttagtcagaaagaccaaagaggatgttaacagaaaaacatcagatatacagaaagaactataggttctataaagctgtggggctcatctccacacctacaacttaacttggcttaagtttcacaaggattagtgggaggttaggaaagaaaaagttttcccttttatttatttttgttttgttttgtttttgatttttttaatttatatttcaaatattatcccctttcctggtttccctttcataaaccccctactttatcattttatccccctgccccttcttctatgagggtgttcagccacccaaccacacacaccttcccgcctcccctctctgacattcccctacactaggggggtccagccttggcaggacccaggggttctcctttcactggtggccaacaaggccatcttctgccacatatgcagctggagccataggtctgtctgtgcatactctttggatggtggtttagtccctgggagctctggttggttggtattgttgtttttatggggttacaaaccccttcagctccttgaatcctttctctaactcctccaatggggaccccattctcagttcaatggttggctgctagcatcctctgtatttgtcatgctctggcagagtctctcatgagacagctatattaggctcctgtcagcatgcacttcttgacctcagcaatattgtcgagtttggtgtctgtatgtatatgggctggatccccagttgggacaggttctgaatggccatttcttcagactttgctccaaattttgtctccctatctcctcctatgaatgtttttgttccccctttcaagaagaactgaagcatccgcattttggtcgtctttcttgagtttcatggtggtctatggattgtattttgggtaagctgggcttttgggttaatattcacttttcagtgagtgcataccaggtgtgtgtgtgtgtgtgtgtgtgtgtgtgtgtgtgtgtgtgtgtgtgtatgtgtgtgtgtggttgggttacctcactcaggatgatattttctagttccatccatttacctatgaatgtcatgaagtcattgttttcccttgttctaatccttatcctcggcatcccactgatacctctcatccactccagtactggagctgctaaaacattcagccttagttactccatcttgtggctaaactgctttgtgaggcagccgttcaagcctaatgaaaccgttcaatgtatgctaacagtttattttaaaaagacaatattgaacctggacccttcttggtgttaggagactcttgtgtaaatgctgcctttttcagaaattgacttcaagctgactcctcaggaggcaaaaattccaactactctggtcgatttcactcaggtttagccatatacctgcctattatgatctaggtgcttctcgagggtattagttttataaagaaaatttataattatttctgtatgttttagaaatagaaatttattttccaatgttcattaaatataaccaaaacttaaatttttgtagtttgttttttaaagtactttattgcaatttatatttactttgttcaaaaaaattcaacctaaatattcttgcactatttataaattaatctaaatatttttagtaaacaaaatactctttggatcatatacatgcataaacttaatactcatttatatcaataagaaagcagatgagaaatttaatgaaactaacattcttgctcttcccactttattcttttacttttttctgagtaatgtgtatactccaccatctgctaataaatatatttttaaaatgatgcctctcattctttttccaaaatccttgtagaagctataggaagagaaaaaaagatgacctctccatctttagtctttcaaaagtgtgggtacaactgatgttttacaaaatataaaaattcattaagacttacttcattgcagcaagaacatttcaaagaacaattctgagacatattggcattcggaaaaggaattgcacttggtttgtcagtcctaattctttaaaatctgtatatgaaaaactggtaatcatgattattaaaacagcaaatatttgctttaaagttccatcgattatagttatcttcctcaagtttaagtaaaactcttgttttcagattatcaaacctacacagtcattctgtttctggaaaacattcaagagtggcatttgcatctaagtaaataggaaattaacaaagaaaattcttaaaaagcaaaatcaactatttaattaggattggaccaggtttcatttgttggaatctgagtaaatatttaggtacaagaaaagtgagtttactcattcacctggacatagaagctgtcaacttccccgtgtcttaaaagtcttaagttgaatcacccgtctgaaaatgtgttcatcctttcgaaagcacttctctactccctatgtaagaaccacctgccctgctttcattaacaacttctcatttatttcaagcaaatgtgtttggtgtttggtgtacatttaggttgacagatggagaacatgaatgagcagaacttgttcctgtctagttagaacgcctggacggctactttcagtggaacgtgaaaaaatgtttgccaccctcaagacacacttaactgttattgtcgaaatacagtgaacgattactttaactatttaagccagaacacgagttatggatacacattatgttgagactctaaacaaagacaaacagcaactgaaaacagagggattgtttattttcccgagagcaacaatttttttttttttccgaagaccctggttttggcggtggcagtggtggggtattagcgccacctagtgtggagaagtttaactactgaaatgatgatcaaactaaagctcaaaaaactagcgaaagactcaaaggaaacccgacagcctaaacaattgctctattcttctataaaacatagcagtccttttatttcacatgctgtgtaccatcttgtagatggaagttccaggtgaaatatacgcagtagggtgatccattgctttttaaaagagtagaaaagattagtaaagtagagcgaattgtcataaaatcaagaagtaaaagacatgggcaatttgaacagtatttttagaaataaaatgaataatgagcctagaacctgccatctaagaagcaccatgctgggttttactaacaaccatttaaatatcagggtatttgttacaaagttaagcagcaggcaatattaaatgtgattctatgccttagcactaatgttccatggtcacaattccagcgcctgggagtttaaggcaggaggactatgagatggagaccaacctggtctacaaagattttgtctcaaaaacaataaataggcaaagggaaggatacacggaaggataggtgcacaactactgtagtaaaatgttgattgttggacctgcgtgttagcgtcattggttttttactgtaaaatcaaactttcaaatacattttgaattttctgtaaaaaaaaatgttaagcgaaattcttctctgataaaacttaagaacacagctcaggatctccaatttacttcctatgcccaaacttaagtactagttgaaaaacgcgagccccaaacttaagtccagttcaaaaacacgagccctgttgtctgcacacttatcttctgcttctgccactttcagaaatcttgaaaaagttagtagatatttgaatttccatgtctttacataacaaaaagaagacaatgaaaataaataaagaaatacaatcaagaaacacaaactccccacaaacattttctccctattcttttaattatttgggaatctcatatcatacatatctacaattgcactcatctcctcttctcacatttgcccccttacctgtgagctccctcacccacaaccccgagagagagagagagagagagagagagaggagggaagagcgaaggaagagaagagagagggaagggaagagagagggaagggaagagagagggaagggaaaagggaagtgaagggaaaagggaaaggactagccaaggcaagtattcactgaatcacggtcaaattcctagtggccaagagaggttttttttttttttcctctgcccgcatccttggttgccagaagccaggagctgaggcaagccatgtagtagctggagcagggtaaatctagcaatcccaagcacatgtccctgcctgtactgcagtgctgtgggccagtgaaggacagggccagttctctcagacccatggacatagatagcgtggcttcaggcaacagcagacatcaacgtggtccatggccatatcaggaccactgaccaactaatggccctcaggggatgaatgcatggaccacgagcctccacatggtcttacgccacatcagcatgccccccatctcccgaccccgaggcagcaaagccagacgacatcactaaggtatcacacagcaatatagatctcatacgtccacatggatctcaggtttcttttggggctggtgcaacagcatagaccacagacaccatgatggcccttcaaggaggttgattccagaaagtgaacctttccttgtcttgggcctccattgttgctcataacttggggcatcttgaaactgtgtggcatgttgagggacagggggtggggagtatgggctacatatgatccaagatgataagttatgccaactctactgggcaatgacagcatgttgagcttagccccatctcacacttgtctctagttctgcttctctctctaggcacacacctctccatgtgtgcctagttcacttatgtgttcataatagtagtgctgggtggctttaggtcgactcacagctaccatgtctcaaccggtacttgcttcccattatgtacataacatataaatatatattatatgcatatatgcatatattgtatactacttttaatatattgaaaagtaaaaggaatagaacaaatgctaattttattaactttatatatttaaaatatataacattgtgttctgggtgatgcttgcttcccgttttacatacatatatacacatatatatatatacatatatatgtatatattatatactatccttagtaaacatattgaaaagtaaagggaatagaatacattttgttaactttttgtatttaaaatatgtgacacataccattgaattaattatgaacatagtatattactaattattattcatccataccacaaaacatagaatttccagcacctcagaagatctctgttggtttcttgcatatggaatgaattattttcatagttataggtacatatttgctcttaattgtttcacctcctatatgtgcctatgtgatttgtacaacagcacctcagtgcatggccactgtcaccctacaccactttgtgctggtcaggaagcacagagacactgctctgagggtgagaaagcacagactgagatgtgggagagccagagctggtttgggggtccccaggcctgtggggcctgcaagaaggcagggccccaggttggggacagcatctagctcagggcttgaggagagggcagctctggaccagcagggattgtccttagcttggaagaggaaggcttcttagcagttgtggttgggagtgctgagaagcctgctacaggagacttagctgctgccctgtagagctagttacctggaaagaccaccttcatgacattccccatggtggtggtagatgacagagacagtctgtgtttacccatattgtttattggctgttcattatggaaaatggatgcatacccacttctcagggtctgacctaagattaaatacctttcaacgtctggaatgtctgggaaggaaagcttattggctaagccctccgggcctctaggtaccttattagcacggagaattctgttctgccttacatgacctgtcacatttccttatacggggagtgtggcacaaattccaggtacaaaatactcacattttcaatgatcattttattcacttcagctgattcattctttaaacttcccttatcttgaggatcagtttcctttaacctaaagaactttagtgtacatttataattgttaaagtttctacttcgtttgagaaagtgtcctattccaaagtaaacacagaaatctgaaggttctcatctaacatccacagtgaaagaaaatatgcaaactctccctttggagtctgggatagcttattccacatgatttgtttccaactccacctgcgaatttcctacttttccccactgtgtaaacagaccatatttttgttatccattcttcagctgatagacatcctggctgtttctacttcctggatattgttggtagagcaacaacgatcatgggtgaacagatatctctgtggtagggtatggagttctttgggagtatgtttagaagagtagtatagttatattctatggcagacctgttgctagcttttgggagaaactttactctgattttcataatggctgcagcagtttgcactcccatcagctatgaaaaagttccccctttcctcacattccacactgatatctcttgtcattaatttatttaatcttattcaggctgggagaagatgaaatcacagagtagttttaacttttattccccaaatggctaatgatattaaacatttttaaaagtttctcaattatttttatatcatttccttcattgaaaataaattttgataaaatataatatattttgtttatagtttccccttctccaactcctcccagatccctcttcccaacccacccaaatctataccatttctttctctcatttgtatacaagcaggcgtctaaagacaaataataataataaaacaaaattacataaagtaaaagtcaaacaaactttataagaactctcctgtttttaaaatggcttgttctcattcttgatgctaaggatggcttttagtagagcctgagaaagttgtttggctttttgttatcattgtttttataaatagatactaggaattttatgcaatcattctgattttgagttgataactttagtcatatttggaaaactttaaatgttcaggtgtcatttctgctagttctctcatctacctttgaaccttcagatagatgtagcctgcatcttttgctttctgcacaaaagttggcttctgcagatagttctctttccaccatatttgaacatttctatctcaattttcttcaagtggagtacatttctttctgatttcagatgactgcagatcaaacaatataacaatattatttgtgatattaattcataacattaagataacataatttagagccatttttattttgaacttttaaaattatttttgtctttttcttaaagttcattaaagatgattgacttagttatttaaaatatatttttgctaactaatatctagatcagtgttgattttactgcttatttactcttcatgtctattttcctttttgtattttattttttaattttgtattgttattttacttatttacatttcaaatgtcatcccttttcccagtttccctctacaaactcctatcccattccccttcctcctgcttctatgagggtgctctcccacccacaaacccactcctgcctcaccaccttagcattcccctacactggggtattgagtcttcacaggaccaggggtctcccctcccactaatgccaaataaggcccatcctctcctacatatgcagctggaaccgtgggtccctccatgtatactctttggttggtggtttatgccttgggagctctggggggtgtggttagttgatatggttgttttctatggggttgcatcatgctcagtctgatggttggctgcaagcattggcatctttactggacaggctctggcaaagcctctcgggagacagttatatcaggctcctttcagcatgaatttcttggcttcatcaatattgtctgggtttggtgtctgcatatggatggatccccagttggggcaatctctgaatggtctttcctttagtctctgtgccacgctttgtcttatgtcttggaatatcctctttgtattttaattttcataatagttactatattttatagaaaatatagtgactaaagtttacgttatgcactcatactaagaagaacatttatcccaagactgaacccccagagaactggatggttgggggtggaggggaggatagggaggggaacatccatagagaaggggaggaggaggggttagggggatgttggcccggaaactgggaaagggaataacaattgaaatgtaaataagaaatacccaagttaataaagatgaaaaaaaaatgcttggaaaccatggggggggggaataaacgtctattcttgaaccttaaaaaaatgaagaacatttatctttcttacttcaatcattaatttaattaaattgtatctgggctgcaattttagcttgcattagctcacttctggtctcaaatatttcaaagcaaagaccttcttatgtatgagcttttgcacatgtgtttaagcacaaatctctcctttctaatagactacaataaatctgtcttctttcctgctatcttgagacatgttttatattagacactaaaagactcaaatattctaatgtgttgatgaactcaccagttctgtattttaaggaggactattaatcttgctgtgacttctgtgagactataggaacatccaggcttcacttaggaatcaggtaattccaataagacaactagattcagattctgcatgattcagaatgtttcaggttagacacaccttcaatatacatgtcttatttctaacatcgctaccattcttgaattcacataacccgggaccatcaattcacatacagaactaacacatataagaaatactgtagacctcagatatgaatagtacaggcccattccacctagatttagttcatgaattttcattgctcttaaaatctgtgctaaggcactcttataaatacctccacaccaacttttctgcactccatatttatatagtaggaacataactctgttctatctttttatattatttgaatgttgaatgtctccatatagtttcatgttaacttatatagaccaattttaattcagcaatatggctgctttagcaagggatcacatacaaagactttatctatctagaatgccacacctttaatccctctgggtggaaatagagatatgcccttagtacacacctttaatcccaaaccatgaaagtaaagctagttgttaaaaaaaaaagcaaccatgtgtggatgtaatgtcaaattgaggggcaaagtgatgaatcagagaaagattagacagaatgagttagtaataggatatgcccaactctcacgagaacagacaggaaaaggggatgagatgacttaacagtgcagcagggatggagagagagagagagagagagagagagagagagagagagagagagagagagagagagagagagaagaggaggaggaggagaaggaggaggaggaggaggagaaggaggaggaggaggaggaggaggaggaggaggaggagaggagagacgagacgagacgaggagaggagaggagaggagaggagaggagaggagagaagagaagagaagagaagagaagagaagagaagagaagagaagagaagagaagagaagagaggagaggagaggagaggagaggacaagagaagagaagaggagaagtcctggagcagagacaggttgtaggttaaggcagaatgagccagagaatgagaaggagccaaaagattagaaaaaattgtcagagtttgtttgagatcaagcagaataattcagtgataactcaagagaagtttgaatcagttatgttggaaagaagtttggaccagaacggttgagttgagtcagccagccagagtttcaaaagaactggaaagggtgagcttattcaacagtaagcctgcaagagtacaattatatctggtgaatgagttattttataaccttacttgctttatttttataagtagaaattattctataattcatggcatgagtttagaaaatactgcttagatttgctactaggaaatattttgagaatagtttattttatccatagttttgtttgtttgatttttttgtttgttctttacaacttagaagattgcatagtaaattttcataaagtcgtgcacataaatagctggatggacctgtaattggtatgattcaaagaaaaacaacatgcatattgtttttgaataggtatttcaaatactggtatgtttttattacttgtagattgtaaaggtcctcctccaagagaaaattcagaaattctctcaggttcgtggtctgaacaactatattcagaaggcactcaggcaacctacaaatgccgccctggataccgaacacttggtactattgtaaaagtatgcaagaatggagaatgggtaccttctaacccatcaaggatatgtcggagtaagtacttcatgtttgtaaaacttaagaaaatttcagctttgtactaaatcctttacattgtagcaatataaattatattactactgtaactaaagtgtaatcattttaaaatgtacttgtcctaaaaaaaaaaaaactaaatatggaagcgtgaagttaccttcaattataaaacatgtttttatattttcagtttctcttctattcaatgatatccaaatgtgctttcctgacttctacaaaaggtgtatttcatggaccatacactaatattatcttctttttattttagaaaggccatgtgggcatcccggagacacaccctttgggtcctttaggctggcagttggatctgaatttgaatttggtgcaaaggttgtttatacatgtgatgaagggtatgttgttaatattaaaaggcttatccttgaaaccatgtaggaacgctacaaatttgtactttagcaagaataaattttctattaacatctaaaatgtaatacagaaataaaactacgtcatgaatgcttttaattggatatcatgtgatctccataacactggaaagtaagcaatttatggctgttctgacatagtgttgaaataagggtgtattaagttgctatacacttaatacacaaaaattaagcattcaactcacaagtccttagtacattccactattgtacaatatcgtatgagatgggatagtttttttttttttatattagggacaatgagaattgtgaaaacaactacattatatggtaaccctcttaaagagattttatagtattcaaagaaagcaaaacttttatgtgtgaaaaattctttctcttgaatgctatttttaaagttgtatgcaaattactcttattccataggtgcgaaaggctaatttttcagaatcattgacttccctctctgcacagccactggttcgtcattcactccacagttcttcatttcctatcatacaagaaagttagagttgtaacattattccaaataattataaagaaaagtaaacactttgaatggaatctttttagttgccttttatttcctaacttgagacagtgaactataacggtttattctattcaagttttagaattagctccaaaatatccctatgctcaaatgctcaatgtttgtaacatcttactccgatcccctctcttacagaagcagaaaagtgcttatgagcatcataggattagcaggagaaataaatatgacccacccttgcagcacttcaaaatgatcccagatgaccacaaatacccactagatgctcatttttttatttaacttctccttgtttcacaacgtgaaggagacttttcaaactacaattttcaaggtcactgctgaccttattatttaaagccaacaaagatttctttggcctggatttttcaggttgttccattcttcacctttgaattagctcatcctaggccgtagaaactctctcatttctagtcctataggaaacaccaaatacgactcagcagttgtgacttcagtaggcaagcagacagcacacacaaattggaagctacagactagtccttttggcaggtcaacaccagacccaaaccagcagctgtccaaagctgaaggaaccattgggcttaccaaccatcctgacgtaatactgtggaatctgcaaattgccagaggaacttcaggagaatttcttagagaagcttctcagtggcagcatagtgaagaatagtgagacagagtaaacaaaatcaatgctcagtactcgtctcccactatctgtgtgatcataattatactctgtcgtctagagtcctttcatgtgtgtgccccagcaaaacatcatttgacataacttactttccaaaccgactagaagtttccacttcacttatttacctctgattctggctctcttcaagtcactgttgccaccttgtatttatcaagtgtaaacactgatagaacccatctaggtcaatagctgtgtatattgattctgaatcaccaatatcaaatcaatcaaattactgacaattatcgcgtaaagtcctcataccacgtaggataaaaataggtaaaaagcagttcatattcattcaaatttctgttgatgaatgttctatctatcttgggataattgctttttttaaacccagaagtgaaaggtaaggataggagaggcttatttcaaccctattttttttactcatcctttttagtcctgtgcttttggctaaattttctctgctaaaaataaacaaatataaataaatataaatatagggttttatgtactttgtagtagaatgactccttaggaacaataatgttattgtccaaaaccatcgtgaatgattttgagatgacactgcaaactgattttcccccatatggacaaccattttttttctcctttcccctccctccatgaacagaaatccagtaaggttttgtgtagaattttatagattgtctgaaggaacttagtgtgatggatggatctctgcagtgaataaaaagtctttaccaggagcttcatttcttttctactggaaaagaaattattctgtctcctctacagcaagcatcaaggaaacacttaagtccaatatccaaaactaacatattctattgaagtattttatttccacaaagatttaatagagagatgaaaataataaaagaatgagaaatatttttcccttccaaatctcttactggaggatatccaagactgcacagagcttcaaactacacaaaaacacatgatgtctcaacacaaattattatgcttgcatttttaggtaccaactcttaggtgaaattgattaccgtgaatgtgatgcagatgggtggaccaatgatattccaatatgtgaaggtaaatgaaaaacagatttgtatgtatgcctaaagatctaaaatagataagatttcccaagctgtgtagaaaaatattcttaaagtatatacttaagtatttcatatatttatgtgtgtgtgtgtgtgtgtgtgtgtgtgtatatatatatataattttatataacttcaattctctttttacagtccagtcattatccccctcccagtctgccctcatcccagtcccccaccccatcttaaagaggatgtcctcatccccttcatccctgccccaccagaccttcctactccctggggcttcaagtctcttcaggattaggtgcttttttctcactgaggccagatcaggcagttctctgctacatatgtgttgggaatctcatattcgctggtgtatgctgcctggttggtggcttgtctgagagttctcgagagggtccagattagtctggtcttcctatgaggttgtcctcctcagcttctttcagtttttccctaattcaaccacctgcgtctgactctttcagctgttttttgggcctatcagagggcagccatgttaggctcctgttcttaagtacaccatagcattgataatagtgtcaggccttagagcctcccctcgagatggatcccaatttgggatgattactgagcctcctttccctccctcagtctcttctccatttttgtctctgtagttcttatttatatcttttagtttctagtataaaacataagtactttgttatagtactattttgtatttgtatcaatattctgagaacactaagtctagagaatggtgaatttctcaggactactgtagattccttgaggtcttaggcttgacacacattctcatcaatataacttaaaactatctaaaacataatagatataaatagagattgatatacttttatgatcaaagttctgaatattagaaataccaaagccattttttccattttacatttcaaacactaacaatacataagaccatcactagcctataaaaaaagaccagaatttgaggtatgtttgtgaagaatgacacccctaataacatctagctagttacaggtgtgtaggctatcacatccatacattcctggtagagaatgttattgaaatacctttcacaattatgatgctgtgaaggttttatccatagtcttaattttagaaaaaaaagggggggagggaagcaagaattacaaaagaactcttgcctttcaattcttgctcacatgctgcttataggtagagcaaacagcaagaatgagaaaatgcaggtcttgtttgtaagtttggcgatagcatgtaaataacaaaggtccatccaaatgctgtatcctacttccatgggaagcaataaattagagaaagaagtggagtggaaggagagagggatggagaatgagaaggcacagtaagttctcctaatgagacttttctagtaaggaaatgagaagatgttcccggaacgtctgcatcagaatttacatggtgcttgtttaaaattgatgtttgaggcccctgaatggcctgttgagaaagtatctttgagtgagaagagcagaaaacctcactagcatatccattacatccaaagtttccttcagaaaagcaacttcaaatttcttcatggcggagaaattctaaattaaaaaaaaagtttaaaatttttgagcaatgaggtgaaaaggaaggaaacattacaaaaagtttttttcccctatgagaagaaatatcttcaaaattcattgatttaaaccttattagaatgcaatatcacgttgctttgaagaataaataatacatttgtattagactattccaaaatctcatatgtgttcaccatttaggagacacttgctatcacgaagatgtaaactgtcactctaagtaatagttttcttttcccattcccatagaagctgataagcgaactacccgagctacttagatgttgtgcaaacagtgatgctgaatgtttctcaaacctttaagtcctttccggcaggttgagcaggctgcgtggtgttttcattcatatacgtgtgttttatgtggaagctggtaaggtctgttagtaaaagcgatgcctgtattttcagttgtgaagtgcttgccagtgacagaactggagaatggaagaattgtgagtggtgcagccgaaccagaccaggaatattattttggacaggtggtacgctttgaatgcaactccggcttcaagattgaaggacagaaagaaatgcactgctcagaaaatggcctctggagcaatgaaaagccacagtgtgtgggtaagatacacagatgtgtctgcttcacatattctagtgaaagtatacatttcttttttaaagtacatttttaattataatagaattgcacaactcggatgctaatgaagtatgactgtttccttgtaactgaagttctttgcatgaagccttctattttgctttcagaactatatatttcatgcccttgtgtagtctctttaattgaaatagccaaggtgtccatgcttactgtggcttaatgacttggacaagatgtaaacacaggtgttgcaattcagtctagcctcagcgtctctggtgagtgttgtaaaactaccttgcagagcatatttttttaataaggtttttggaagctaaaggcttggcatgtgtttacaatcacacattatgatgatattttgttttcaatttatagttaggatgtatattttttagaaatctatttgctgcaagnnnnnnnnnnnnnnnnnnnnnnnnnnnnnnnnnnnnnnnnnnnnnnnnnnnnnnnnnnnnnnnnnnnnnnnnnnnnnnnnnnnnnnnnnnnnnnnnnnnnnnnnnnnnnnnnnnnnnnnnnnnnnnnnnnnnnnnnnnnnnnnnnnnnnnnnnnnnnnnnnnnnnnnnnnnnnnnnnnnnnnnnnnnnnnnnnnnnnnnnnnnnnnnnnnnnnnnnnnnnnnnnnnnnnnnnnnnnnnnnnnnnnnnnnnnnnnnnnnnnnnnnnnnnnnnnnnnnnnnnnnnnnnnnnnnnnnnnnnnnnnnnnnnnnnnnnnnnnnnnnnnnnnnnnnnnnnnnnnnnnnnnnnnnnnnnnnnnnnnnnnnnnnnnnnnnnnnnnnnnnnnnnnnnnnnnnnnnnnnnnnnnnnnnnnnnnnnnnnnnnnnnnnnnnnnnnnnnnnnnnnnnnnnnnnnnnnnnnnnnnnnnnnnnnnnnnnnnnnnnnnnnnnnnnnnnnnnnnnnnnnnnnnnnnnnnnnnnnnnnnnnnnnnnnnnnnnnnnnnnnnnnnnnnnnnnnnnnnnnnnnnnnnnnnnnnnnnnnnnnnnnnnnnnnnnnnnnnnnnnnnnnnnnnnnnnnnnnnnnnnnnnnnnnnnnnnnnnnnnnnnnnnnnnnnnnnnnnnnnnnnnnnnnnnnnnnnnnnnnnnnnnnnnnnnnnnnnnnnnnnnnnnnnnnnnnnnnnnnnnnnnnnnnnnnnnnnnnnnnnnnnnnnnnnnnnnnnnnnnnnnnnnnnnnnnnnnnnnnnnnnnnnnnnnnnnnnnnnnnnnnnnnnnnnnnnnnnnnnnnnnnnnnnnnnnnnnnnnnnnnnnnnnnnnnnnnnnnnnnnnnnnnnnnnnnnnnnnnnnnnnnnnnnnnnnnnnnnnnnnnnnnnnnnnnnnnnnnnnnnnnnnnnnnnnnnnnnnnnnnnnnnnnnnnnnnnnnnnnnnnnnnnnnnnnnnnnnnnnnnnnnnnnnnnnnnnnnnnnnnnnnnnnnnnnnnnnnnnnnnnnnnnnnnnnnnnnnnnnnnnnnnnnnnnnnnnnnnnnnnnnnnnnnnnnnnnnnnnnnnnnnnnnnnnnnnnnnnnnnnnnnnnnnnnnnnnnnnnnnnnnnnnnnnnnnnnnnnnnnnnnnnnnnnnnnnnnnnnnnnnnnnnnnnnnnnnnnnnnnnnnnnnnnnnnnnnnnnnnnnnnnnnnnnnnnnnnnnnnnnnnnnnnnnnnnnnnnnnnnnnnnnnnnnnnnnnnnnnnnnnnnnnnnnnnnnnnnnnnnnnnnnnnnnnnnnnnnnnnnnnnnnnnnnnnnnnnnnnnnnnnnnnnnnnnnnnnnnnnnnnnnnnnnnnnnnnnnnnnnnnnnnnnnnnnnnnnnnnnnnnnnnnnnnnnnnnnnnnnnnnnnnnnnnnnnnnnnnnnnnnnnnnnnnnnnnnnnnnnnnnnnnnnnnnnnnnnnnnnnnnnnnnnnnnnnnnnnnnnnnnnnnnnnnnnnnnnnnnnnnnnnnnnnnnnnnnnnnnnnnnnnnnnnnnnnnnnnnnnnnnnnnnnnnnnnnnnnnnnnnnnnnnnnnnnnnnnnnnnnnnnnnnnnnnnnnnnnnnnnnnnnnnnnnnnnnnnnnnnnnnnnnnnnnnnnnnnnnnnnnnnnnnnnnnnnnnnnnnnnnnnnnnnnnnnnnnnnnnnnnnnnnnnnnnnnnnnnnnnnnnnnnnnnnnnnnnnnnnnnnnnnnnnnnnnnnnnnnnnnnnnnnnnnnnnnnnnnnnnnnnnnnnnnnnnnnnnnnnnnnnnnnnnnnnnnnnnnnnnnnnnnnnnnnnnnnnnnnnnnnnnnnnnnnnnnnnnnnnnnnnnnnnnnnnnnnnnnnnnnnnnnnnnnnnnnnnnnnnnnnnnnnnnnnnnnnnnnnnnnnnnnnnnnnnnnnnnnnnnnnnnnnnnnnnnnnnnnnnnnnnnnnnnnnnnnnnnnnnnnnnnnnnnnnnnnnnnnnnnnnnnnnnnnnnnnnnnnnnnnnnnnnnnnnnnnnnnnnnnnnnnnnnnnnnnnnnnnnnnnnnnnnnnnnnnnnnnnnnnnnnnnnnnnnnnnnnnnnnnnnnnnnnnnnnnnnnnnnnnnnnnnnnnnnnnnnnnnnnnnnnnnnnnnnnnnnnnnnnnnnnnnnnnnnnnnnnnnnnnnnnnnnnnnnnnnnnnnnnnnnnnnnnnnnnnnnnnnnnnnnnnnnnnnnnnnnnnnnnnnnnnnnnnnnnnnnnnnnnnnnnnnnnnnnnnnnnnnnnnnnnnnnnnnnnnnnnnnnnnnnnnnnnnnnnnnnnnnnnnnnnnnnnnnnnnnnnnnnnnnnnnnnnnnnnnnnnnnnnnnnnnnnnnnnnnnnnnnnnnnnnnnnnnnnnnnnnnnnnnnnnnnnnnnnnnnnnnnnnnnnnnnnnnnnnnnnnnnnnnnnnnnnnnnnnnnnnnnnnnnnnnnnnnnnnnnnnnnnnnnnnnnnnnnnnnnnnnnnnnnnnnnnnnnnnnnnnnnnnnnnnnnnnnnnnnnnnnnnnnnnnnnnnnnnnnnnnnnnnnnnnnnnnnnnnnnnnnnnnnnnnnnnnnnnnnnnnnnnnnnnnnnnnnnnnnnnnnnnnnnnnnnnnnnnnnnnnnnnnnnnnnnnnnnnnnnnnnnnnnnnnnnnnnnnnnnnnnnnnnnnnnnnnnnnnnnnnnnnnnnnnnnnnnnnnnnnnnnnnnnnnnnnnnnnnnnnnnnnnnnnnnnnnnnnnnnnnnnnnnnnnnnnnnnnnnnnnnnnnnnnnnnnnnnnnnnnnnnnnnnnnnnnnnnnnnnnnnnnnnnnnnnnnnnnnnnnnnnnnnnnnnnnnnnnnnnnnnnnnnnnnnnnnnnnnnnnnnnnnnnnnnnnnnnnnnnnnnnnnnnnnnnnnnnnnnnnnnnnnnnnnnnnnnnnnnnnnnnnnnnnnnnnnnnnnnnnnnnnnnnnnnnnnnnnnnnnnnnnnnnnnnnnnnnnnnnnnnnnnnnnnnnnnnnnnnnnnnnnnnnnnnnnnnnnnnnnnnnnnnnnnnnnnnnnnnnnnnnnnnnnnnnnnnnnnnnnnnnnnnnnnnnnnnnnnnnnnnnnnnnnnnnnnnnnnnnnnnnnnnnnnnnnnnnnnnnnnnnnnnnnnnnnnnnnnnnnnnnnnnnnnnnnnnnnnnnnnnnnnnnnnnnnnnnnnnnnnnnnnnnnnnnnnnnnnnnnnnnnnnnnnnnnnnnnnnnnnnnnnnnnnnnnnnnnnnnnnnnnnnnnnnnnnnnnnnnnnnnnnnnnnnnnnnnnnnnnnnnnnnnnnnnnnnnnnnnnnnnnnnnnnnnnnnnnnnnnnnnnnnnnnnnnnnnnnnnnnnnnnnnnnnnnnnnnnnnnnnnnnnnnnnnnnnnnnnnnnnnnnnnnnnnnnnnnnnnnnnnnnnnnnnnnnnnnnnnnnnnnnnnnnnnnnnnnnnnnnnnnnnnnnnnnnnnnnnnnnnnnnnnnnnnnnnnnnnnnnnnnnnnnnnnnnnnnnnnnnnnnnnnnnnnnnnnnnnnnnnnnnnnnnnnnnnnnnnnnnnnnnnnnnnnnnnnnnnnnnnnnnnnnnnnnnnnnnnnnnnnnnnnnnnnnnnnnnnnnnnnnnnnnnnnnnnnnnnnnnnnnnnnnnnnnnnnnnnnnnnnnnnnnnnnnnnnnnnnnnnnnnnnnnnnnnnnnnnnnnnnnnnnnnnnnnnnnnnnnnnnnnnnnnnnnnnnnnnnnnnnnnnnnngtggcaggggtcctgccgctcctgggccctcccccacgggagcccagaggccttatacagtttcctcttgggccagggatgtgggcaggggtgagcagtgttggtggtctcttccgctctgcagcctcaggagtgcccacctgaccaggcggttgggtctctttctcaccgggtctgggagcagagagctgctgcgggccgggatctgctgcaagttttaattttttttttttttgattcttttttttcggagctggggaccgaacccagggccttgcgcttcctaggtaagcgctctaccactgagctaaatccccagccccgcaagttttaatttttaagacattctaatttttattaatattgttaggataaaatatatacatatacatatatcatacaacacacacagacatacacacatatgtattgcatgtttacaatcagttttaggtatcttaattgaatccactaagcctttgaattttgacaaactgatataatatattgttacttaatatttcttttctttcctcctcctcctcctcctcttcctcttcttcatcttcttcatcttcttcttcttccccttcttcttcttcttcttcttcttcttcttcttcttcttcttcttcttcttcttcttcttcttcttcttcttcttcttcttctagacagcctttcataatgtaatcatggccggcctgaacctgatatgtagtccatatagcttctaccttgcagcaggctccttagagttccgacaagagttttgaaattgcctgcatgtggcactggtcttatactatatttatttttcaatattatctaacacctccattattttcaccattccttagtattgtccaccttagactaaagaagacagtgttttcttcttttcaaatttagtttgcttttgagattataactacatcatttctttcctcaaggattgactagttgctgctaacaactctaacagcactgattcatcatgagaataatgatataccaatatgtatagtcaatgtggcatatatttgacatattgaagtttaatggctgatatcttttggactttaactaattgtctattgctaatgaaacctaggaaattctgatccttgagattatttttaaagtgcacataaggtatattcaggtgaaaataaagaagacaagcatagcagcccccagaaggccatgtggagaaagataaaaaaaaaaaaaaaccagcaaagtatctacagcaagatgtgggcctgagggtcttctgtgcagctcagttcaaccaaaagtatatcacagcagttactactgtttatgtatgcattcggaagacgggagggacctagtcaatatggtcaatttcaaggacttcctgaagcttttgaattgtttacttcctgagcttccttagaggatgggattttttagttccctttagagcaatggttctcaacctgtgaccccctctgaagtcaaacaaacctttcacatgggttgcctaaaaccattgtaaaacacagatattattattaataatagttgcaaaattacagttatgaaatagcaacaaaaataattttatggttatgggatcgccacacaagaggaatggtattaaaggaccaaagcattagggaggttgaaaaccattgctttatctcatcctatttttatgggtgcttctctctgagacggagtcttttatcttaaagaaaattgctattcaacaattgaagagaggtattaggtcagtaagagtatggtatggtcataggccagcacaattcctgcatatgcttgtcataaataactcacctcttcttcagattgactgggaaaagacaaaacatttcaaagtgatcttttaaaagtttccttcgttataaagaaggaaaaatggattaaaaggatggaagaaaatgctttgaaagaccagttactactgccatagtcttagagtagtgtatttgagagaactgtgttaaatgtggttgctaggacttttgaaggtttttttctcccgtttttgtttttgccttttgtttttatggtttgcttgttttgttatttgtgtgtgtgtgtgtgtgtgtgtgtgtgtgtgtgtgtgtgtgtgtgtgttgtgtgtttgtgtgtatggagaaggcaccatgacttttcaaagataaaatgaaaagtgaatctaatggatttccttgaaaagctgtcttgaaaattactgtcagtaatccaaagttgtattattttgaagattattcaatgaaaatattaatctacaaccacgtgtctatttttattttcacaagagtctgagattgttactggctgtcgtttatttcaatttgtcatcatgttcaatataattaatcatatacttttaatttcttccaaaaatgaaaatttgaaatgacagatatatgatcaagagggcagtcaggccaaaacaatgtttgtttggtcactgattttgactgattgacctaatgggaacaaaacactgtcattataaaagtatgttactcagcagatttcctcttatagtaaacactatacaattactcttttgcatttagaaatttcttgcctgccaccacgagttgaaaatggagatggtatatatctgaaaccagtttacaaggagaatgaaagattccaatataaatgtaagcaaggttttgtgtacaaagaaagaggggatgctgtctgcacgggttctggatggaatcctcagccttcctgtgaaggtgacattattcttattttctacgtcttttattatataagaagtagaacagtgaatggaaaagaaagatggtgtcacaaatccatgtttagctgattgcattgagtctaaccatctgttttcatggtgtttatgtatcctagtcagagaagtatctcagtagtcctttggcattaaacctctgcacaagattaactccaggtgtcctcctaaatagaccatttatccactaaaggatcaaactataacccatgatgtagctattttgtattgtcttgtgcttaagaggaacttttcaaacaatcattccagtttcaggtgaatccagttttccatggaagcattaggattcaatagaatagtcatgccacaccaaataacagagcagagcagaatgcctgttctgtactgaattcacctaaagctgaaatgatttttacctagttaaaatctcttccttaacctagatttgttttcaaactgagaaatatatttggttccctaaatgtgcttctacagatgctacatagccttgcttcttttgaaccctaggaaagaggagaggagtgtgagtagagggagagaatagaggaagggaagaaaggaagcagggaatgaaaaagactctccattaaagttcattttgaccatttctcaaacacaaagtcaagtatgaaaagtatagttctgtgttcttgggggtctttttcttcagggaaataggtgacagagggtactctcatctgatagtaaataagcatttgatgatatgaataaagagacctgcatcttaactcatataggcatgcaaatctctaacaatggacttcattttactgaagaaaactttatactcctatatgaaaagtagtttcttattaatgaaaatagtgcatcactctgtacctcagctgatatgtttggccaatgcattgtctttgttttcctggagcagaaaaatagcttacttgtgttgatgtacaattatctggaaattatcagaacactttaatctctctgacaccatatagtggaatacattatttgctgcagctgactttacaagaatcttagactctataagacaccaaaattaaaataagataatataaaaataaataaactttgttccacctgatcataatgtgaacagggggtttaaaacaacttcccagagcatttggatctctagtatatagtagacagtctctaatgacaagcaggaatgatgaaaaataccacaatcttctgaacaatttattttgatgcatctgtttcctgtacagagtagattttgtaaaattgactttccaatgtaagagaactaaacttgaaatatcccattccaaatgtctctactaaataatttgaaataagaaaactgtacatttgggaaaatgtacaagggaaaaaagacactatgcatttgaaaaattaactacatatagtcaatcagacattatcaggggtttatgttggcagcttagggtaatctccaaaagtctttttgttaataagttttacaaagttcttcccatactgtttgcttgtcctcttaaattcttggacatattgttgttgtttgatatcttatagctgtaccttaaaaagatactgagtaaagctgcaatattaagaaaacctaagtagaaaagcataaactacaatggtcctatgaaaacatgacaagcagagtgctgtgaagagaaaaacgatcaaaggaacacaatgttgattcaaaaattgttgttaagtggcataaaagttaggagacatacttgatttgagtagttatcttagggtgaagagacaccatgaccaaaggaatatttaattagggctggcttacaagttcagaggttcagtatactatcgtcaagggggaaagcttggcagcatccaagcaagcatggctttgaagaaggtactgagagttctacatcttgatccaaaggcagtcaggagaagactggcaaagcccaccctaacagttatacatttccttcaacaaggccacacctattccatcaaggacacacttcctaatagtgtcactccctggtccaagtatattcaaaccatgacagtagtcagatattactttagctaagtttttactactatatatgtatattacctgtcttcatgagggaccccagcaactgaagcaaggactgtcgctgactttgttgcctgtctgtggatcctatcccccttgactgggctgccttgtctggcctcagtgagagaggatgtgcctagttttacagtgacttgatataccagaatgggctggtaaccagggggccctccccttttcagaggagaaggggtagaagggatggggcaaggggctatatgtggagagactgaaaggaaagtagagggcttcaatagggataaaatttataaaaaaaagaaatacatatatactgtggcacaaatttaataccagtagaaaggttactgccatactttcaagggctaagtgtacacattagcattatatatggaaaggcaaaaattcaaataacacttaaaaccaaagaattatgtgccagattgagtataagaatgatgaataaatctccagactcttatcataatatttttgttttataagttaaaatattagatttagatggaaaagtatgaatggaggaaagttaatgatagagattgccattttaaaaactggattgccttcaaattctgtatatgagcatgattcatttacctatatggattttgattaaaactacagaattattagcataagagccagactttaattatggaggttatcttgagtgccataaaggacagaagaaaaaagaacactagtgaagaatacatgctcataaaaaccaactataaggcaaaaaagttatttgtgcagaaactgtagctacttaaaaataattttttaaatgtagcaatggtatcaattagaagatctgggttaagatgatttaaggcacataagacataaaatgtacatttgagaaatggcttggtgtttgtgaaggttagattcatgattttgaaagtcaaaaattacactatgtttcttccttgttcagtagattttcccaaataagtcagaggacatgttcaattcaaagagaaagaggtgtaaaatcttcatgaatatttagaattaaggacctgtgaatattaataaataggctcaaatgagaatcaaggccagcaatttcaatgaaagaaatagaaactggatggaaacatgtttcttgcactgaaggtctgtatgatgaagttattatcatctttagaagcataaggtactatatgggacagcatcaagagagaattagtaccagagaggcacacatacaccaggaggagagagaagaagtctgactgatatgcctagcctatgaagatgcattcttttcaatgtctattatatagttatcagtacaaataactggtgtctgccatttagttttaatattcttaacctaaatgagattaaatatttctcattacttatatctgattcttttcagaaatgacatgtttgactccatatattccaaatggtatctacacacctcacaggattaaacacagaattgatgatgaaatcagatatgaatgtaaaaatggcttctatcctgcaacccgatcacctgtttcaaagtgtacaattactggctggatccctgctccaagatgtagctgtaagcttcacttatatctttaatctccatgatcctgaaattagactaataagcatgcatagaagaaaatatagtaatagcaaatatttaattttttatctatgtacaacacttaaaaatattctacttttaaaagtcaagaaaaattaacataatattatattttaatattaaaatttaaaattgcaagtaatatttaaaatacattatagaaaactaaaatttttaatttacttctacttaaatatataggcatctgtacattttttttcttttttttcatttattttttttttattaacttgagtatttcttatttacatttcgagtgctattccctttcccggtttccgggccaacatcaccctaacccctggttgcttggcattgttgttcataagaggtctcgagccccttcaagcttgccagttctttctctgattccttcaacgggggtcccgttctcagttcagtggtttgctgcaggcatttgcctctgtatttgctgtattctggctgtgtctctcaggagagatctatatccggctcttgtctgcctgcacttctttgcttcttgtctaattggatggttgtatatgtatgggccacatgtggggcaggctctgaatgggtgttccttctgtgtctgttttaatctttgcctctctattccctgccaagggtattcttgttccccttttaaagaaggagtgaagcattcacattttgatcatccgtcttgagtttcatttgttctaggcatctagggtaattcaagcatttgggctaatagccacttatcaatgagtgcataccatgtgtgttttctgtgattgggttacctcactcaggatgatattttccagttccctccatttgtctatgaatttcataaagtcattgtttttgatagctgagtaatattccattgtgtagatgtaccacattttctgtatccattcctctgttgaagggcatctgggttctttccagcttctggctattataaataaggctgctatgaacatagtggagcacgtgtcttttttatatgttggggcatcttttgggtatatgcccaagagaggtatagctggatcctcaggcagttcaatgtccaattttctgaggaacctccagattgatttccagaatggttgtaccagtctgcaatcccaccatcaatgcaggagtattcctctttctccacatccttgccatcatttgctgtcacctgagtttttgatcttagccattctcactggagtgaggtgaaatctcagggttgttttgatttgcatttcccttatgactaaagatgttgaacatttctttaggtgtttctcagccattcggcattcctcagctgtgaattctttgtttagctctgaaccccattttttaatagggttatttgtctccctgcggtctaacttcttgagttctttgtatattttggatataagccctctatctgttgtaggattggtaaagatcttttcccaatctgttggttgtcgttttgtcctaaccacagtgtcctttgccttacagaagctttgcagttttatgtgatcccattggttgattcttgatcttagagcataagccattggtgttttgttcaggaaattttttccagtgcgcatgtgttcgagattcttcccaactttttcttctattaggtttgagtgtatctggtttgatgtggaggtccttgatccacttggacttaagcttgtacagagtgataagcatggatcgatctgcattcttctacatgttgacctccagttgaaccagcaccgtttgctgaaaaggctatcttttttccattggatggttttggctcctatgtcaaaaattaagtgcccataggtgtgtgggttcatttctgggtcttcaattctattccattggtctatctgtctgtctctgtaccaataccatgctgtttttatcactattgctctgtaatactgcttgagttcagggatagtgattccccctgaagtccttttattgttgaggatagctttagctatcctgggttttttgttattccagatgaatttgcaaattgttctgtctaactctttgaagaattggattggtattttgatggggattgcattgaatctatagattgcttttggtaaaatggccgtttttactatattaatcctgccaacccatgagcatgggagatctttccatcttctgaggtcttcttcaatttctttcttcagagtcttgaagttcttattgcacagatcttttacttgtttggttaaagtcacactgaggtactttatattatttgggtctattatgaagggtgtcatttccctagtttctttctcggcttgtttctcttttgtgtagaggaaggctactgatttatatgagttaattttatacccagccactttgctgaagttgtttatcagctttagtagttctctggtggaacttttgggatcacttaaatatatatcatatcatctgcacatagtgatattttgacttcttcttttccaatctgtgtccctttgacctccttttgttgtctgattgctctggctagaacttcaagaactatattgaataagtagtgagagagtgggcagctttgtctagtccctgattttagtgggattgcttcacgtttctctccatttagtttaatgttagcaactggtttgctgtatatggcttttactgtatttaggtatgggccttgaattcctattctttccaggacttttatcatgaaggggtgttgaattttgtcaaatgctttctcagcatctaatgaaatgatcatgtggttttgttctttcactttgtttatatattggattacgttgataattttccgtatattaaaccatccctgcatgcctgggatgaagcctacttgatcatggtggatgattgttttgatgtgcttttggattcggtttgccagaattttttgagtatttttgcattgatatttataagggaaattggtctgaagttctctttctttgttgggtctttgggtggtttaggtataagaataattgtggcttcatagaacgaattcagtagcactccatttgtttcaattttgtggaacaatttggatagcatatgaggtcttctatgaaggtctgatagaattctgcactaaacccgtctggacctgtgctctttttggttgggagacctttaatgactgcttctatttccttaggagttatggggttgtttaactggtttatctgttcctgatttaacttcggtacctggtatctgtctaggaaattgtccatttcctgcagattttcaagttttgttgaatatatgcttttatagtaagatctgatgattttttgtatttcctctgaatctgtagttaagtctcctttttcatttctgattttgttaatttggacacactctctgtgtcctctcattagtctggctaatggtttatctatcttgttgattttctcaaaaaaccaacttttggttctgttgattctttctatggtcctttttgtttctactttgttgatttcagctctgagtttgattatttcctgccttctactcctcctgggtgtatttgcttctttttgttctagagcttttaggtgtgctgtcaagctgcttacatatgctctttcctgtttctttctgcaggcactcagagctatgagttttcctcttagctcagctttcattgtgtcccataaggttgggtatgttgtaccttcattttcattaaattctaaaaagtctttaatttctttctttatttcttccttgaccaggttatcgttgagtagagcaatgtgcaacttccacatatatgtgggcgtttttcccttattgttattgaagacagctttaggccgttgcggtctgatagcacgcatgggattatttctatctttctgtacctgttgaggcccgttttttgacccgtttttaaatggtcaattttggagaaagtaccatgaggagctgagaagaatgtatatccttttgctttaggatagaatgttctataaatatctgttaagtccatttggctcatgacttttcatagtctgtctacgtctctgtttaatttctgtttccatgatctgtccattgatgagagtggggtgttgaaatctcctactattattgtgtgaggtgcaatgtgtgttttgagctttactaaggtttcttttacgttttaggtgcccttgtatttggggcatatatgtaggattgagagttcatcttagtggatttttcctttgttgaatatgaagtgtccttccttatcttttttgatgacttttagttggaaattgattttatttgatattagaatggctactccagcttgcttcttccgaccatttgcttgcaaagtttttttccagcctttcactctgaggtaatgtctgtctttgtctctgaggtgtgtttcccgtaggcagcagaatgcagggtcctcgttgcgtatccagtttgttaatctatgtctttttattggggagttgaggccattgatgttgagagatattaagcaatagtgattattgcttcctgttatattcatattttgatatgaggttatgtttgtgtgcttttcttctctttgttttgttgccaagacaattagtttcttgcttcttctagtgtagagtttgcctccttatgttgggctttaccatttattattctttgtagtgctggatatgtagaaagatattgtgtaaatttggttttgtcgtggaatatcttggtttctccatctatgttaattgagtgttttgcaggatacagtaacctgggctggcatttgtgttctcttagggtctgtatgacatctgtccaggatcttctgactttcatagtctctggcgaaaagtctggtgtgattctgataggtctccttttatatgttacttgacctttttcccttactgcttttaatattctttctttattttgtgcgtttggtgttttgactattatgtgacggggggtgtttcttttctggtccaatctatttggagttctgtaggcttcttgtatgcctatgggtatctctttctttaggttagggaagttttcttctatgattttgttgaagatatttactggtcctttgagctgggagtcttcactctcttctatacctattatccttaggtttgatcttctcattgagtcctggatttcctgtatgttttggaccagtaactttttctgctttacattatctttgacagttgagtcgatgatttctatggaatcttctgctcctgagattctctcttctatctcttgtattctgttggtgaagctcgtatctacggctccttgtctcttcttttgtttttctatatccagggttgtttccatgtgttctttcttgattgcttctatttccatttttaattccttcaactgtttgactgcgttttcctggaattctttcagggatttttgtgattcctctctgtatgcttctacttggttatttatgttttcctccatttctctaaaggagttcttcacgtctttcttgaagtcctccagcatcatgatcaaataagattttgaaactagatcttccttttctggtgtgtttggatattccatgtttgctttggtgggagaattgggctctgatgatgccatgtggtcttggtttctgttgcttggattcctgcgtttgcctctcgccatccgattatctctagtgttactttgttctgctatttctgacagtggctagactgtcctataagcctgtgtgtcaggggtgctgtagacctgttttcctgttttctttcagccagttatgggaacagagtgttctgctttcgggcgtgtagtttttcctctctacaggtcttcagctgttcctgtgggcctgtgtcttgagttcaccaggcagctttcttgcagcagaaaatttggtcttacctgtggtcccgaggctcaggtttgctcgtggggtgctgtccaggggctctctgcagcggcagcaaccaggaagatctgcgccgccctttacaggagtttccgtgcaccagggttccagatggcgtttggtgttttcctctggaatcagtaatgtgggcagagtgcagtctcttctggtttcccaggcatgtctgcctctctgaaggtttagctctccctcccatgggatttgggtgcagagaactgtttatctggtcggttccttcaggttctggtggtgtcttagacgcaggggacctgctgctgctgtgcccttatccaagggaacgcagaggccgtatacagtttcctcttgggccagggatgtgggttaagggtgggcagcgttggtggtctcttctgctctgcagtctcaggagtgcccacctgtccaggtggtgaggtctctctcccatggggtttgggagcagcgagctgctgcgggcagggatccgcgggttttcatctgtacactttttaactaaacattttctaagaattgtatgaaattaataggtaagagacgcaggggacctgctgctgctgtgcccttatccaagggaacgcagaggccgtatacagtttcctcttgggccagggatgtgggttaagggtgggcagcgttggtggtctcttctgctctgcagtctcaggagtgcccacctgtccaggtggtgaggtctctctcccatggggtttgggagcagcgagctgctgcgggcagggatccgcgggttttcatctgtacactttttaactaaacattttctaagaattgtatgaaattaataggtaagaatattgtcaggtaagaactgattttacttatttatttacatcatagtaaatatccttcaatagtatttgcctcatagcaaacctttgtcatccctccatttttgttagccacatttgaagataacttggctgctggctgcatgagtgtggtgctgtcagacattgtcttggctcttagtcatcaggagactttgctgggctgtaggccatatgttcaacataccacattcactaggatttggcaagagggttcaattccttatcagataagcctgtggatagattgattcacaaaattgattcttgccttagagttactgatcaaagagacattggggggcctagaatccatccataacctacctataccatacaatgtttttgctatggctgtttcttgtatactgggttcaatatgcatatgaagaaggaaattatgtttatctgtagagagttgctttgaatgatgtcggtggcttctcaacacatgcataccacagtgttatttgagtcaagaatatttaattcctggaatattccattcttttcagatttttgtctatctacatccatatatttttcttttatctaacagtctatgttaaatgtttatcatacgtaaccctgatatcccctaaggaataaagtgtatgacagataagcagccaaggatctcttcctactcatctttctgttgtgatgttaatattactgaattaactacttagaagaagaatttattttgttttgctgacttgaattcatggtcaagttgttctgtcattttcatcctgttactaggaggttatttatgttagggaatgagtggtaagtctaagctgcttggcttatgaccaccagcaagtagagatataagagaatgaccaagatctcaatatccccttcaaaggcatagtcccaatgacctaatttatttcactgtgtccagaaattctgaaatttataaccttcctaatagcaccagcaatgacaaaccaagcttttaactaaggtgaaattctaggaaatctataatatccaactcaaaagaatgaaagaagctatttacactaagaaatagtattgataaatatagtaattgtataaaaattgaatttttaaaaatattaaaatttagatttcttacaaattatttttcttacttttattggtcctatttatttatttattatttgtttttgtcattaggttgttttttataaaatttattctctcatatattacatcctgattgcagtttcttttcccttaatgtcccaactcctccatcccctcaacctcattcctccccatccactcctcctttatttcccttcagaaaatagggggaccctcagggaaatcaactgattattccatatcagatttcaatgtgtcagtacaaggcaccccagtatgaggacaagggtccccaaaataggcaaaagaatcaggaacaactgcaactctctctgttaggaattccacaaaacaccaggcttcacaactataacaaatatacagagggtcaaggttagatccaggctctctgattgtcagttgaatctcagtaaaaccctgagtccaggtgagttgactctgtgagttttcttgtggtgtccttggctgctctgctcctataatctttcttctctaacttcaacaggattccccaaactctaaactaaaggtcagtggaaaagtaccttttcttctcctgagtaattgcttcaaagcctctgctaacctaggcctagttctttaatctttctctagcctctgtataatcttatctaggtcaagaatgtttacagtttttgaaacttacttgtgaataagatcacatcgtcctatttctttctgaactctggctggcttgttcagctcaactgttctggcttaaactcctctgcaaactgtttcaaactgacttctttttcagcctttgacttggtgctatgcttggcctcagattaaccctggcaatctgttttaatcctccgactccttcttattctctggcttctcttacctttacttgtgactagcttgttctctctctgcagcttgtactggtaaaactgcccctccctcacctctttctctgtgctgccctctcgtaaagaggtagcctctttctctctgttctcatgagagttgggcatatcttattctgttaaatctttctctgatttaacatctctttcaaacaagggtgattccttctacaaaataactttaccttcattgttttggattaaagccctttgtagtgttactaaggacttgtctgtattccagccagaaggattaaaggtatatgctgaggctgcgccacaccacagctaaaaacaggtttttcttgtaaacaacacaatcttggatttcacagtgttaccaaaagtcctaaaacagtttgaatctctgcatctgtttctattagttgtggagtagagcctctcctatgatgactgggctaggcaccaatctataagtacagcagagtatcattaggcatcattgaattgacttttttttctttgccagtcatggttggttctattctaggtctctgggccgtacagcctctggtttctggtcctcaagtcagtgtcaggcatgggtttcaagctgtacctgtcattagttagtcactttcacaatttctgtgccaccttcaccccagcacatcatacaggtgagacaaattgtaggttgaaggttttatgtctggtttggtgtcccaaaacctttgtagggttatgtccctgttttcattactgactttgttagtttttatatttaatctgtctttcagttagtttggctaagggtttgtctatcctgtagattttctcaaaagaccaactcttcttttcatagattctttgtattgttctctttgtttctattttattgatcttagccttataatgtttcttagccccaagttggtttatttcctgctctctactcctcttccagagctttcaggtgtgctgttaagtcacgagtataagatctctctaatttctttatgaaggcacttagtgctatgtagtttcttcttaacaccacttttattgtgtcccatacgtttggtatgttgtgccttcattttcattgaatactagaagccttaaattctttatttcttccttgacccagtggtcgttcagtaaagaactgttcagtttccatgagtttatggagtttatgttattgttcaagctcagctttaatccatgtattctgaaaaaatacagggggttatttcatttttcttgtatctgttgagactcgctttgtgacggagtatatggtcagttttagataaagtactgtgagatgttgagacaaaggtgtattcttttgtctttgggtgaaatgttttatagatttctgttaagtccatttgattcataatgtcttccagttccatttttctgttccttttttgtttggatgacatgtccattggtaagagtggggtatggaagtcttccactattaatgtatggtgttcaagatatgttatgaaatatttttgttagttagtttgttttatgatttttatgattgcggtttcccttgcatttggggcagatgttcagaactgagaggttatactcatgaaatattctttttgattagtatgacgtttcctttgtaccactaatgattaattggtttgaataatattttgttaaatattggaatggctacatgatcttgattctttggtccatttgctagggaaatcttttctagccttttattattaagtaatatccacttctgatgttgaggtatatttcctgtatgcagaagaagggtggatactgttctcacatccattttgtgaaacctgtgccatttttattggagaattgaatccattgatactgagagctatcaatgactaatgattgttcattcctattattttgatggtggtggtggcagtgtttgtgtttgagtgtgtgtgtgtgtgtgtgtgtgtgtgtgtgtgtatgtctttttttgctcatatgagattgtttattgcctgtggtgtagatgatctttttgtgttagggtacaagttatttatttcttgggtgtagttgatctccttgggttggaattttctttctagtaattttttttgtagggcttggctgtggatagatattgtttaaacttggctttctcatggtatatcgtgttttctcctactcttattgagtattttgctgactacttcagtcaggatgcaactgtgattgttcagaatgcccaggcccttcttgctttcagagttttcactaagaagtcaactatattctgatagctttgcctttgtatttcacttgcttttttcctttcacatctttcactaatcattatttgttttgaatatttagtattttgattactgttttgacaggacttcattttctttttccatctagttggtgttctataagcttcttgtgcttttatacgcatctccttctttaggacctttttcttttattattttgttgaaaatattttctgggccttctaaaatttattccttgtaagtttcacaagcacctgatcccattcttctttccattcttccatatctactcttttcccttgtaaatgttcccccaaaacaaaacaaataaaaacaaaccaacaaacaaatagacatcttgtcaaggtagctataggcattgcagtgtgtcacacagggacaaaaatctcttttgtccaaacagctttacttgcagatattcatcgcatttagtcatttctttggttcaagatctctggcttctagtacaccacaatacattctgaatattttatctttcacattgctccaactcgataaacaacacatcatccatatctgtcctttccccagaatcataattttgagtgtttttgtatgatgcatttggcttaactcaggaaatatgtggaccacttgaattggagctgtattttcgaacctgatttactcacgagtgggtatatacctgaaagcactgactccctatgtttctgaatctattagcgtaaaatagttccaaggtgagggccaaggttccctatgatcttactacagtcatgcctggatatgagggcccattcttaagaggtgtctgtaattgttgagagtttgtgattttaatgataatgtttttgttcagaagatatcatagtcttaatcactctagctcttagaacctatgtgctccttcattcacaggttgcttgtaggggatagtgctcctgttttgtttaacacttcacaatacactcactatttctagtaccttgtgtattactacatctatagttttattataatttaccagaaaaaagagtcttctctgatgttgacagtgttattagctatgaatataaacatagttacttataaggttgctcagtgttaagtcaatgtattttaatagcagaattaatatgtgtgtctgcactcagatcttatgacatccttgccatgggcttttaagtaggtttacaaatacaagcctgggatctgtgtagcgcaatgagtcacaaacccaactatgtttgagtttccccaatgtagatttacccaaatatatctgggctgcttgtaacttaaatatatatgaatttcgtttattctacactgaactttctgatacttcctggataagataaaaatgattaatctctctgtaatgtcattaaataactttttctacttaaaatctttagtactcactcctaagggatgtttaattactcaccactttcatcaaatcttttactatttgggagaaaatgcattgtaaaatgataactggcacaattcagaagatggtgattgtgaatctgtgttagaagtgattctagaaattaatcttttgtgtcatgttgaagatgtagtaggatgagatttatcaataaaaattagaagatcttgggattgaagatcagtaaaaactggaatatcttgcgctgtgttcataatatttagaacagttgtaaaactggtcaatatattgatcagcagtctgagtagagtgcatcaacactgtgatgtatggtccaggaatcactgctgatgcagccacgacctgcatctggaaagtgtaagatgttaaacaaagctcacttaggtactgaccacctcaggtgtctgttactttaaggagtattatgtttgcttcaagaaccatgtataacggagtaaacctgtgcccactggagaatgaagaataggtaaaagtctgaggtctgtggtaataatgatactcctactctgaaccatgctttctttcattacttttcaaaacaaaatctcagtgagctaatttgacttattgatgtcctatgagaagtgtgattcttaaaattgttaaagaagaacaatttttaaaccatgtaaaaatgtgtaaaaaaactcttgaaatatttaataaaacaaaaactaaaatgaatgaggaagcttgaggaaatttgtttgattttttatgtatttgttgaaataacttttaatgtattgcatgaggttccttgaagcagaatcatacttaatataaaagggatattattctcatactaaagtacaaatgataaatagtaatcacaaataattacatgtaataaagtaatcatatattacatataaacttaatataatgaacaatatggcatttcaatacaaaggtacaaaaatagctccatatcgttccatgttcatactatattttagtttcagtgaaaattataaataagaaattatattgaatattaacaagtatctccaatccaattatctggtggagtatcagctacaacttgacttcatgttgaaagacatcctcacaaaccactgttgtcttttgttttattttcttatcccacacattcactgttctgtcattctgttattttgattagtttaaagtaatttactgatcaagagttttttttcctctgatatgagtgttttatggttgttttattttattatttttttctttcaagtgaaaccttgtgattttccacaattcaaacatggacgtctgtattatgaagaaagccggagaccctacttcccagtacctataggaaaggagtacagctattactgtgacaacgggtttacaacgccttcacagtcatactgggactaccttcgttgcacagtaaatgggtgggagcctgaagttccatgcctcagtaagccaatgcctttatagttaactatgttgattcttttaaagagagagcacatacataattaagttattcataacaaaaataagaccaacaaaagaatttgtgagcaaaatggctagtttctgttatgaaatgtttcttcatgaaacatgcaatagggactatggaaatatctttatcacttgcatattttatttttacaaacgaaagataaatgctattctcttaaatgtttgttattaattttatttttgaatgatgtgcatactcattaaacagttttaaagataacatttatcttagtttatttttaaacaaattaaagattttatttttttaatttttaattattatgtttcttagggcaatgtattttccattatgtggaatatggagaatctttatactggcaaagaagatatatagagggtcagtctgcaaaagtccagtgtcacagtggctatagtcttccaaatggtcaagatacaatattatgtacagaaaatggctggtcccctcctcccaaatgcgtccgtatcagtaagtaactaatacttagatcgcaagaagatcgtgactctctgtcccatctgtatttgtttttattggctaatttttatgtacatttcaaatgttattctttttcctggtttcccatacataagccccctatccaatccccctcacacttctttgagggtgttccccttccccaagaacccatcctttcccacttccctaccctgacattcccctactaatacttagatcgcaagaagatcgtgactctctgtcccatctgtatttgtttttattggctaatttttatgtacatttcaaatgttattctttttcctggtttcccatacataagccccctatccaatccccctcacacttctttgagggtgttccccttccccaagaacccatcctttcccacttccctaccctgacattcccctacactggagggcccagccttagcaaaaccaaggacttctcccctcattggtgcccaacaaagccatccttgttatatacagctacatatgcatctggagccatgagtctgtccaaatgtcctctttgggcagttgtttagaccttgggaactctggttggttggtagtgttgttcttatggggttttaagacccttcagctccttcaatccttcctctaattcctccagtgaggaccccattctcagttcaatggttggctgctagcattctcctctgtatttgtcacactctggttgagcctctcaggagacaactatatcatgttcctgtcagcatgcacttcttggctccatcaatattgtctaggtttagtatgcatgtgtgtttatatatatatatatgtatatatacaggtgtagtatgcataagtatatatgtatatgtctatgtttatttgttggatccccaggtggatcaggctctgaatgtccattccttcagtgtctgctccaaacttggtctcaatatctcttcctacaaattttcttctattagttcgagagtatctagcttcatgtggaggttcttgactaactttgacttaaggatttttgcagggtgatgaaaatgggtcgatttgcgttcttctacatgctgacctccaggataaccagcaccatctggtgattccactgaatgattttagttcctttgtcaaatattaagtgaccacaggtgtgtgagttcatttttgggtcttcaattctactccaatgatctacttgcttgtctctgtatcattattgctctgtaaaacagcttgaggtcatggatgagattaccaaagaaccttttttattattgaggatagttttcactatcttggatttttttgttagtccaaatgaatttgcaaattgctctttctatgtctatgaagaatttagttgggattttgatagggattgcattgaatttgtagattgcttttggcaaaatggccatttttactgtattaatccccccaaaccacaagcatgggaaggttctccatcttctgagatctttgatttctttcttcagagacttgaagtaattgtaagatctttcacttgtttgagtagagtcacaacaaggtattgtacgtaacttgtgaccattgtgaagggtgtcatttccctaatttctttttcagcctggttatcctttgagtagaggaagggtactaatttatttgagttaaatttatacccagccaatttgctgaagttatcatgcttagtagtttgctgatggaacttttggggtcacttaaggatagtattatatcatctgcaaatagtgatattttgactcttcctttccaatttgtatcccattgaccttttgttgtttgattgctctgaccaaaactttgagtactatattgaataagtagggagagagtgggcagccttgtctagtccctgattttagtgggattgcttcaagtttctctccatatagtttgatgttggctactggtttgctgtatattgcttttaatatgtttgggtatcggccttgaattcctgatctttctacggcttctatcatgaaggggtgttgaattttgtcaaatgctttctcagcatctaatgaaatgatcacatggtttttttctttgagtttgttaatatagaggattacgttgatgaatttctgtattttgaaccatccctgcatccctgagatgatgcctacttgatcatgagggacgattattttgatgtgttcttggattctattgacaagaattttattgagtatttttgcatcaatattcataagggaaattggtctgaagttgtctttctttgttgggtctttctgtggtttaggtattagtgtaattgtgacttcatagaaggaattcggtagtgccctgtttctcttttgtggaatagcttggaaagtgtgaatatgaggtcttctatgaaggtctgatagaattctgcacctaactcatctggtcctgggccctttttttcttaggagacctttaataactgcttctatttctttaggagttatggggttgtttagatggtttatctgttcctgatttaacattatacatggtatttgtctagaaaattgtccatttcctcgatattgaatataggcttttgtagtaggatctgatgatttttttaatttcctcagattctttcgttatgtctccattttcatcttgaattttgttaattggaaatactctctgtgacctctggtttatctggctaagggtttatctatctggttgattttctcaaagaactatctcctggttttgttgattcttttttttttcttccttttattgaatatatttttttcagagggaaaatgtttattagtttcatagttttatacctttcagcttattttaacttggtctctggagcatttggaagactagctgcttacatcagagcagtgctgaaatagagacaactataaatccagagacaaacatagccttcaaagttatttagccctacttctaaacagatagtctataatatttattctcaataactgtaaagaaacttatattctccccctcccacaaaacatcactgaaagacgaaagaattggttccatgtatgaccttcttgtttgaccagtggcttcattagggtcatttacaggagcatgccaagaagttacttaaaagaatagtaatgattcaactgaagtttcattaaagatatgtctcatcacagaatgcttttcaattcataaatcacctctagaatgctatccacaccatcgagaatcctgtgatctcctctcaatctataataacatattggcttggggagggtttatgaaagaatagtggggtgtgtgtgtgtgtgagtgtgtgtgtgtgtgtgtgtgtgagacaaaaaaattgatttaaagttaacttctaagtcccagctaacaaccaatgttctgatcagagagctttcagaatagactctattttctctatattctgctccaaacaactttcctgatggctgtctttctataagtagtttgctttgcatgacacagctttctcttactattcctttttttttttaacttaagtatttcttatttacaattcgagtgttattccttttcccggtttctgggccgacatcccctaacccctccccctccccttctttatgagtgttcccctccccatcctccccccattgctgccctccccccaacaatcacgtttgctgggggttcagtcttagcagtccccttccacaggtgatcttactaggatattcattgctacctatgaggtcagagtccagggtcagtccatgtagagtctttaggtagtggcttagtccctggaagctctggttgcttggcattgttgtacatatggggtctcgagccccttcaaggtcttccacttctttctctgattgcttcaacgggggtcctattctccattcagtggtttgctgctggcattcacctctgttttagctgtattctggctgtgtgtctctcaggagagatctacatccggctcctgtctgcctacacttctttgcttcatccatcttgtctaattgggtggctgtatatgtataggccacatgtggggcaggctctgaatgggtattccttctgtcactgttttaatctttgcctccctattcgctgccaagggtattcttgttccccttttaaagaaggagtgaagcattcacattttgatcatccatcttgagtttcttgtgttctatgcatctagggtaattcaagcatttgagctaatagccacttatcaatgagtgcataccatgtgtgtttttctgtgaatgggttacgtcattcacgatgatattttcctgatccatccatttgcctatgaatttcataaatgcattgtttttgatagctgagtaatattccattgtgtagatgtaccacattttttctgtatccattcctctgttgaagggcatctgggttctttccagcttctggctaatataaataaggctgctatgaacatagtagagcacaagtctttttatatatccgggcatcttttcggtatatgcccaagagaggtataactggatcctcaggtagttcaatgtccaatattgtgaggaacctccagactgatttccagaatggttttaccagtctgcaatcccaccaacaatggaggagtgttcctctttctccacatgctcaccagcatttgttgtcacctgagattttgatcttagccattctcactggtgtgaggtgaaatctcagggttgttttgatttgcatttcccttatgactaaagatgttgaacatttctttaggtgtttctcagccattcggcattcctcagctgtgaattctttgtttagttctgaaccccattttttaataagattatttgtctccctgcggtctaatttcttgagttctttgtatattttggatataaggcctctatctgttgtatgattggtaaagatcttttcccaatctgttggttgccgttttgtcctaaccacagtgtcctttgccttacagaagctttgcagttttatgagatcccatttgtcgattcttgatcttagagtataagccattggtgttttgttcaggaaatgttttccagtgcccatgtgttccagatgcttccctagtttttcttctattagttagagtgtatctggtttgatgtggaggtccttgatccacttggacttaaggtttgtacagggtgataagcatggattgatctgcattcttctacatgttgacctccagttgaaccagcaccatttgctgaaaatgctatcttttttccattggatggttttggctcctttgtcaaaaatcaagtgcccataggtgtttgggttcatttctgggtcttcaattctgttccattggtctatctgtctgtctctgtaccaataccatgcagtttttatcactattgctctgtaatactgcttgagttcagggaaagtgattccccctgaagtcctattattgttgaggttagttttagctatcctgggttttttgttattccagatgaacttgcaaattgttctgtctaactctttgaagaaatggattggtattttgatggggattgcattgaatctgtagatcgcttttggtaaaatggccattttgctatataaatcctaccaatccatgagcctgggagatctttccatcttctgaggtcttcttcaatttctttcttcagagtcttgaagttcttattgtacagatcttttacttgcttggttaaagtcacactgaggtattttatattatttgggtctattatgaagggtgtcatttccctaatttctttctcagcttgtttctcttttatgtagaggaaggctactgatttatttgagttaattttatacccagccactttgctgaagttgtttatcagctttagtagatctctggtggaactcttgggatcacttaaatatattatcatatcatctgcaaatagtgatattttgacttcttcttatccaatcggtatccccttgatctccttttgttgtctgattgctctggctagaacttcaagaactatattgaataagtagggagagagtgggcagccttgtttagtccctgatttcagtgtgattgcttcaagtttctctccatttagtttaatgttagcaactggtttgccgtatatagcttttactatgtttaggtatgggccttgaattcctattctttccaggacttttatcatgaaggggtgttgaattttgtcaaatgctttcccaggatctaatgagatgatcatgttgttttgttctttcagtttgtttatataatggatcacgttgatggttttccgtatattaaaccatccctgcatgcctgggatgaagcctacttgatcatggtggatgattgttttgatgtgctcttgaattcggtttgccagaattttttgagtatttttgcgttgatatttataagggaaattggtctgaagttctctttctttcttgggtctttgtgcggtttaggtataaaagtaattgtggcttcatagaaggaattcggtagtgctccatctgtttcaattttgtggaatagtttggatagtattagtttgaggtcttctatgagggtctgatagaattctgcactaaacccggctggacctgggctctttttcgttgggatacctttattgactgcttctatttccttaggagttatggggttgtttaactggtttatatgttcctgatttaacttcagtacctggtatttgtctaggaaattgtccaagtgtttcttttctggtccaatctatttggagttctgtaggcttcttgtatgcttatgggtatctctttctttaggttagggaagttttcttctatgattttgttgaagatatttactggtcctttgagttgggagtcttcactctcttctattcctattatccttaggtttgatcttctcattgagtcctggatttcctgtatgttttggaccagtagctttttctgctttacattatctttcacagttgagtcgatagttttctatagaatcttctgctcctgagatcctctcttctatctcttgtattctgttggtgaagctcgtatctacggctccttgtctcttcttttggttttctatatccattgttgtttccatgtgttctttcttgattgcttctatttccatttttaattccttcaactgtttgattgtgttttcctggaattctttcagggatttttgtgattcctctctgtaggcttctacttctttatgttttcctgcatttctctaagggagctcttcatgtctttcttgaagtcctccagcatcgtgatcaaatatgattttgaaactagatcttgcttttctggtgtgcttggatattctgtgtttgctttgttgggagaattgggctctgatgatgccatgtactcttggtttctgttgcttgggttcctgcgcttacctatcgccatcagattatctctagtgttactttgttcttctatttctgacagtggctagactgtccttataagcctgtgtgtcaggaatgctgtagacctgttttcctcttttctttcagcaagttatgggaacagagtcttctgctttcggccgtgtagtctttcctgtctactggtcttcagctgttcctgtgggcgtgtgtcctgagtccattaggcaggtcacttggagccgaaaagttggtcttgcctctggtcttgggccaaaatttgctttccgtgagggctgcaatcaaagggcttgctcagccttctctcaggcctagatggcactagaacttttcctctagagtcagaaatatgggcagagagtagtctcctctggtttcccaggtttgtctgcccctctgaaggtctagctctcccttccatgggatttgaatacagggagctgtttgaccgggtcccttcagaactgggcgcagtctggaacctagcgctcctgcagcttgagtgaccatatcttcctgttcccagaggccctgtacagtttcttcttgggtcagggatgtgggcaagggtgggcagtactggaagtctctcctgccttgcagtctcaggagtgcccacctgtttggttgatgagctctctctcccacggggtttgggaacagggagctgtgggccaggatcagcgaggtttgggccccagctagaaaccagaagtgtctggtcccagaagaattttgcctttgtgtatcctgaatccagcaggcaggtcacttggagcagaaaagttggtcttacctcttgtctcgggcctgaagtcgctcctcggagctggttttcagctctccatcagggcagcaaccaaaagggcctgccccgccttctctcaggaccctgtgcacagggggcccagatggtgctagacctttttctctagattcagaaatgtgggcagagagtagtttcctctgccttcccaggcatgtctgttcctctgaaggtctagctttccctcccatgggatttgggtgcagggagctgtttgaccaagcgctcctgcagcttgagtgcccctatcttccttttcacagaggccctatacagtttcatcttgggccagggatgtgggcgagggtgggtagtactggaggtctctcctgccctgcagtctcaggagtgcccacctgtctgggtgatgagctgtctctcccctggggtttgggaggagggaactgtgggccaggatctcttcacctattcttaacattaataattcaacacacacacacacacacacacacacacacacacacagcccctagtgagtcactatactgctggtagcctgaatgtatgttttatgcttgatcacttgggattagataacttatcagagagaggcttattcttagagtagattgaattttcagcaagtattaattacctgttgttcttcattgagagggttagtgattatgaaaatttctccatatgcattgaaatgtcaactggtattgtagtaaactcacatagacaatcatagttttgaaatttcatgggctctgcctgcctgtcatatatagaaagcttttctcatagtaggcatcctagtttttgcccttaaattctttctgctccttctcaaatgatgattccccaagccttaggtttgtttagtgactactacttacataagacttaatatcttataatattagacattaaatttatttgttcctaaacagctacatttaaaatatttaaacgaaagtgcaagttgtagaaatttattgttaagaaatatactatttctattaataaatatagtatgtaatatttacattaggtttaaaatatctagatgtttgagcactttgaagaaatgtcttgctatggtctcttgccatgtgacttttagagtaagcttgctcatgcatgaaaaattcatttctggattcaattttgagaaaattgatacagcaccattaattttttctattaataactacgatatgtctatgatttagttagacccttagtctcttgtggcactgttctgttttatgcagcaacttcagtagatggatagctaatagacgttttcaaattgtagtaattgtattcatgttatctatttttcttgggtatagtttatggttttcattaattctattcattttatcttgccaaattaattgacgtgaatgttcataatattctccaattatttttgaaatttatgtaaaagcacataatgatacaattcccatcattgctgataatgttaatttgatctttctctaccttttccctacctttctctgctatgtctgcttaaaagatgattaatttaggtgtctttcataggatcgagatgtaaagttaattctgctttgtgttattttaaatgacatgactcccactcccaattctactccccctttctttaaattttctgctttttcctaatgtcttaatgagatctcaggcaactgatgtgagcccgtgttccttgtccatttgaatgttgagtgcagccagatttttgttatcatcccacatagttgtgtgtgttaatttatctattggtacttggatacaatgggtgaacattatcagtttattgttggggaaataattcagtgccacaaatgtatatgttttcattcacctctgccacaatcccttgaataataaagcagcactccatgaaaactttttgctagtgcttgggcttggaaaattgcagaataaaaatactgagtttgattttcctttgaaattattttagattggtttgccacacattttttgtacaacttgagtgttcagaatatcaataaaactctccagggggatgtctttctaaaggattatggtgattacacgaatctttactgtctacacctttgaatatcttgaattgttggtgttctgggtaccttttcctgtaatttttggggtagttattcttctcatgttcttcatcagagaatcttgtaatgtgctagactgtgctgatagaggatggcaattgagaaatgcagagttccgctccatattttctttgttcttgcttttctatgccacacgttcagtgactccagtctttttgagcaaagtaatttttgttgcttaaattcaataaaatacccatttttcttctttagttcacaatttgcaattttctggaaaactctcctttacataaagccacctcaataatgaacatcattaatctgttgcctctggtactggtaattttcaactaaatatgttcttatcatttgagtctgctacactattttatttttgtttctttataattttattatatccttttacagcaacaaaatctcattactttttctaatctttattaacctttgaacaaccattctattttaggcatgcagctgaaattattggcactggagtctgtagtaactttggatatattttttaagatcatcattcgactccagaatccctagtgggatgaaatgagatctaggttcctaagagatccaattattcttaagcagaaagaaaaaaaatgaaagaatgaatgaataaaaaaagagagaaagaaaggaagagagaaagaaagaaagaaaaaagaaagagaaaaagaaagaaagagagaaagaaaatattgtccagagttctgatggtctataagatatatattcatttggacaaaaatgttaaacatatttaagaacatattataaatcctttcaattttactttgttagaaaaaaactttctcagaggactatgatgatgtatgtttaaaacgaaaggtttgttgttttttcttttctttttcttttcgtttcttttttttgtttttttttgtttttttttctttttttggcctagtgatgggaaagactttgattatttcatgtacaaatgactaatgactacttctgcacctttaatattgtagatccctaggctgccatgcctatactcacctcttttcttactttttacccttttagagacttgttcagtatcagatatagaaattgaaaatgggtttttttctgaatctgattatacatatgctctaaatagaaaaacacggtatagatgtaaacagggatatgtaacaaataccggagaaatatcaggaataattacttgtcttcaagatggatggtcacctcgaccctcatgcattagtgagtattttattatattgttgcaattatactaatgatgcataggagtttagtgttattctttttgtatatgattgatattctttcatttgtaaacagctttcaaacttcaagaaaaaatacacagcattttttttatttagacattcctgcattgtaaaatatcagttcatttgcctttttctaggctctaaaatagcctagttttaaatctagtgaagaagtctttgaccagatgcaaattcctgaatatatgataaccttataatatgtacgtgacactatgagttacgatctatttcagaacatctcccttttagaagatctttttaaatattttgatattggaaagaaagaaatgcttccaggcaccaggaaattttggtatttggaaacattcttttgttttaggacatacagttaatgaggattttctaggattaacaattagctcatctagtcttatttataagaaaaatacccagtgctatttttcaagatgtattcaatttataccttattgtttaaggtatgatttaaagtattcactaagttcataatttttcgtctactgtgattttacaggatttaattaaagaaaaggaaattaaaattattcccatataacattcatttatattaaattataattggtaaggatttattgaatttttttactgtgaaagggaaaacccttgatataatatctgcttaaattcaattcatctactttcctatattttatgagtcatttgatgtactaattataggaccttaattcgcaaaatgctatcatactttcctaaaattatgtatttgcacttgtctattttttggagtatgtgataagtataagaaaaattgagctgagaaatgatttctaaaataaaattttataaaagcttaagaaaggagatgaatgttacatagagtatatctcaattttaataactttcaagaaaataaattattactggtctccttagtttccttcaatacagtatttaatttgctatcatatattaatttataaagacttttttctcatgagaattatttctacttgctattgacacattagaaatgacattgtctctcttattttgcattagagtcttgtgatatgcctgtatttgagaatgctatgactaagaataataacacatggtttaaactcaatgacaaattagactatgaatgtcacattggatatgaaaatgaatataaacataccaaaggctctataacatgtacttatgatggatggtctagtacaccctcctgttatggtaagtactattttctctggaatatttttagataaaaataaatgtttgtgttattaataactgaatgttctagaatcttccttatgagttaatgtagcctaagaaaaaggactgttatgaaagctatcgataataatatttacatttattatatcattacattcatttatttatcctgtgtgtatacatgcacacatatgtgtgtttctggaagtgtgtatactgcattatacaggtaggtgtcagagaacttgtgagagtcagttccctctttcatcatatggatctgagggattgaagaggactccaggcctaaaggcaagcactcttactgactgagccatctttctggcctgataatctgtttttaaaaaattctatattcatcagttgtatatggcactggattatgattctagcaattaggaccctgaatcaagagatttttaagtttgaaggtatattggactacatactaagttctgtttctaaaaccaaacaaaccaaaaatttcattaaattaatgattcctttgtgtggcctgtgtgtatcatgtatctctgatttgaggacaattcttttgttattcaagctcttatgtagactaggtctccattatcaaatttatgatctgaagcatgaaactaggtaatgaaaacttgaggcctggagagatggctcagcaggtaagagcatgggctgctcttccagagatcctgagttcaattcccagcaaccacatcatggctcacaatgaaggaggtagaagtatggcattcttgaaatctaggccagtctgggctatgtaggaattgtaagtggtaagtgcaggaattgtaggaatacagctctgaagggaaaagcttccccaatggagatgctgcagctctgagtgtctcagtgcaagtatgacagctctgaagggaaaggtatcctggcagtagggagctaaggaaaaccacaaacttacactgcacaaaacaaacctggcacaagaactttattgggaaaaacataagaaagctgtttctgctccagattaaagcagcaaagaacaagctcagtgattggtgagattttgagtttatcttgggcttccaccccatccctaccctccagaaaggaacttggccattagcacctcaaggggctagactgccattatagtagtctggaggtggggcttggtcacttgcgtgacttcaagggacttaccttaagatggtggctgcctctgtttgaccaacatacaacaggaaactgagcaggagacagataaatataagttgtttttttttccgggggtctgggggtagggtgggttttggaggataaacatttccaaggtggggaatggtgagattttcaagatcaagactggtgggtattcacactcagggcttggtagggtttcctatttagggattggtaggtttgggtaggttttaagccatgaaatgggctcagaacttttaccctaaatgaagacatctcacaaacagacaaacagcaacaaatgatgtacatagtaagaaaaaaatcaaactaaacaaacggtgatcactagtttctctctgattataagcagttcaacattatgaaatcaggactttctataatacaatactaaagtagaatggaaggggagggatattagtttcacaatacaatactttgcctaaggatcagtactaacactacaagtataaaataaaatataatataaaattatttatatactattctgatgtgtgagaattttttttctgtgaagtcaatatacaaacatctactcaccccaagaaagagcccatgacagaccaatgtacagataccactaatttccaacttcatgaaccttgagtcattgtgtccagttgcaaaatccccaaagagactacccggaactgcaacttccacacacgcacaggagagtctttattcaagctcgagcttgggctacgtaccttcctgatggaataggaaggagagagatacttgagtctaggggcttagggcttatatagggaaaaatctcaagctggagtcttcaagccttggcattacatgtttgggtaaaggggtaaaggaatgttaaccttcagactgatatcatcagggggagaccacacatttaaaagaggcatcttgtccttggaatgatttatgtttttttaacttattattgtgaccagttttcctgttgttgcaagctggccactgctgttatatctattttcaactgctgggaagggttggttgtctcttttccagagcccaagatgggggccatatcacttcaaggacagcagttttctccaaggacagcagcttttcccaaggacagcaattttctccaaggacaagatcttaaaattgaatttaaaggaaaagatggaatccctcctgctgccttttgccttttcagagttttattaaggttgctttcagaaatatgaatgagggtgttctcataggagaagaaatggctcaaagacagctacatcaccaaagcctacccagtatggctgacaattcacaaaacacaatggatcatataacataatgtgtaggcagcacatagattgaggagtgtcttttcaagtgagtcagctgatgaagcacctaccactgggtaggatccttcttctaggaagttaattatctcattctttgctccatctagggagctctgagctccttccttgcagttttgcttgtctgagtgattctcaccaattcagctagcttgtttactctggaagtaaggggcctgctaaatctgcttagtttcagggactccctgaagctattttgagttgtttacttccctccttaaggagcttccctgcagtatggagtatttcagtctcaaggaaactgttgcccaacaaattcccatggtctttcaatgtctccaggtctgacaggtgattgtaaagcagaggagaattgcacaaattattttttcactttaagacagagtattatggtatgtttgctaaacaatttgtataaaataagcaaagagaatacacaaataggtgcaaaacaaaaaatagttatagatgattatattgtgccattcaaatccacttggaaagagcacacacgtagattcaattcaagtttaggttaaatgaatttcttcttatttctatcaacacagaagggggaggaagggagggtttataaagttggattcctaaagttgcatattacaattagccatgaaatctgcagctggaccaaaaagtgtttttgcatccctcagttgttctttacctttgtatgccaataaaaagatcacttcatccctgtcccacaaaagcaaaaaacaaactgtcaaacatcttacaacaggaactctagtaacctatctaaacttttctgttttctttacttttctttttacttattcttctctcttacaataaatatatcctgattgtagcctcccttcccccaactcctccctgttcccactttcccttctctaccagacctactgctcctccctttcccttcagaaaagagcaggcgattcatgaatattaatcaaatatgacataacaagatataataagcctaggcataagcccttatttcaaggctggatgaaacaaccaagtaggataatggtctcaagagcaggcaaaagaattagagacacccatgactcccattgttaggagtcccacaaaattcccaagctaaagaacactatgcaaaggacctagcacagacccatacaggctctttgatttcagctcctgtctctgtagcctctatgagtcctacttagttgattctgtggcccacgtttttctgctgttaccattccacacacaaaattcattctattgccccttcccagggtgatttccttcttacttctctccacttcttacttagcctccctttgtctgtgtgctgtcacatgattagcctttacttagctctaataactacttatgaatacataattatttttgtctttccaggtctggttgcctcactcaggatatgtttttctagttccatcatttgcctgaaaatttcatgatggcatttctctaacatctttcataatataccattatataaatataccacatttttatgcactcttcagttgaggggacatctaggtttctaagctatccagtctctgtttgctggccctcaggttagtgcctggcatggctctttctcactgcattgggatgaagctgtaccaatcattgattggccactcctgcaagttctgcagccgtatcttgcaggagaaatagtcggctgaagattttgtggcagggttggtgccccaattcctcaactggaaatcttggttagaaaagttggctggttcaggctccttaaaccccagtactaggagtctttactaggctcacactcaaagattccttggaatttcccttgcactaaggtttggtcttgtccctgaaataccccaaattctaatcatctctttcaatactttctcactccaccacacctgatttctcctcttaccatcccttcagttttgaacatagcagttgtcttttatgaatgactctaattaaaaattatgacttttaatatatacattggaaagaaaggagatttttaaggcagaaatgtgttatttatttatttacatatttttggtaacactcaacaatgacaaaaattgaagaaaaaatttttcatacaggagaatgtgtcatacattcttaatttgagtcagaataattcacaattaattaattaaaaccagaattataaaactggtttaatgtaaaggttttgcacaacttttttatagtctacttaatcataaaatatactatattttcctaacttcagataaattagaaattattttatatattttagtttctcattatattaaactgaaatgatttcaatatatgatgtagatatagtatgacactaatttcaaatctgaaggaaagaattttgtgttgtagaataggaaagttattactttaacattaatatttatctgcagcagctcagatccactggaagacagttggttttattaaatcagttttgtgattaatacattatgctttgttatgtttctcagagacgtccacattgacttagaggctatattaaagctaggacacaatgtttttcctaaggaagagggtttctgaagcttccctgtgaatgtacatgagaaagataaaaatacttatcaatgattaatggtatattctaattatcttttcaagaaagagaatgcagcattcccctgttacaccaagacttagttgtttttcccagagaagtaaaatacaaagttggagattcgttgagtttctcttgccgttcaggacacagagttggagcagatttagtgcaatgctaccactttggatggtcccctaatttcccaacgtgtgaaggtcagtatctgttttatatttgatgaactaagatcagaagtttattttttttcctcttttagtattccccagttatcaagtatgtctataatataaaaatcttcagagaaatgaacattcattcagatacacagccacatgtttatgaggttaatttgaagctaacttgcttctttaaatgtgttatccatgtgtttacacatgcagacatgatggctgagactgatgggatttctttcattttgcctatattaccattagtgctggtgtttttataccataggccttcccgcatattgtatagagtacgtccaaacctgtaaaagcaggttgtaattaattcaaaaccaggttcaatatctatttaaaatagatacgaggtacaatgctgattttttttacaatgtggtaaatgtatgataaaatagtaccagtcaatgtgaaaatcattataatcaacacaacaattactgagtgattgcatgtatcttcaggctgtcaggtttatcaaaaattcttccacctccaatatatttgcaatgctattgcaacagttgtattaaagttgtgaaatgtaaatttagtgtaaatactatttagaaaagtgtaaaagaaagttatatagtgtatacatttaaattttctccatttactaaaattttagactgtaagatggacattttcttttatatttatacagtatttctgtaacaggccaagtaaaatcatgtgaccaacctcttgaaatcccgaatggggaaataaagggaacaaaaaaagttgaatacagccatggtgacgtggtggaatatgattgcaaacctagatttctactgaagggacccaataaaatccagtgtgttgacgggaagtggacaaccttgccgatatgcgttggtaattaaaataattaacacttaaaaattgttttgcatctcatgtgacgttttaattataagtaacttaagtgaaatacctacagagtatgagagaacatgtggagaccttcctgcacttgagcatggctctgtccagttatctgtccctccctaccaccacggagattcagtggagttcacttgtgcagaaaccttcacaatgattgggcatgcagtagttttctgcattagtggaaggtggaccgagcttcctcaatgtgttggtaagtatgtgtgcataaaatggatacttcataaagtttaatatttatattgcagaaatatttgctactgtgtacttctgaagtaagtagtcattttggaaatatctagtcttaaataatatgaatccaaactttcattgtttatattttgatggatgtctacaggtgaacagaaattcttaacatacaatatataaaagtttgttcattaccacaagataaatctagttgttaattataaattgtcatgtgactgacatgtgaatattaacacccaagtaggtttgactatggtacaaaaaagatcattgtttttattgtatgagactctcctctcaggacttggaaaggtaagaattaaagtctgctaatcacccatttcctactctcattatagacttaccctgaagcatgtctgtaatgtttgtgtttattctacagactgcattctaaagtcaatgtgccaaagttgggactctccaccctgccatcagctgtagaactcagggattagatgggaaacataatcccatatatgactccacttcacactgattccccatgttcctttgctgattcagtcttaatgagttactggaagaatcttggtgtctacattttcttttctctgaaatggaagtttttcattgattgaccttggtcatccaggcttcactatttgttggagttttggatattctttaatgccagggaaacatggagctcctttggaacgggcacctattcttgtgctgcttaatgatatgctctctctgcccagacacccaaacttcataacagtttgccatgtaaatgaatacctttactacatatcaatcataacaatttttgctcagcaagcagattttgccaaacccatcttcatcattgctttaaaactgtttaacactttcataagaagaaagatcagatataatatcatatataaaaactgaatccttcattttatattagtttatgcttatttttatgtactctattgtactctagtatttgttcatatatcagaggtttagtttggtttatctgcctgcagccaccttaatatgactccagttatgtcttcctggattgcaaagttaatgttatgatacaaatatttttaccttgacactctaccttacttttctccaaacccttggctttcacctgatgaataagagattcagaagcaaatcaaccacacagtcaccatgcccctttgactttcttctttttcctttacagaaattggctttgtgtgtgtgtgtgtgtgtgtgtgtgtgtgtgtgtgtgtgtgtgtaccaatctttagtaagggacgaattctcaggagtctttagtgtttgcatcactctatcaacattttaaatattatacaactttgtctaattatttacttttatttgtactgtgtttattttattttagatttcaaattattgataaaaattatccatgacctatacagaaatgtcaaattcaaaaggactctcattttcaccaaataattaaaatgtatagtacactaaaatgcttccatatatatatacatatatccttatttaacttataaaacaaccatacaatcagaacaatttattattataacttaatattgctgtattatagaataacgtcatatgaaaatatatcttatagactcatatgtagggtgtataaaggagatagatgttgactacaagcccctaatatcctataccaattctctctcataaaatagtttgaaatatttgtattctatacaatataaattaaatgttattttcttgtatcacatctattaaaaaagatgtcccgatatcttatcaacacattttttattttaaaatttttaacattttaacattatgaaaaaatctgagagtaatgaatttgcatatttttataggttttaagtctatgaccaaagctggtcatatcataatcatttcttatgtagagcatctgagaaagtgtttttttaatgcttttgtaattgtctagtacccaagttccttcatgacacaaaatgtctctgagacataaatgagtgggcatgatatctagttcttatactataggccactttcgcatggtgagtctcaacattttagttggcagaatttatagtactaagttgtgtttcattgtacatttactgcatgcacattttaatgtagtagctcactcacttcttataagtgtttttatttttcatgaaaatattttcatacagcaacagatcaactggagaagtgtaaagccccgaagtcaactggcatagatgcaattcatccaaataagaatgaatttaatcataactttagtgtgagttacagatgtagacaaaagcaggagtatgaacattcaatctgcatcaatggaagatgggatcctgaaccaaactgtacaagtaagttcttcttggcattgtgttctcatgagtgttctagccttttctcaactagagcagttgtgtctttatttacttaaaaaatttttcctcaaattttatgggtaaaacctgtatttatattatttttacctctccctcttcccactccaactcaactccttttgtgtccctccaattttatatccaatttatgtcctcttcttgaagtatatgtgtaagcatacataatatatgcataatatatacaaatgaaacttgtatatataaattcaacctgattagtccattcagtgtttctcctatgtgtatgtgctaagactaagtgcatgggtttcaataacctatttgtttgctccagagagaaggctgattattccactctagacagccattaatcacctgtaggggaagggtcatgtagcattttccctatccatactaatttgtcagttggtaatgtcatcatggatatcttgttgggtgaccacacttttgagatttcatgagttcatctactctgccatatatgaagatattatcttctaacacattttctggaaaaaatattttttaatctagaggttgatttagaaattacaatatcatgcttgttagtgacctatagtgtaaaacacagaaacaaacttgctcaacatggcttttcctatgtgtcataatggattcttaccattccactacatgtgattaatttatcacaacaaatgtgttatgcctctcctatgcttcatcatcatgtctttcggtatgattgtgtgttctgtcagaccaaccatttatttaactctcctaacaatcagcttacctggaaaacctcgatttatttgacaccttctattctatgttactgggcaacagggccattctactactatttctgcttccctatttgtctttatcaccgttgttgtggaggccctgtctcatttgatattttaaatatttcttaaagacgaaagttcacagaaagtatttccatgccattctaaaattaaacctactacaggcatgttaatgcagtgcatgtgttgttttgaaattgtctatgttaggatatcatttctggtgtcattttgattatagtattaagatagtaattgcttttctcttatgtatggctagctagttgttcaaagaatgtatttactacgtagtgctgatttctatttattccactctacttaagcaaaaatataaaaagaatgaaattattagtaaccactaagaaagtaccctttcatattatgaatctgagaggagagtctgagtgatgaatgtgaggtgtcttgattttgtagctacgtagtgaaaaacttgtcagaagcactacattatcctggctgcgaaccatccgttttcacatgtgtaactagttcaggttaaatggaatgtccagcataattgaaattttgtacaacatagtataaaccactttgggtcacactccatattcttgttgaccaagaaccaaggttaagttaactatcaattgtgataactaattcttatttgctatctgacagagtccacaatttcctaagaaaaacgtatctgagcatgtttgtaggggcgtttctagtttaggttaactgaggaggaacaatacactgtatgtgtagatggcaccattttatgggcagggttcctagcataaataaaaagagaaaggtgactgtgaatcctgagtatagatacagtatgagcaacagcctcacatgtctactgccattgctttcctgcgcgatgagctaacttaaactattccttcttcttttctaccctccttcctatcttccttcctaccttccttcctttcttagcttcttttgtcaagtgcttcatcacagaaatgagaaaagtcactagtatatcaagtaaatgaaagtaccacttttcctaatcaactttcatttataaaatagtccctgaggatttttaatgtaagtcaacatattagattataaatagtcatagacagctctagaaaaatattcatgtaagcttaatcttaacataatatattttttatgactcacttaaaatattttaaaatctagaaatgattgaagtatgttttataaaaatatataaaactgcattaaaatgaatgagaaaaaatttggagtacaagaattgctatattaaattgctatacaattgaaatatgcaaaatatagacaatttttttgcaactcaacaatcagatttatatgctaaattctcaatccacaatagattcacacagtaaacttacaagcaatcgataaggatataaactgccaacctagatgagataaatttgcctacagaaatccatgccaacaaccttggcaatactatatatatatatatgtatacatatatatgtatatatgtgtgtatatatatgtatatatgcatatatagagagagacagttattaaatttcattactaacttactttttaatgaaaattatcacttcaataatttaagatattctctttagtaaagaactctgattatttttttctaggaaatgagaaaagattctgccctcctcccccacagattccaaatgcccaagtgattgaaaccacagtgaaatacttggatggagagaaagtatctgttctttgccaagatggttacctaactcagggcccagaagaaatggtgtgtaaacatggaaggtggcagtcgttaccacgctgcacgggtcagtagataggatttactttgcaccattagaacgtaggtgaggggtgggtattgaaaaaaaaagggcatactataaatgttctggacacattattcaaattgtgtatatttatttctaatgtaagtttttatttcggcttgactatttcatttctgttctctatgtagaaaaaattccatgttcccagccccctaaaattgaacatggatctattaagtcgcccaggtcctcagaagagagagatttaattgagtccagcagttatgaacacggaactacattcagctatgtctgtgatgatggattcaggatatctgaagaaaatagggtaacctgcaacatgggaaaatggagctctctgcctcgttgtgttggtgagactgacatgaaaattcaattttcattttcaatatgtcattaccaatattctactcttatccaagccagagagaaagaataatttaggatagcacatatatacatttatatattttactatacatttatacttgcacactataatctatgctgttttagttcattgtgccatttctgtagacatatactttcactcttgcattaccgtttttaaatatgatgtattacagactccatgtgctcatgtgaattctactgtttgatttgccaccaagtattaaagtccaaagtatcttttgcctaaaatgtcctccccactcccatcccacaatacatggtattttctgatatttgtaatactttcaagttgtttaacagatgcaagacaacagaatgtgctattaggaagcactgcccaccttccttatgatgatgcatctttcatattaacacttccttcttgtacccctacacacagaactgatacatacaagcaaatttctgtattagtgcaatgtggaattgtttaactatgtaactctcatttgtgtctttttcaggaataccttgtggacccccaccttcaattcctcttggtattgtttctcatgaactagaaagttaccaatatggagaggaggttacatacaattgttctgaaggctttggaattgatggaccagcatttattaaatgtgtaggaggacagtggtctgaaccacccaaatgcataagtacattttaattttcattcttttgtctagtatataatacaattcaatctatatgtggtacaattaagaagctaagtcatactttgattccatatctcctcctatgaatatgtttgtttcccctctaagaaaaactgaagcatcctcactttggttatccttcttgagcttcatgtggtctgttgattgtatctttgggtaaactaaggttttggactaatacccacttatcagtgaatacatagtatgtgtgtttttttgtgattgggttgcctcactaaggatgatacttcctttttttatttttattatttttatctttgttaacttgagtatttcttatttacatttctattgttattccccttctcggtttccgggccaacatccccctaactcctccccttcccctttcatataggcttcccctccccatcctccctctattaccaccctccccccccaaaatcacattcactaggtgttcagtcttggcaggacccagggcttccccttccactggtgctcttactaggatattcattgctacctatgaggtcagagtccagggtcagtccatgtacagtctttgggtagtggcttagtccctagaagctctggttgcttggcattgttgttcatatggggtcgcgagccccttcaagttcttccagtcctttctctgattccttcaaaagaggtcccgttcttagttcagtggtttgctgctggcatttgtctctgtatttgttgtattctaggtatgtctctcaggagagatatatatcaggttcctgttggactgcaccttttgcttcatccgtcatatctagtttgatggctgtatatgtatgggccacatgtagggcaggctctgaatgggtgttccttctgcctctgttctaaactttgcctccctattccctgccaagggtattcttgttcccgtttaaagaaggagtgaagcattcacattttggtcatccttcttgagtttcatgtgttctgtgaatctagagcaattcaggcatttgggataatagccacttatcaatgagtgcataccatgtgtgtttttctgtgattgggttagctcactcaggatgatattttccagttccatccatttgcctatgaatttcataaagtcattgtttttgatagctgagtaatattccaatgtgtagatgtaccacattttctgtatccattcctctgttgaagggcatctgggttctttccagcttctggctattataaataaggctgctgtgaacataggggaacacgtgtcttttttatatgttggggcatcttttggatatatgcccaagagacgtatagctgggtcctcaggtagttcaatgtccaattttctgaggaaaccccagactgatttccagaatggttttaccagtttgtaatcccaacaacaagggaggggtgttcctccttctccacatcctggccagcatttgctgacacctcagtttttgatcttagccattctcactggtgtgaggtgaaatctcagggttgttttgatttgcatttcccttatgactaaagatgttgaacatttctttaggtgtttctcagccattcggcattcctcagcagtgaataatttgtttagctctgaaccccattttttagtagggttatttgtctccctgtggtctaacttcttgaattctttgaatattttggatataagccctctatctgttgtaggattggtaaagatcttttcccaatctgttggttgtcgttttgtcctaacaacaatgtcctttgccttacagaagctttgcagctttaagagatcccatttgtcgattcttgatcttagagcataagccattggtgttttgttcaggaaatttttcccagtgcccatgtgttcgagatgcttccctaatttttcatctattagtttgagtgtatctggtttgatgtggaggtccttgatccacttaaacttaagccctgtacagggtgataagcatgcatcgatatgcattcttctacatactgacctccagttgaaccagcaccatttgctgaaaatgctatcttttttccattggatggttttagctcctttgtcaaaaatcaagtgcccatatgtgtgtgggctcatctcagggtcttcaattccatttcattggtctatctttctgtctctgtaccaataccatgcagtttttatcactattgctctgtaatactgcttgagttcagggatagtgattcccccagaagtcctttcattgttgaggatagttctagctatcctgggttttttgttattccagatgaaattgcaaattgttctgtctaactctctgaagaattggattggtagtttgatggggattgcattgaatctgtagatttcttttggcaaaatggccatttttactattttaatcctgtcagtccatgagcatgggattctttccgtcttctgaggtcttcttcaatttctttcttcagaggcttgaagttctcatcatacagatcatttatttgcttgattaaagtgacaccgagggattttatattatttgggactattatgaagggtgacgtttccttaatttccttctcagcttctttctctttcatgtaggggaaagctactgatttatttgaattaattttaacccagccacattgctgaaagtgtttaacaggtttagtagttcccttgggatcacttaaatatactatcatatcatcagcatatagtgttattttgaattcttcttttccaatctgtatcctcttgatctccttttgttgtctgattgctctggctagaacttcaagaacaatattgaataagtaaggagagagtgggcaaccttgtctagtccctgattttagtgggattgcttcacgtttctctccatttagtttaatgttagctactggtttgctgtatatggcttttactatgtttaggtatggaccttgaattcctattcttttccaggacttttatcatgaaggggtgttgaattttgtgaaatgctttctcagcatctaatgaaatgatcatgtggttttgttctttcactttgtttatataatggattacgttgataattttctgtataataaaccatccctacatgcctgcgatgaagcctacttgatcatggtggatgaatgttttgatgtgctcttggattcggtttgccagaattttttgagtatttttgcgttgatatttataagggaaattggtctgaagttctctttctttgttgggtctttgtgtggtttatccatcttgacctgggctctttttggttgggagacctttaatgactgcttctatttagttcagagttatggggttgtttaaatggtttatctgttcctgatttaactttggtacctggtatctgtctaggaaattgtccatttcctgcagattttcaagttttgttgaatataggcttctgtagtaggatcttatgattttttgaatttcttctgattctgtagttatgtctcccttttcatttctgattttgttaatttggacacactctctgtggtctctcattagtctgactaagggttaatctatcttgttgattttctcaaagaaccagcttttggttctgttgattctttgtatagtcctttttgtttctacttggttgatttcagctctgagtttgattattttctgccttctacgcctcctgggtgtatttgcttctttttgttctagagcttttaggtgtgctgtcaagctactgatatatgttctctcctgtttctttctgtaggcacttagagctataagttttcctcttagcaccgcttccattgtgtcccataattttgggtatgctatactttcattttcattaaattctaagaagtctttaatttctttatttcttccttgaccatgttatcattgagtacagcattgttcaacttccatgtatatgtggacgttcttcccctattgttattgaagaccagctttagcctgtgatggtctgataggacaaatgggattatttctatctttctgtatcttttgaggcctgttttatgacttactacatggtcaattttggagaaagtaccatgaggtggtgagaagaagttatatccttttgttttaggatagaatgttctataaatatctgttaagtccatttggttcatgacttctcttagtctgtctatgtctctgtttaatttgtttccatgacctgtccattgatgagagtgtgtgtgtgtgtgtgtgtgtgtgtgtgtgtgtgtgtgtgtgtgtgtgtgtgtaatctactatcattgtgtgaggtgcaatgtgtgttttgagctttagtaaggtttcttttatgtatgtagatgccttgtatttagagcatagatacttaggattgagagttcatcttggtggatttttcctttgatgaatagaaagtgtccttccttaccttttttgatgacttttagttgaaaatcaattttatttgatattagaatggctactccagcttccttcttcagaccccttgcctggaaagttgtttttcagcctttcacactgaggtagtttctttctttgtctctgaggtatgtttcctgtagacagcagaatgccaggtcctcattgcatatcaggttcattaatctatgtctttttattggggcattgagacgtttgatattgagagatattaaggaatactgattattgcttcctgttatattcatatttggatgtgaggttatgtttgtgtgcttttcttctctttgttttgttgccaagacgattagtttcttgctttttctagggtgtagcttgcctccttttgttgggctttaccatttatcctttggagtgctgagtttgtagaaagatattgtgtaaatttggttttgtcatggaatatcttggtttctccatcaatgttaattgagaattttgcaggatacagtaacctgggctggcacttgtgttctcttagggtctgtatgacatctgtccgggatcttctggctttcatagtgtctggtgagaagtctggtgtgattttgataagtctgcctttatatgttacttgacatttttccttactgcttttaatattctttctttattttgtgcatttggtattttgactgttatgtgatggcaggagtttcttttctgatccaatatatttggagttctgtaggattcttgcttgtttatgggcatctctttctttaggttagggaagttttcttctatgattttgttgaagatatttactggtcctttgagctgggaagtcttcactcttttctatacctatttatcttctcattgagtcctggatttcctgtatgttttggaccagtagctttttccattttacactatctttacccttgtgtcaatgatttctatggaatcttctgctcctgagattctttcttctgtctcttgtattctgttggtgatgcttgtatctatggctccttgtctcttcctttggttttctatatccagggttgtttccatttcagctttctttattgcttctatttccctttttaattccttcacctctttgattttgttttcctggaattctttctgggatttttgtgattcctctctatagggttctacttgtttatttatgttttactgcatttctttaagggagttcttcatgtctttcttgaagtcctccagcatcattatcaaatgtgattttaaatctagatcttgcttttctggtgtgtttggatattcagtgtttgctttggtgggagaattgggctctgatgataccgtatagtcttggtttctgttgcctgggttcctgcgcttgcctcttgccatctagttgtctctggttttatcttctgctatttctaacagtggctagaccttcctatagggctatgtgtcaggagtgctgtagacctgtttcccttttttcgttcagctagttgtgggaacagagtgttctttagggtgtgtagtctttcctgcctagtggtcttcgctgttcctgtgggactgtcctgagtccaccaggcaggtcacttggatcagaaaagttggtcttacctgtggtcctgtgtctcaagttgctcgtggggggctgcttttgagctctctgtgagggtggcaaccaggagggtctgtgcagccttttccatgagcccccgagtactggggtcccagacggcattaggtgttttcctctggagtctgaaatgtgggcagagtgtagtctcttctggcctcccaggcgtgtctgcccctctgaaagtttagctctctctcccatgggatttggctgcagagagctgttgattggtcccttcaggtcaggtgggtatctggatcccaggggacctgctgctccagtgcccctgtcttccatttcccagagactgtatacagtttcctcttgggccagggatgtgggcaggggtgggcagtattggtggtctcttctgctctgcagtctcaggagtgcccacctgtccagatggtgagctctccctcccacaggatttgggtgcagagagctgttgatccggtcctttcaggtccaggcgatgtctggagcacaggggacctgcagctccagtgcccctatcttccagttcccagaggccgtatacagtttcctcttgggccgcggatgtgggccggggtgggcagtattggtggtctctccctctctgcattctcaggagtgcccacctgtctgggcggcgagctctctctcccaggggtttgggagcagtgaagtgtggccgggatcagcgagattcgggctccagctaaaaaccagaagtgtcctgttccagaggaattttgcctcagtgtgtcctgagtccaccaggcaggtcgcttggagcataaaagttggtcttacctgtggtcttgaagctcaagttgcttgtgagggggctgcttttgagctctctgtgagggcggcaaccaggagggcctgcaccgccttttcctggagcccctgtgcaccgggatcccagatggcattaggtgttttcctctggagtcagaaatgtgggcagagtgtagtctctttttgcttcccaggagtgtctgcccctctgaaggtttagctctccctcccatgggatttgggtgcagagaactgttgagcagtcccttcaggtccgggcagcatctggaacgagggggacctgctgctccagtgcccctgtcttccagttccaggaggccctatacagtttcctcttgggccacggatgtgggcaggggtgggcagtgttggtagtctctcccactctgcagtctcaggagtgcccacctgtctgggtggtgagctctctgtcccacagggtttgggagttgggagctgtgggccgggatcagtgaggttaggaggatgatactttctagttccatccatttgcctatgaatgtcatgaatcattgtttttagttgctgagtaatactccattgtgtagatgtaccacattttctttatttattccactgttgaggaacatctgggttctttccagcttctggttattataaataaggttgctatgaatataggagaatatgtgtcctggttatatgttggaacatcttttgggtatatgcccaagagaggtatagctgggtactcaggtaggtcaatgtccaattttctgaggaacctccagactgatttccagaatggttgtaacagcttgcaatcccaacaacaatggaagagtgctcctctttctccacatccttgccagcatctgttgtcacctgagttttttatcttaagaatgtccattcagatactgccccacctggggatccagccaatatatatacagccaccaaacccagtcactatatgccaagagctgcatgctgacaggaacctggtatggaagtctcctgagaggctctgccaaagcataacaaatacagagatggactgagaactgggtgcatattggaggagttagagaaaggattgaaggagctgaaggtgtttgcaaccccctaagaacaacgatacccaccaaccagagctttcaggaactaaatcactgtccaaagagtacacatggacagacccatggctccagttgcatatgtagcagaggatggccttgttggccaccaatgggaggagaaacccttggtcctgtcaaggctcatcctccaaccctttcctatctgacattcccacccccccccccagtttaggcgactgtaagataggaaagggttggaggatgggcaggggaacaccctcatagaagaaagtggagagggaatgggacagggggtttgtgggcaggaaactggaaagtgggatggcatttgaaatgtaaaaataaaaatatccaataaaaaaactaatgaaggagaatcgggtatagttaaaaaaaaaaagaaacgaagccataattctagcatataaaaagtttttgctgcataatttgaatgctggaagacaaatacgatatgagtcaaaacaaaatttttcctttccagcccacctaagttgtttttgttccatgtagtctgagatatctgaattatcagaattctcagaatccaggaacacacaggctcctctaaacagtctcatcactacaatgacagttttagagcaatgccactacaattacatatgctctaaatttttcaaataattatgagtaagttacattttataaagtcaaacataaatactctaattttggaaagtacaagaaaaattgaatgcaaaatttaaaatttcaaaaattataaccatcaggattctgtgtctatcttatttattttcataaatatagaagaacgtcagtgtaactaagtaaaaaatggaaaacctactgtatgtattgttttctatgaagttaactattgtttcatatatcgtatgttctacaacttcctgaaaacaaacacccacatactcttttatttttttaagaaactgattgtgacaacttgcccacatttgaaattgccaaaccgacagaaaagaaaaaaaaatcatacaggtcaggagaacaagtgacattcagatgtccacctccgtatcgaatggatggctctgacattgtcacatgtgttaatacgaagtggattggacagccggtatgcaaaggtatttgaatgggtttttaacatgcatttattctagtgtcaaagaatgacataactgaaaatggtgcagagattacttttaaagtaagatcaagtttgtttgtatcaaataataaaagcattgaattaaaaaaactgatggctaagctgatagcatgatggtgttcagagtttgatttcatggtcagcatcatcagtatcattagaatacaaacattttgaaaatgtaaattaacagctaggagtacatgctagatatcctaaataggacgacatctaaagatgagaccttcaatctccttttagggatctgtgtatgactaagtttggaatgtgctgtaggctgtcaatatttgttaatatgttgttaaataattagccttcaattgaaatcttgcttatatctcattttatcaaattcattggaatattaggatattttatttgattatcactttcttatgactatattattcttaaaacaatgttctttttcctctaacattgcaaatagatttttttctcacataatacatatcctgattgttttctcttccctccactcatttcagctccttcctaccccttttttcatctaatttttcccctttctgtatttcaggagaaaggaaagtcttctaaggagtaatactaataaaacaaaaatgaaacaaatacagtaggaggtaacaaacaaataattttagggaaaacagcataagaaaatagataagaaacaaaatagacaaaatgtcccactttatacacctaggaatcccttaagaatactcacctgaaaaccataatatatattgaacagcatgcaaagtaccttcctgtaccaaagatgcttcccttaggggtgaaggctctatgtaggcatcagtgacactttgctatgatcagtgagttgcatatttgttgtttttcacagtgtagacttgccttcaggttgtgtggtataatctgtagtcttctcaacagcctgcctgtgttattcggaagtttccatgtgacccctctggtacacatttaattagatgtaaccttatcacagtactagaagcttcattagtgacatgatatgtccctcggggctctgtctccttacacttttggtgattgcacttatatttcctttatatatgtatgtattttagaaagcttatattgaattaggttttgataatatccctcaaatgacacttaacttttgctgttcctctctgtattctgatttttgtctacccttcttgacatccataactatctactctatttctccatcctaaggagacagtactttgcccccaattccttaggcctacacctaaattctgttgttctgtggattgtaaagtgactttcattggctttcagctaatatctacatatcagcaaatatatacatgtgtgtctttctgggtctgagttcttcactcaggatgaatttttgtctattacccatcatttacctgtgacattcatgatttcatttttgcatgtaaataaatgtagcaaattttctttatccattcagcaagtcagaaatatatttggaatcttatgcattaattggacactcaagatgagcaaataggtactaatactttattttactctttagataattcctgtgtgaatccaccacatgtgccaaatgctactatactaacaaggcacaagactaaatatccatctggtgacaaagtacgttatgactgtaataaaccttttgaattatttggggaagtggaagtgatgtgccaaaacgggatttggacagaaccaccgaaatgcaaaggtagggcatcatttcccctaatgtttatttgacaatgcaatttagttattgtacattagtgaaaggaaactgaagcaatttttaaactttttttaacttttacaattattttatttatttacatcccaaatgatgtcctctccctgtccccactccaagaactctttcccccatacccctctacttcacctctgagatggtgcttacccatccctcttgcctggggcatcaattttttaaaggattaggtgcatcctatcccttcgaggccagaaaagggagtcctctgctatatgtctgccaggagcttgtaattagcctctgtatgctctttggttttgtggcatagtctgcgagctgcaagtggtgagtggtccatgttagttgacactgttggtcttcctatggggttcccattcccctcaacttctttaatacagcccctgacacttccataggtcaactgctggtagagtttattagaggaaagccatgctaggctcctgtctgcaagcacaacatagcatcagtaatagcatcagtgcttggtgaccctccccacctccatgagacagaactcacattgggccagcaactagtcaataattccttcagtctctgctccttttttgtctctgcatttctttcagagaggaacaatttggagtcaaaattttgaagttggtttggttgtcacacccctcctctgggtgtcctattgaactattggacttcaggttcctcttcccaccattgagtattttgcttaaggtcacccacattaaaacctgggagtctctccaccctgggtttctaggattttaagcagtttctgttgattccctgtctctggaaaatttatgtttccacttatttttctggtctgctgggcttctcttccgttttgccccatatctgaccctgccccaccccatgcccccgttatcccttcccctcccttctcccacctaggtaaccccctccctctacctcccatgattattttgcctcatattctaaggtaaatttgaagcatcccacatttgggctttccttcttgtttaacttcttaagctatatgggggaaccccatgggaattctggactttttaactaataccccttaccaatgagtccataccatgaatgtcctttgagtcttggtttctcagtcaaaataatttttcttttctttttatattttgtttactcttttttacactccaaattttattcccctctttgtccaccctccgactgttccacatcacatatgtcctcccttcccctgcccctgccttccatctaggaggatgtcccctacaccccaccccacccccagatctctaaactccctggagcctccagtctcttgaaggttaggtgcatcttctttgattgaacacagacctggaagtctagtgctgtatatttgttgagggtctcatatcagctggtgtatgctaccaggttggtggtacagtgtctgagagatctcaggggtccaggttagttgagacagctggtcttcctatgggaccaccctaatcatcatcttctttcaagcatttccctaattcaaccacatggatcagcatcttctgtccactggttgagtctaatatctgcatctgaattttccagcttcttgttgggtctttcgggtggcagtcatgagaggtccctttttgtgagtgctccatatccttagaattactgtcagaccttatagcctccccttgagctgggtcccaatttgggcctatcaacagatttcctttccctcaggctcttctccatttttgtccctgtagttcttacagataggaacatttctgagttacagtttttttgactgtgggatagcaaccccatccctccactttatcctttctcttcctactggaggtagactctacaagttccctctccccactgtagggcatttcctctaaggtcctgccttttgggacctgagagtctctcatggccaaggtgtctggtaatttatatagggttccctccatcttctacctccagaggttgcttatttccatttttttctgctaacccaaaggacttcagtcctgttttccctgcctccaatatgtgatcatgtcatccttttcactcgctcatccaagtacctctctctcctgactgccccatgattgcatggggtgttcaaatctcctattattattgtgtgaggtgttatgtgtgcttcaagcttcagtaagtttttttttaataactgtatgttgccttgcatttggagaatagatattcaggattaagagttcatcttggtagatttttttcctttgatgaatatgaagtgtctgttcttatcctttttgataacttttggtagaaagttggttttatttgctattagaatgtctactccaacttgtttcttggaaccaaatgcttggaaaattgtttttcagccttttattctgcggtagtatctatctacagtcactagagtgtgtttcctttaggcagcaaaatgctgggtcctctttctctatccagtctgttattggggaattgggtccattggtgttaagagatattaaggaatagtgattgttgttgtgtagctctcttcttttggtttcgttgtaaggagattactttcttgctttttctagggtgtagtttttnntgtggaaatatattgtataaatttggtttggtcatggaatatcttttttctccacctgtgttaatcaaaagttttgctggatatagtagcatggactggcatttgtattctcttagggtttgtatgaaatctgcccagtatcttctggctttcatattctctggtgagaagtctggtgtaactgttttaggtctgtctttatatgttacttgacctttttcacttactgcttttaatattctttcttcgttttgtgcatttggtgttttgtctattacgtgacaggaatttcttttctgttcaaatctatatggaattctgtaggcttcttgtatgtttatgggaatttctttctttaggttagggaagttttcttctataattttgttgaagatattactggccctttatgttgggagtctttggtctcttctatgcctattatccttaggttgatcttctcattgcttcctgaagtttctagaggttttgggttaggagctttttgcattttacattatctttgacatttgtgtcgatgttttctatggtatcttctgcccctgagattctctcttctatctcctgaatctctgttggtgatgcttgcatctatgactcctgatctctttcctaggctttctgtctccctttgtgatttccttattgtttctatttcaatttttaaatcctgaatagttttgctcaattccttcacctgttcggttgtgtttttctgtaactctttaaggaatttttgggtttcctctttaagggcttctgcttgtttacctgcattgtcctgtatttctttatgggagttatttatgcccttcttaaagttctctatcatcaccatgagatgtaattttaaatccaaatcttgcttttccagtgtgtttggacatccagtattttctttggtgggagaacttggctctgatgataccaagtagtctttgtttctgttgctttggttcctgtgcatgcttcttcccatcagtttgtctctgctgttagcttgtcttgctctctctgacagtggtttgaccctcctgtaagctatgtgtcagcattcctgcagacctgtttcctttcagtcagatctgggaagagagagctgttcctggttgtgtgtcctgaagcctccaagagggttgcatggagcagaagagttggttttacctctgttctctggtgtgtcagggctccaggctattggctttcagctctgggctcaggcagaaaccggattgattctgcccctgactattcctaggttcttgtattcagagggctctagacagatttctcttgggacaggaatgtgagcagaagtgggggtcttccctgatctctcaggattgtctgcacttctgagggtccagctgtctccctcacaggatttgggtacagagaactgcaggacctgttcaggaccttgtgcaggcagaaactggtagtggactgtccaagaagacttctgtctttgtgtgtcctgaggccaccaggtgtccacttggagcagaagagttggtcttacctctgctctctggtgtgtcatcactcctgatgactggctttcagttttgggtgcaggcagaaacaggaagagacctgcccctgactgctctaatttcttgtgcccagagagcagaggaggcactagacaggttcctgttgggccaagaatgtgagcagaagtcggggtctcccctgagctctcaggattatctgcacttctgagggtccagctgtctccccgataggatttgggtacagagaactgcaggaccagttcaggtccttgtgcaggcagaaactggaagtgtactgtcccagactgctcctgcctttgtgtgtcctgaggccaccaggcagatttcttggagcagaagagttggccctccctctgctcttagatgtgcaggcgctcctggaaaccgactttcagctctggatacaggcaaaaaccataagtttcctccgctgaatgctcccaggttactgtgcttagaggtcacagagggcactaggaaggttcctgttgggccaggaatgtgagcagaggtgggggtctctcctgagctctcgggattgtctgcacttctgagagtccaattctctctcccacgatatttgggtacagaaatgtgggaccaggtcagccctgggtgcaggtgcctatttctattattcttagatttgatattttcattgtacctggatttcctggatgcttcatgttgcaagatttttatgtcttgacttttctttgacagtgtgtcaatatcttctaaaatatcttctacatctgaaaattctatataatatctcttatattctgttgttgatgctttcatccataattcctgacctcttttctaggttttccaattcaagcactgcctctctttgtgttttctttatagtttctacttccacttttagctcttggaccacattcttcaattgcttcacctgatttctttctttcttttcccccctgtatttctttaaggaatttatttgtttcccctttaaaggcttctacccgtttacctatgttttcctgtttgtctttccatgacttacttctatcctctttaaaggatgctattatcttcatggatagtatattaggtcagcttcctgtttttcaagtttgttgttgcacacaaggcttgctgaagtgagagaattggtttctgatgacgccaaagtatattgacttctgtttcttatggtcttgggcttgcctctagcaaactggtcatctctggtgttagctgttctgggtgtctctgtcttcatcctacttcctatgtccctgggttgctagagttctctgggtaggcttgtgtttctggctgtagctgaccactggtgaagacttcagaatgtgaggtcttaataggggcatgtacactagtgacctgctgccctggctacagagacaatctgctgatctgttgccctgtgtgcagcagatctctttggaggccttcagactgtggggtctgttgctcagtgtgtagcagaattcgcggaggacttcacactggtcagttatcctgcatgtaccagaactcgtgagaggccttcagactgtagtatctttagaggagcagacaagctgatgatctgccattgcagaaggtgcaggatggaaagcattcttgtttgggagggtcccttacttattgccctgtgtgctgcagaactcctgagaggccatcaggctgtgataccttcagaagagcagccaagctggtaggggtcttatttctctttttatttcttgttttggaggagtggttctcaagaatttaacagtggcatgcatttttattacttttgaacacatagtctgagtatgctatctctaatagtttcctaaccatctgttactcaagtcaaccaggctgatattttatataagtagaaactgaacttatcttcaaaatccaattacattttccattttttgtgttttccttaaaaattccttcggagttttctcttacatatattaaatgccacccttttttatttttatttttttcagagtccatgatttatttgtttactctccttcctgggattgccctttcaataaatcccctttctttgcttttcattgttattcatcaattttttcttcttattattttatttacttacattccaaacattggcccccttcccagtaccatatcctcaagttattcattgtccccctttcctttgcttctgagagtgtgctccctgacacacccacctacctacacctcacccctaccagcatcccttctcccctcttttcagatttctacaggatttggctgttcctctcctactgaggtcagataaggcagccctctgccacatatgtaccaggagctatggatcagtccatgaatactcttttgttggtggcttagactctgggatctctgaggtgttctggttatttgatactgttgttctttctgtgataccacaatccccttcagcaccatcaatcctttgcttaactcatccatagacatcccagacctcattcactgttggctgtaaatatttccatctgtttcagtcagctgctaaatagagcctctcatgggacagccatgctgggcttctctctgcaagtacaacatggtgtcaaagtttggtgcctatacatgggatgcatctcaagttgagagggtcactggatgggctttccttcaggctctccacaatttttctccctgtgtttcctttagacaggaacaattcttggtcgaacatttataaggtgactgggtgaccccattcctcaactgggtgccatgtctacctactgttggtctctttaggttccaactcctcacttttggacattctgattaagcttatccccattggatcctaagagccccctctcatatctttgatgtctgagtctttctagggattctccagttcccccaaccattcactggtgcatatttctgttcattcttctggccctctagaattctgtcctgtgtccccccatattttatccagaccttcctcttctccctcctcatcccctctgccattcatgtccctccctccctctgcctcctatgattatttttaacactcttcttatatgcaagttttcacttgaaacacaaatctaattttatgaaaacaaagatcacctactatatagccctaatcttacagttaaatttgtcctactcttaatttttatttttcacttatataatgaattctggtagttattctttagggaggactctctgatggagataaatcccctttatctcttttatctgataatgtctcatcaatgtctttattcaaaaggcaaacaacacaggatatagaacttaaggcttacactcattttcttttccttactatggtctgcatggtgagaggataggagtcactttctttgggatctgggtccagtgtggttgatgatgacttcctactgatttttgtccaagatgttttctttaagcagtttcagtagagagatctccaggagtttcatgggacttgtcctatttgactttactcagttcttgaatatgtacagtcatctattatggagaattgttttcattttccttcatagtaaaacattaattttgcttgaatattgaatattttgtttttacctaaaaatatttgaatttttttcagtttcatgatgttcctcttgaggtcatactgaacataatcagtacttttgatttcatatttttcctgtgtcctcacaagaacaatcagtagtctaaaagaaaaacatataacacaacagtgtgacattagatgagtttggaatttctttgctagaattttcaatgtctcatctcttcatataatgtttactaaaaattctatgtccaagcttttcagatatacctagttaaagtatatcatagatgtctatgcttattttaaccatatcagaaacccagaaaacctcattagccttctgttacattataggctttcaagtcttgttttaaatgtacttatacaaaatgataaagagtgggaatatatacagtcatatactattgagtttcttcaaaaaaaaatgcctatctacattggccatagcacctaatccttctcaggttcagaagctgttaagagatttactactacttgaagttttcaggcagacatgtttgctgtagttaagaaatgtttcaggtgagaaaaaaagaagaacttgtaactctcagtttatatgattaatctttcttcaaataatcatttatacagccagaaatcactaaagacttaatacttaatgtttttggttctgcttgagcctgtagttttacttgatattcaaacattcaaatgttgtctccttagattcaacagggaaatgtgggcctcctccacctattgacaatggagacatcacctccttgtcattaccagtatatgcaccattatcatcagttgaatatcaatgccagaactattatctacttaagggaaataagatagtaacatgtagaaatggaaagtggtctcagccaccaacctgcttacgtaagtaccttattcacatagattataagaaattctgttttatattgtgggtatttttctgtttataatataacattcacaaaataaaagtactgttttgtttgtgtttcagtatcaaacatcagcatgtgataaaacaagattattagattctttttataaaaaatacctgttaaataaaattgtatatattattcttaataattgtttttttctaatatgtattaacatctacaaaactgggtgccagcataacattatataactgttgtctcagtcagtgttctattgttttaaagaggaactatgaccatggcaactcttttaaaagaaaccatttgttgggggttgcttacaattttggaaatttattctactctcaacatgtttgggagcatggtggcacagaggtaaacatgatggtgaagaagtagctaagtattccatatctggctctgcagggagcagaaagtgataggcatacttctaacaagtctatgcaaactcccacaaggccgtagccataatacttcacaagtaccaccattctccaatgaaaaatctgtatgtgtatctatggaggtcattccttttcaaataagcacatctgtatacatcttgcagttattaaatccatacaacatctcctttccttagataaggcaactgacatctattaatcactgttatgcattctaaagtaattctctctgtgagaaagagcacaaagtagttgtctttctgtgttggttatatttgacttaatgtccttcaatgcccttttctaagtaaaataataaaatatatctttaatgacttaatattttacatttaaatataccatgatgtcattataaattcaccaattagtattagttcagctttcttcaccttaccaacttccatgtagcagtttagaataaacatatagatccaggttgagtactttgattttatttcctttgcgtacattccagaagaaacaataggaacaatacataaatatctatttttaaatttgtaagaaatctcaatttttatccatagtaacttcacaaaatcatattcctgtcaatggtttgtgaagtgttcaccacacactaatgagcagttgtaatttttagggctccttcctctggtgctactttaactgagttaaaagatatcttactatggcttttcaatggaatgacagcaatgatatttatgtgtttttcttagaagtatctattcatttatccagatttgatcagcttatttttcctttaaaatgtgctttaccacagactaatatagttcagcgaaaggttatcagcagactggaatatttttcaattatttaagtataatttatgacagatatagtgcaaagccttttcacaatcaatttactaaaaaaggtgttctaacttctaacagaccagcaaggcccaaagcaatgaaatcaaattatataaaaacaaaacaaaagcaaataaatatatttatgcactttgtacgaaatggaggtcacatctttatgctttcttgacccaggacacccccctaaaagatatgtaaatacctaaaaataaagaatagacaaccatatacttcaattaaacttgctgccaatttcttaggtgtattgactatgctctgtgatatgcaccagtaccacaatgggatcaaatccacaggtcaaagtttgctttttgccttgtgatttggagtcccagccaaacacacagtgtcaaaaccatgaaatgtttccctgttgtgcttcctgatactttcagtggtttgttcttatatcaatgtctttgaccaaatttcagttgaatttgcccataatgacaaacagatataaaatttcaatcatcgccatatggatatcaattatcattttatcatttattaaatatgatatcagttcattaacataagttttgggaaagtttattaagatcagtaacctgtagatgcatagatcaattttcaaatcacttttctcattcattggagtcttccgagtgttctggttactgtggggttcctggtgtatattgaaataaagtattatggtatctcctgatttttcctttctgttctagttacagttgtctattcattctattgtagttccatacaagttttagatttttatccctattagtatgaaaaatgttattgatatttcagtgtcagctcacagagtctgctattagccataggatatgtggacatgtctatacctatattaattcttacaacccattaatatacaagctttctctatttctgtcttttcagattattttaccagttaactaatatttttgattgaagttttcacttctgtttataaattcatagctgaattaattttgaagatactgaaaatgacattgcatttatagttaattctcagaaaaatggaatttttctatagaaagggggtgatttctgtaggtttatatattaattgttgaactttggtaatttatctttcagatgcatgtgtgataccagaagatattatggaaaaacataatatagttctcagatggagggaaaatgcaaagatttattcccaatcaggggagaatattgaattcatgtgtaaacctggatatagaaaattcagaggatcacctccgtttcgtacaaagtgcattgagggtcacatcaattatcccacttgtgtataaaatcgctatacaattattagtaaaccttatggatgaacctttgtttagaaatgcacatgtatattactaatacagtttgaatttacatttgaaatattgtttagctcatttcttctaataagtatataaactttttttatatggtggttaatcagtaactttacagactgttgccacaaagcaagaacattgcattcaaaactcctaatccaaaatatgatatgtccaaggacaaactatgtctaagcaagaaaataaatgttagttcttcaatgtctgtttttattcaggacttttcagattttcttggataccttttgttgttaggttctgattcacagtgagtggaagacacactgactctgacttcaaattagtattacttgccaatacataacaaccaaactatcataatatcacaaatgtatacagctaattactgtgtcctacctttgtatcaataaagaaatctaagaaag

SEQ ID NO: 5 - DNA, 146 bp, Rattus norvegicus
tcttcgagtcaactgctcccagatagatccaagacatgagactgtcagcaagaattatttggcttatattatggactgtttgtgtagcagaaggtaagcttaaaaccaccacctttctcccttctgactgagccgcattataaaac

SEQ ID NO: 6 - DNA, 4176 bp, Artificial Sequence
  Synthetic
  misc_feature (1)..(3): Start Codon
  misc_feature (10)..(30): 5' NLS
  misc_feature (4126)..(4173): 3' NLS
  misc_feature (4174)..(4176): Stop Codon
atggacaagcccaagaaaaagcggaaagtgaagtacagcatcggcctggacatcggcaccaactctgtgggctgggccgtgatcaccgacgagtacaaggtgcccagcaagaaattcaaggtgctgggcaacaccgacaggcacagcatcaagaagaacctgatcggcgccctgctgttcgacagcggcgaaacagccgaggccaccagactgaagagaaccgccagaagaagatacaccaggcggaagaacaggatctgctatctgcaagagatcttcagcaacgagatggccaaggtggacgacagcttcttccacagactggaagagtccttcctggtggaagaggacaagaagcacgagagacaccccatcttcggcaacatcgtggacgaggtggcctaccacgagaagtaccccaccatctaccacctgagaaagaaactggtggacagcaccgacaaggccgacctgagactgatctacctggccctggcccacatgatcaagttcagaggccacttcctgatcgagggcgacctgaaccccgacaacagcgacgtggacaagctgttcatccagctggtgcagacctacaaccagctgttcgaggaaaaccccatcaacgccagcggcgtggacgccaaggctatcctgtctgccagactgagcaagagcagaaggctggaaaatctgatcgcccagctgcccggcgagaagaagaacggcctgttcggcaacctgattgccctgagcctgggcctgacccccaacttcaagagcaacttcgacctggccgaggatgccaaactgcagctgagcaaggacacctacgacgacgacctggacaacctgctggcccagatcggcgaccagtacgccgacctgttcctggccgccaagaacctgtctgacgccatcctgctgagcgacatcctgagagtgaacaccgagatcaccaaggcccccctgagcgcctctatgatcaagagatacgacgagcaccaccaggacctgaccctgctgaaagctctcgtgcggcagcagctgcctgagaagtacaaagaaatcttcttcgaccagagcaagaacggctacgccggctacatcgatggcggcgctagccaggaagagttctacaagttcatcaagcccatcctggaaaagatggacggcaccgaggaactgctcgtgaagctgaacagagaggacctgctgagaaagcagagaaccttcgacaacggcagcatcccccaccagatccacctgggagagctgcacgctatcctgagaaggcaggaagatttttacccattcctgaaggacaaccgggaaaagatcgagaagatcctgaccttcaggatcccctactacgtgggccccctggccagaggcaacagcagattcgcctggatgaccagaaagagcgaggaaaccatcaccccctggaacttcgaggaagtggtggacaagggcgccagcgcccagagcttcatcgagagaatgacaaacttcgataagaacctgcccaacgagaaggtgctgcccaagcacagcctgctgtacgagtacttcaccgtgtacaacgagctgaccaaagtgaaatacgtgaccgagggaatgagaaagcccgccttcctgagcggcgagcagaaaaaggccatcgtggacctgctgttcaagaccaacagaaaagtgaccgtgaagcagctgaaagaggactacttcaagaaaatcgagtgcttcgactccgtggaaatctccggcgtggaagatagattcaacgcctccctgggcacataccacgatctgctgaaaattatcaaggacaaggacttcctggataacgaagagaacgaggacattctggaagatatcgtgctgaccctgacactgtttgaggaccgcgagatgatcgaggaaaggctgaaaacctacgctcacctgttcgacgacaaagtgatgaagcagctgaagagaaggcggtacaccggctggggcaggctgagcagaaagctgatcaacggcatcagagacaagcagagcggcaagacaatcctggatttcctgaagtccgacggcttcgccaaccggaacttcatgcagctgatccacgacgacagcctgacattcaaagaggacatccagaaagcccaggtgtccggccagggcgactctctgcacgagcatatcgctaacctggccggcagccccgctatcaagaagggcatcctgcagacagtgaaggtggtggacgagctcgtgaaagtgatgggcagacacaagcccgagaacatcgtgatcgagatggctagagagaaccagaccacccagaagggacagaagaactcccgcgagaggatgaagagaatcgaagagggcatcaaagagctgggcagccagatcctgaaagaacaccccgtggaaaacacccagctgcagaacgagaagctgtacctgtactacctgcagaatggccgggatatgtacgtggaccaggaactggacatcaacagactgtccgactacgatgtggaccatatcgtgcctcagagctttctgaaggacgactccatcgataacaaagtgctgactcggagcgacaagaacagaggcaagagcgacaacgtgccctccgaagaggtcgtgaagaagatgaagaactactggcgacagctgctgaacgccaagctgattacccagaggaagttcgataacctgaccaaggccgagagaggcggcctgagcgagctggataaggccggcttcatcaagaggcagctggtggaaaccagacagatcacaaagcacgtggcacagatcctggactcccggatgaacactaagtacgacgaaaacgataagctgatccgggaagtgaaagtgatcaccctgaagtccaagctggtgtccgatttccggaaggatttccagttttacaaagtgcgcgagatcaacaactaccaccacgcccacgacgcctacctgaacgccgtcgtgggaaccgccctgatcaaaaagtaccctaagctggaaagcgagttcgtgtacggcgactacaaggtgtacgacgtgcggaagatgatcgccaagagcgagcaggaaatcggcaaggctaccgccaagtacttcttctacagcaacatcatgaactttttcaagaccgaaatcaccctggccaacggcgagatcagaaagcgccctctgatcgagacaaacggcgaaaccggggagatcgtgtgggataagggcagagacttcgccacagtgcgaaaggtgctgagcatgccccaagtgaatatcgtgaaaaagaccgaggtgcagacaggcggcttcagcaaagagtctatcctgcccaagaggaacagcgacaagctgatcgccagaaagaaggactgggaccccaagaagtacggcggcttcgacagccctaccgtggcctactctgtgctggtggtggctaaggtggaaaagggcaagtccaagaaactgaagagtgtgaaagagctgctggggatcaccatcatggaaagaagcagctttgagaagaaccctatcgactttctggaagccaagggctacaaagaagtgaaaaaggacctgatcatcaagctgcctaagtactccctgttcgagctggaaaacggcagaaagagaatgctggcctctgccggcgaactgcagaagggaaacgagctggccctgcctagcaaatatgtgaacttcctgtacctggcctcccactatgagaagctgaagggcagccctgaggacaacgaacagaaacagctgtttgtggaacagcataagcactacctggacgagatcatcgagcagatcagcgagttctccaagagagtgatcctggccgacgccaatctggacaaggtgctgtctgcctacaacaagcacagggacaagcctatcagagagcaggccgagaatatcatccacctgttcaccctgacaaacctgggcgctcctgccgccttcaagtactttgacaccaccatcgaccggaagaggtacaccagcaccaaagaggtgctggacgccaccctgatccaccagagcatcaccggcctgtacgagacaagaatcgacctgtctcagctgggaggcgacaagagacctgccgccactaagaaggccggacaggccaaaaagaagaagtga

SEQ ID NO: 7 - protein, 1391 aa, Artificial Sequence
  Synthetic
  MISC_FEATURE (4)..(10): 5' NLS
  MISC_FEATURE (1376)..(1391): 3' NLS
MDKPKKKRKVKYSIGLDIGTNSVGWAVITDEYKVPSKKFKVLGNTDRHSIKKNLIGALLFDSGETAEATRLKRTARRRYTRRKNRICYLQEIFSNEMAKVDDSFFHRLEESFLVEEDKKHERHPIFGNIVDEVAYHEKYPTIYHLRKKLVDSTDKADLRLIYLALAHMIKFRGHFLIEGDLNPDNSDVDKLFIQLVQTYNQLFEENPINASGVDAKAILSARLSKSRRLENLIAQLPGEKKNGLFGNLIALSLGLTPNFKSNFDLAEDAKLQLSKDTYDDDLDNLLAQIGDQYADLFLAAKNLSDAILLSDILRVNTEITKAPLSASMIKRYDEHHQDLTLLKALVRQQLPEKYKEIFFDQSKNGYAGYIDGGASQEEFYKFIKPILEKMDGTEELLVKLNREDLLRKQRTFDNGSIPHQIHLGELHAILRRQEDFYPFLKDNREKIEKILTFRIPYYVGPLARGNSRFAWMTRKSEETITPWNFEEVVDKGASAQSFIERMTNFDKNLPNEKVLPKHSLLYEYFTVYNELTKVKYVTEGMRKPAFLSGEQKKAIVDLLFKTNRKVTVKQLKEDYFKKIECFDSVEISGVEDRFNASLGTYHDLLKIIKDKDFLDNEENEDILEDIVLTLTLFEDREMIEERLKTYAHLFDDKVMKQLKRRRYTGWGRLSRKLINGIRDKQSGKTILDFLKSDGFANRNFMQLIHDDSLTFKEDIQKAQVSGQGDSLHEHIANLAGSPAIKKGILQTVKVVDELVKVMGRHKPENIVIEMARENQTTQKGQKNSRERMKRIEEGIKELGSQILKEHPVENTQLQNEKLYLYYLQNGRDMYVDQELDINRLSDYDVDHIVPQSFLKDDSIDNKVLTRSDKNRGKSDNVPSEEVVKKMKNYWRQLLNAKLITQRKFDNLTKAERGGLSELDKAGFIKRQLVETRQITKHVAQILDSRMNTKYDENDKLIREVKVITLKSKLVSDFRKDFQFYKVREINNYHHAHDAYLNAVVGTALIKKYPKLESEFVYGDYKVYDVRKMIAKSEQEIGKATAKYFFYSNIMNFFKTEITLANGEIRKRPLIETNGETGEIVWDKGRDFATVRKVLSMPQVNIVKKTEVQTGGFSKESILPKRNSDKLIARKKDWDPKKYGGFDSPTVAYSVLVVAKVEKGKSKKLKSVKELLGITIMERSSFEKNPIDFLEAKGYKEVKKDLIIKLPKYSLFELENGRKRMLASAGELQKGNELALPSKYVNFLYLASHYEKLKGSPEDNEQKQLFVEQHKHYLDEIIEQISEFSKRVILADANLDKVLSAYNKHRDKPIREQAENIIHLFTLTNLGAPAAFKYFDTTIDRKRYTSTKEVLDATLIHQSITGLYETRIDLSQLGGDKRPAATKKAGQAKKKK

SEQ ID NO: 8 - RNA, 99 nt, Artificial Sequence
  Synthetic
cauagcagagaggaacuggaugguuuuagagcuagaaauagcaaguuaaaauaaggcuaguccguuaucaacuugaaaaaguggcaccgagucggugcu

SEQ ID NO: 9 - RNA, 99 nt, Artificial Sequence
  Synthetic
auaaugcggcucagucagaaggguuuuagagcuagaaauagcaaguuaaaauaaggcuaguccguuaucaacuugaaaaaguggcaccgagucggugcu

SEQ ID NO: 10 - RNA, 99 nt, Artificial Sequence
  Synthetic
gcaaagauuuauuccccaucagguuuuagagcuagaaauagcaaguuaaaauaaggcuaguccguuaucaacuugaaaaaguggcaccgagucggugcu

SEQ ID NO: 11 - RNA, 99 nt, Artificial Sequence
  Synthetic
uuagauucaacagggaaaugugguuuuagagcuagaaauagcaaguuaaaauaaggcuaguccguuaucaacuugaaaaaguggcaccgagucggugcu

SEQ ID NO: 12 - DNA, 20 bp, Rattus norvegicus
catagcagagaggaactgga

SEQ ID NO: 13 - DNA, 20 bp, Rattus norvegicus
ataatgcggctcagtcagaa

SEQ ID NO: 14 - DNA, 20 bp, Rattus norvegicus
gcaaagatttattccccatc

SEQ ID NO: 15 - DNA, 20 bp, Rattus norvegicus
ttagattcaacagggaaatg

SEQ ID NO: 16 - DNA, 4250 bp, Rattus norvegicus
acagcacatacttctcttcgagtcaactgctcccagatagatccaagacatgagactgtcagcaagaattatttggcttatattatggactgtttgtgtagcagaagattgtaaaggtcctcctccaagagaaaattcagaaattctctcaggttcgtggtctgaacaactatattcagaaggcactcaggcaacctacaaatgccgccctggataccgaacacttggtactattgtaaaagtatgcaagaatggagaatgggtaccttctaacccatcaaggatatgtcggaaaaggccatgtgggcatcccggagacacaccctttgggtcctttaggctggcagttggatctgaatttgaatttggtgcaaaggttgtttatacatgtgatgaagggtaccaactcttaggtgaaattgattaccgtgaatgtgatgcagatgggtggaccaatgatattccaatatgtgaagttgtgaagtgcttgccagtgacagaactggagaatggaagaattgtgagtggtgcagccgaaccagaccaggaatattattttggacaggtggtacgctttgaatgcaactccggcttcaagattgaaggacagaaagaaatgcactgctcagaaaatggcctctggagcaatgaaaagccacagtgtgtggaaatttcttgcctgccaccacgagttgaaaatggagatggtatatatctgaaaccagtttacaaggagaatgaaagattccaatataaatgtaagcaaggttttgtgtacaaagaaagaggggatgctgtctgcacgggttctggatggaatcctcagccttcctgtgaagaaatgacatgtttgactccatatattccaaatggtatctacacacctcacaggattaaacacagaattgatgatgaaatcagatatgaatgtaaaaatggcttctatcctgcaacccgatcacctgtttcaaagtgtacaattactggctggatccctgctccaagatgtagcttgaaaccttgtgattttccacaattcaaacatggacgtctgtattatgaagaaagccggagaccctacttcccagtacctataggaaaggagtacagctattactgtgacaacgggtttacaacgccttcacagtcatactgggactaccttcgttgcacagtaaatgggtgggagcctgaagttccatgcctcaggcaatgtattttccattatgtggaatatggagaatctttatactggcaaagaagatatatagagggtcagtctgcaaaagtccagtgtcacagtggctatagtcttccaaatggtcaagatacaatattatgtacagaaaatggctggtcccctcctcccaaatgcgtccgtatcaagacttgttcagtatcagatatagaaattgaaaatgggtttttttctgaatctgattatacatatgctctaaatagaaaaacacggtatagatgtaaacagggatatgtaacaaataccggagaaatatcaggaataattacttgtcttcaagatggatggtcacctcgaccctcatgcattaagtcttgtgatatgcctgtatttgagaatgctatgactaagaataataacacatggtttaaactcaatgacaaattagactatgaatgtcacattggatatgaaaatgaatataaacataccaaaggctctataacatgtacttatgatggatggtctagtacaccctcctgttatgaaagagaatgcagcattcccctgttacaccaagacttagttgtttttcccagagaagtaaaatacaaagttggagattcgttgagtttctcttgccgttcaggacacagagttggagcagatttagtgcaatgctaccactttggatggtcccctaatttcccaacgtgtgaaggccaagtaaaatcatgtgaccaacctcttgaaatcccgaatggggaaataaagggaacaaaaaaagttgaatacagccatggtgacgtggtggaatatgattgcaaacctagatttctactgaagggacccaataaaatccagtgtgttgacgggaagtggacaaccttgccgatatgcgttgagtatgagagaacatgtggagaccttcctgcacttgagcatggctctgtccagttatctgtccctccctaccaccacggagattcagtggagttcacttgtgcagaaaccttcacaatgattgggcatgcagtagttttctgcattagtggaaggtggaccgagcttcctcaatgtgttgcaacagatcaactggagaagtgtaaagccccgaagtcaactggcatagatgcaattcatccaaataagaatgaatttaatcataactttagtgtgagttacagatgtagacaaaagcaggagtatgaacattcaatctgcatcaatggaagatgggatcctgaaccaaactgtacaagaaatgagaaaagattctgccctcctcccccacagattccaaatgcccaagtgattgaaaccacagtgaaatacttggatggagagaaagtatctgttctttgccaagatggttacctaactcagggcccagaagaaatggtgtgtaaacatggaaggtggcagtcgttaccacgctgcacggaaaaaattccatgttcccagccccctaaaattgaacatggatctattaagtcgcccaggtcctcagaagagagagatttaattgagtccagcagttatgaacacggaactacattcagctatgtctgtgatgatggattcaggatatctgaagaaaatagggtaacctgcaacatgggaaaatggagctctctgcctcgttgtgttggaataccttgtggacccccaccttcaattcctcttggtattgtttctcatgaactagaaagttaccaatatggagaggaggttacatacaattgttctgaaggctttggaattgatggaccagcatttattaaatgtgtaggaggacagtggtctgaaccacccaaatgcataaaaactgattgtgacaacttgcccacatttgaaattgccaaaccgacagaaaagaaaaaaaaatcatacaggtcaggagaacaagtgacattcagatgtccacctccgtatcgaatggatggctctgacattgtcacatgtgttaatacgaagtggattggacagccggtatgcaaagataattcctgtgtgaatccaccacatgtgccaaatgctactatactaacaaggcacaagactaaatatccatctggtgacaaagtacgttatgactgtaataaaccttttgaattatttggggaagtggaagtgatgtgccaaaacgggatttggacagaaccaccgaaatgcaaagattcaacagggaaatgtgggcctcctccacctattgacaatggagacatcacctccttgtcattaccagtatatgcaccattatcatcagttgaatatcaatgccagaactattatctacttaagggaaataagatagtaacatgtagaaatggaaagtggtctcagccaccaacctgcttacatgcatgtgtgataccagaagatattatggaaaaacataatatagttctcagatggagggaaaatgcaaagatttattcccaatcaggggagaatattgaattcatgtgtaaacctggatatagaaaattcagaggatcacctccgtttcgtacaaagtgcattgagggtcacatcaattatcccacttgtgtataaaatcgctatacaattattagtaaaccttatggatgaacctttgtttagaaatgcacatgtatattactaatacagtttgaatttacatttgaaatattgtttagctcatttcttctaataagtatataaactttttttatatggtggttaatcagtaactttacagactgttgccacaaagcaagaacattgcattcaaaactcctaatccaaaatatgatatgtccaaggacaaactatgtctaagcaagaaaataaatgttagttcttcaatgtctgtttttattcaggacttttcagattttcttggataccttttgttgttaggttctgattcacagtgagtggaagacacactgactctgacttcaaattagtattacttgccaatacataacaaccaaactatcataatatcacaaatgtatacagctaattactgtgtcctacctttgtatcaataaagaaatctaagaaagttcttgcttatgaa

SEQ ID NO: 17 - DNA, 24 bp, Rattus norvegicus
catagcagagaggaactggatggt

SEQ ID NO: 18 - DNA, 15 bp, Rattus norvegicus
gcacatacttctctt

SEQ ID NO: 19 - DNA, 26 bp, Rattus norvegicus
gtcaactgctcccagatagatccaag

SEQ ID NO: 20 - DNA, 26 bp, Rattus norvegicus
accaccacctttctcccttctgactg

SEQ ID NO: 21 - DNA, 16 bp, Rattus norvegicus
gccgcattataaaaca

SEQ ID NO: 22 - DNA, 25 bp, Rattus norvegicus
ttgctgataatatttctcatagcaa

SEQ ID NO: 23 - DNA, 22 bp, Rattus norvegicus
atttcctaaactaactttcaac

SEQ ID NO: 24 - DNA, 23 bp, Rattus norvegicus
gtggtaagtttaaaaaccgtgaa

SEQ ID NO: 25 - DNA, 24 bp, Rattus norvegicus
cgcctatgctgctggacttgtggt

SEQ ID NO: 26 - DNA, 25 bp, Rattus norvegicus
ctttcacttgactattgtaattgat